European Patent Specification EP 3 438 125 B1, published October 11, 2023. Title: YEAST STRAINS AND METHODS FOR CONTROLLING HYDROXYLATION OF RECOMBINANT COLLAGEN. Applicant: Modern Meadow. Application EP 18 XXX XXX.X. The sequence listing filed with the application follows.

SEQUENCE LISTING (55 sequences)

SEQ ID NO: 1 - DNA, 4401 bp, Bos taurus
  CDS (1)..(4401): Collagen Sequence 1: cDNA sequence - unoptimized natural DNA sequence from cow
atgatgagctttgtgcaaaaggggacctggttacttttcgctctgcttcatcccactgttattttggcacaacaggaagctgttgacggaggatgctcccatctcggtcagtcttatgcagatagagatgtatggaaaccagaaccgtgccaaatatgcgtctgtgactcaggatccgttctctgtgatgacataatatgtgacgaccaagaattagactgccccaaccctgaaatcccgtttggagaatgttgtgcagtttgcccacagcctccaacagctcccactcgccctcctaatggtcaaggacctcaaggccccaagggagatccaggtcctcctggtattcctgggcgaaatggcgatcctggtcctccaggatcaccaggctccccaggttctcccggccctcctggaatctgtgaatcatgtcctactggtggccagaactattctccccagtacgaagcatatgatgtcaagtctggagtagcaggaggaggaatcgcaggctatcctgggccagctggtcctcctggcccacccggaccccctggcacatctggccatcctggtgcccctggcgctccaggataccaaggtccccccggtgaacctgggcaagctggtccggcaggtcctccaggacctcctggtgctataggtccatctggccctgctggaaaagatggggaatcaggaagacccggacgacctggagagcgaggatttcctggccctcctggtatgaaaggcccagctggtatgcctggattccctggtatgaaaggacacagaggctttgatggacgaaatggagagaaaggcgaaactggtgctcctggattaaagggggaaaatggcgttccaggtgaaaatggagctcctggacccatgggtccaagaggggctcccggtgagagaggacggccaggacttcctggagccgcaggggctcgaggtaatgatggagctcgaggaagtgatggacaaccgggcccccctggtcctcctggaactgcaggattccctggttcccctggtgctaagggtgaagttggacctgcaggatctcctggttcaagtggcgcccctggacaaagaggagaacctggacctcagggacatgctggtgctccaggtccccctgggcctcctgggagtaatggtagtcctggtggcaaaggtgaaatgggtcctgctggcattcctggggctcctgggctgataggagctcgtggtcctccagggccacctggcaccaatggtgttcccgggcaacgaggtgctgcaggtgaacccggtaagaatggagccaaaggagacccaggaccacgtggggaacgcggagaagctggttctccaggtatcgcaggacctaagggtgaagatggcaaagatggttctcctggagaacctggtgcaaatggacttcctggagctgcaggagaaaggggtgtgcctggattccgaggacctgctggagcaaatggccttccaggagaaaagggtcctcctggggaccgtggtggcccaggccctgcagggcccagaggtgttgctggagagcccggcagagatggtctccctggaggtccaggattgaggggtattcctggtagccccggaggaccaggcagtgatgggaaaccagggcctcctggaagccaaggagagacgggtcgacccggtcctccaggttcacctggtccgcgaggccagcctggtgtcatgggcttccctggtcccaaaggaaacgatggtgctcctggaaaaaatggagaacgaggtggccctggaggtcctggccctcagggtcctgctggaaagaatggtgagaccggacctcagggtcctccaggacctactggcccttctggtgacaaaggagacacaggaccccctggtccacaaggactacaaggcttgcctggaacgagtggtcccccaggagaaaacggaaaacctggtgaacctggtccaaagggtgaggctggtgcacctggaattccaggaggcaagggtgattctggtgctcccggtgaacgcggacctcctggagcaggagggccccctggacctagaggtggagctggcccccctggtcccgaaggaggaaagggtgctgctggtccccctgggccacctggttctgctggtacacctggtctgcaaggaatgcctggagaaagagggggtcctggaggccctggtccaaagggtgataagggtgagcctggcagctcaggtgtcgatggtgctccagggaaagatggtccacggggtcccactggtcccattggtcctcctggcccagctggtcagcctggagataagggtgaaagtggtgcccctggagttccgggtatagctggtcctcgcggtggccctggtgagagaggcgaacaggggcccccaggacctgctggcttccctggtgctcctggccagaatggtgagcctggtgctaaaggagaaagaggcgctcctggtgagaaaggtgaaggaggccctcccggagccgcaggacccgccggaggttctgggcctgccggtcccccaggcccccaaggtgtcaaaggcgaacgtggcagtcctggtggtcctggtgctgctggcttccccggtggtcgtggtcctcctggccctcctggcagtaatggtaacccaggccccccaggctccagtggtgctccaggcaaagatggtcccccaggtccacctggcagtaatggtgctcctggcagccccgggatctctggaccaaagggtgattctggtccaccaggtgagaggggagcacctggcccccagggccctccgggagctccaggcccactaggaattgcaggacttactggagcacgaggtcttgcaggcccaccaggcatgccaggtgctaggggcagccccggcccacagggcatcaagggtgaaaatggtaaaccaggacctagtggtcagaatggagaacgtggtcctcctggcccccagggtcttcctggtctggctggtacagctggtgagcctggaagagatggaaaccctggatcagatggtctgccaggccgagatggagctccaggtgccaagggtgaccgtggtgaaaatggctctcctggtgcccctggagctcctggtcacccaggccctcctggtcctgtcggtccagctggaaagagcggtgacagaggagaaactggccctgctggtccttctggggcccccggtcctgccggatcaagaggtcctcctggtccccaaggcccacgcggtgacaaaggggaaaccggtgagcgtggtgctatgggcatcaaaggacatcgcggattccctggcaacccaggggcccccggatctccgggtcccgctggtcatcaaggtgcagttggcagtccaggccctgcaggccccagaggacctgttggacctagcgggccccctggaaaggacggagcaagtggacaccctggtcccattggaccaccggggccccgaggtaacagaggtgaaagaggatctgagggctccccaggccacccaggacaaccaggccctcctggacctcctggtgcccctggtccatgttgtggtgctggcggggttgctgccattgctggtgttggagccgaaaaagctggtggttttgccccatattatggagatgaaccgatagatttcaaaatcaacaccgatgagattatgacctcactcaaatcagtcaatggacaaatagaaagcctcattagtcctgatggttcccgtaaaaaccctgcacggaactgcagggacctgaaattctgccatcctgaactccagagtggagaatattgggttgatcctaaccaaggttgcaaattggatgctattaaagtctactgtaacatggaaactggggaaacgtgcataagtgccagtcctttgactatcccacagaagaactggtggacagattctggtgctgagaagaaacatgtttggtttggagaatccatggagggtggttttcagtttagctatggcaatcctgaacttcccgaagacgtcctcgatgtccagctggcattcctccgacttctctccagccgggcctctcagaacatcacatatcactgcaagaatagcattgcatacatggatcatgccagtgggaatgtaaagaaagccttgaagctgatggggtcaaatgaaggtgaattcaaggctgaaggaaatagcaaattcacatacacagttctggaggatggttgcacaaaacacactggggaatggggcaaaacagtcttccagtatcaaacacgcaaggccgtcagactacctattgtagatattgcaccctatgatatcggtggtcctgatcaagaatttggtgcggacattggccctgtttgctttttataa

SEQ ID NO: 2 - protein, 1466 aa, Bos taurus
MMSFVQKGTWLLFALLHPTVILAQQEAVDGGCSHLGQSYADRDVWKPEPCQICVCDSGSVLCDDIICDDQELDCPNPEIPFGECCAVCPQPPTAPTRPPNGQGPQGPKGDPGPPGIPGRNGDPGPPGSPGSPGSPGPPGICESCPTGGQNYSPQYEAYDVKSGVAGGGIAGYPGPAGPPGPPGPPGTSGHPGAPGAPGYQGPPGEPGQAGPAGPPGPPGAIGPSGPAGKDGESGRPGRPGERGFPGPPGMKGPAGMPGFPGMKGHRGFDGRNGEKGETGAPGLKGENGVPGENGAPGPMGPRGAPGERGRPGLPGAAGARGNDGARGSDGQPGPPGPPGTAGFPGSPGAKGEVGPAGSPGSSGAPGQRGEPGPQGHAGAPGPPGPPGSNGSPGGKGEMGPAGIPGAPGLIGARGPPGPPGTNGVPGQRGAAGEPGKNGAKGDPGPRGERGEAGSPGIAGPKGEDGKDGSPGEPGANGLPGAAGERGVPGFRGPAGANGLPGEKGPPGDRGGPGPAGPRGVAGEPGRDGLPGGPGLRGIPGSPGGPGSDGKPGPPGSQGETGRPGPPGSPGPRGQPGVMGFPGPKGNDGAPGKNGERGGPGGPGPQGPAGKNGETGPQGPPGPTGPSGDKGDTGPPGPQGLQGLPGTSGPPGENGKPGEPGPKGEAGAPGIPGGKGDSGAPGERGPPGAGGPPGPRGGAGPPGPEGGKGAAGPPGPPGSAGTPGLQGMPGERGGPGGPGPKGDKGEPGSSGVDGAPGKDGPRGPTGPIGPPGPAGQPGDKGESGAPGVPGIAGPRGGPGERGEQGPPGPAGFPGAPGQNGEPGAKGERGAPGEKGEGGPPGAAGPAGGSGPAGPPGPQGVKGERGSPGGPGAAGFPGGRGPPGPPGSNGNPGPPGSSGAPGKDGPPGPPGSNGAPGSPGISGPKGDSGPPGERGAPGPQGPPGAPGPLGIAGLTGARGLAGPPGMPGARGSPGPQGIKGENGKPGPSGQNGERGPPGPQGLPGLAGTAGEPGRDGNPGSDGLPGRDGAPGAKGDRGENGSPGAPGAPGHPGPPGPVGPAGKSGDRGETGPAGPSGAPGPAGSRGPPGPQGPRGDKGETGERGAMGIKGHRGFPGNPGAPGSPGPAGHQGAVGSPGPAGPRGPVGPSGPPGKDGASGHPGPIGPPGPRGNRGERGSEGSPGHPGQPGPPGPPGAPGPCCGAGGVAAIAGVGAEKAGGFAPYYGDEPIDFKINTDEIMTSLKSVNGQIESLISPDGSRKNPARNCRDLKFCHPELQSGEYWVDPNQGCKLDAIKVYCNMETGETCISASPLTIPQKNWWTDSGAEKKHVWFGESMEGGFQFSYGNPELPEDVLDVQLAFLRLLSSRASQNITYHCKNSIAYMDHASGNVKKALKLMGSNEGEFKAEGNSKFTYTVLEDGCTKHTGEWGKTVFQYQTRKAVRLPIVDIAPYDIGGPDQEFGADIGPVCFL

SEQ ID NO: 3 - DNA, 4404 bp, Artificial Sequence
  Col3A1 cDNA sequence (Sequence 2)
  CDS (1)..(4404)
atgatgtcttttgtccaaaagggtacttggttactttttgctctgttgcacccaactgttattctcgcacaacaggaagcagtagatggtggttgctcacatttaggtcaatcttacgcagatagagatgtatggaaacctgaaccatgtcaaatttgcgtgtgtgactcaggttcagtgctctgcgacgatatcatatgtgacgaccaggaattggactgtccaaacccagagataccattcggtgaatgttgtgctgtttgtccacagccaccaactgctcctacaagacctccaaacggtcaaggtccacaaggtcctaaaggtgatccgggtccacctggtattcctggtagaaatggtgaccctggacctcccggttccccaggtagcccaggatcacctgggcctcctggaatatgtgaatcctgcccaactggtggtcagaactatagcccacaatacgaggcctacgacgtcaaatctggtgttgctggaggaggtattgcaggctaccctggtcccgcagggcccccaggtccgccgggtccgcccggaacatcaggtcatcccggagcccctggtgcaccaggttatcagggaccgcccggagagcctggacaagctggtcccgctggaccccctggtccaccaggtgctattggaccaagtggtcctgccggaaaagacggtgaatccggtagacctggtagacccggcgaaaggggtttcccaggtcctcccggaatgaagggtccagccggtatgcccggttttcctgggatgaagggtcacagaggatttgatggtagaaacggagagaaaggcgaaaccggtgctcccggactgaagggtgaaaacggtgtccctggtgagaacggcgctcctggacctatgggtccacgtggtgctccaggagaaagaggcagaccaggattgcctggtgcagctggtgctagaggtaacgatggtgcccgtggttccgatggacaacccgggccacccggccctccaggtaccgctggatttcctggaagccctggtgctaagggggaggttggtccggctggtagtcccggaagtagcggtgccccaggtcaaagaggcgaaccaggccctcagggtcacgcaggagcacctggaccgcctggtcctcctggttcgaatggttcgcctggaggaaaaggtgaaatggggcccgcaggaatccccggtgcgcctggtcttattggtgccaggggtcctccaggcccgccaggtacaaatggtgtacccggacagcgaggagcagctggtgaacctggtaaaaacggtgccaaaggagatccaggtcctcgtggagagcgtggtgaagctggctctcccggtatcgccggtccaaaaggtgaggacggtaaggacggttcccctggtgagccaggtgcgaacggactgccaggtgcagccggagagcgaggagtcccaggattcaggggaccagccggtgctaacggcttgcctggtgaaaaagggccccctggtgataggggaggacccggtccagcaggccctcgtggagttgctggtgagcctggacgtgacggtttaccaggagggccaggtttgaggggtattcccgggtcccctggcggtcctggatcggatggaaaaccagggccaccaggttcgcagggtgaaacaggacgtccaggcccacccggctcacctggtccaaggggtcagcctggtgtcatgggtttccccggtccaaagggtaatgacggagcaccgggtaaaaatggtgaacgtggtggcccaggtggtccaggaccccaaggtccagctggaaaaaacggtgagacaggtcctcaaggacctccaggacctaccggtcctagcggagataagggagatacgggaccgccaggacctcaaggattgcaaggtttgcctggtacatctggccctcccggagaaaatggtaagcctggagagccaggaccaaaaggcgaagctggagccccaggtatccccggaggtaagggagactcaggtgctccgggtgagcgtggtcctccgggtgccggtggtccacctggacctagaggtggtgccgggccgccaggtcctgaaggtggtaaaggtgctgctggtccaccgggaccgcctggctctgctggtactcctggcttgcagggaatgccaggagagagaggtggacctggaggtcccggtccgaagggtgataaaggggagccaggatcatccggtgttgacggcgcacctggtaaagacggaccaaggggaccaacgggtccaatcggaccaccaggacccgctggccagccaggagataaaggcgagtccggagcacccggtgttcctggtatagctggacccaggggtggtcccggtgaaagaggtgaacagggcccaccgggtcccgccggtttccctggcgcccctggtcaaaatggagaaccaggtgcaaagggcgagagaggagccccaggagaaaagggtgagggaggaccacccggtgctgccggtccagctgggggttcaggtcctgctggaccaccaggtccacagggcgttaaaggtgagagaggaagtccaggtggtcctggagctgctggattcccaggtggccgtggacctcctggtccccctggatcgaatggtaatcctggtccgccaggtagttcgggtgctcctgggaaggacggtccacctggccccccaggtagtaacggtgcacctggtagtccaggtatatccggacctaaaggagattccggtccaccaggcgaaagaggggccccaggcccacagggtccaccaggagcccccggtcctctgggtattgctggtcttactggtgcacgtggactggccggtccacccggaatgcctggagcaagaggttcacctggaccacaaggtattaaaggagagaacggtaaacctggaccttccggtcaaaacggagagcggggacccccaggcccccaaggtctgccaggactagctggtaccgcaggggaaccaggaagagatggaaatccaggttcagacggactacccggtagagatggtgcaccgggggccaagggcgacaggggtgagaatggatctcctggtgcgccaggggcaccaggccacccaggtcccccaggtcctgtgggccctgctggaaagtcaggtgacaggggagagacaggcccggctggtccatctggcgcacccggaccagctggttccagaggcccacctggtccgcaaggccctagaggtgacaagggagagactggagaacgaggtgctatgggtatcaagggtcatagaggttttccgggtaatcccggcgccccaggttctcctggtccagctggccatcaaggtgcagtcggatcgcccggcccagccggtcccaggggccctgttggtccatccggtcctccaggaaaggatggtgcttctggacacccaggacctatcggacctccgggtcctagaggtaatagaggagaacgtggatccgagggtagtcctggtcaccctggtcaacctggcccaccagggcctccaggtgcacccggtccatgttgtggtgcaggcggtgtggctgcaattgctggtgtgggtgctgaaaaggccggcggtttcgctccatattatggtgatgaaccgattgattttaagatcaatactgacgaaatcatgacttccttaaagtccgttaatggtcaaattgagtctctaatctccccagatggttcacgtaaaaatcctgctagaaattgtagagatttgaagttttgtcaccccgagttgcagtccggtgagtactgggtggaccccaatcaaggttgtaagttagacgctattaaagtttactgcaatatggagacaggagaaacttgcatcagcgcttctccattgactatcccacaaaaaaattggtggactgactctggagctgagaaaaagcatgtatggttcggggaatcgatggaaggtggtttccaattcagctacggtaaccctgaacttcctgaagatgttcttgacgttcaattggcatttctgagattgttgtccagtcgtgcaagccaaaacattacataccattgcaaaaattccatcgcatatatggatcatgctagcggaaatgtgaaaaaggcattgaagctgatgggatcaaatgaaggtgaatttaaagcagagggtaattctaagtttacttacactgtattggaggatggttgtacgaagcatacaggtgaatggggtaaaacagtgtttcaatatcaaacccgcaaagcagttagattgccaatcgtcgatatcgcaccatacgacattggaggaccagatcaagagttcggagctgacatcggtccggtgtgtttcctttgataa

SEQ ID NO: 4 - protein, 1466 aa, Artificial Sequence; identical to SEQ ID NO: 2
  Synthetic Construct

SEQ ID NO: 5 - DNA, 940 bp, Artificial Sequence
  pAOX1 (Sequence 3)
agatctaacatccaaagacgaaaggttgaatgaaacctttttgccatccgacatccacaggtccattctcacacataagtgccaaacgcaacaggaggggatacactagcagcagaccgttgcaaacgcaggacctccactcctcttctcctcaacacccacttttgccatcgaaaaaccagcccagttattgggcttgattggagctcgctcattccaattccttctattaggctactaacaccatgactttattagcctgtctatcctggcccccctggcgaggttcatgtttgtttatttccgaatgcaacaagctccgcattacacccgaacatcactccagatgagggctttctgagtgtggggtcaaatagtttcatgttccccaaatggcccaaaactgacagtttaaacgctgtcttggaacctaatatgacaaaagcgtgatctcatccaagatgaactaagtttggttcgttgaaatgctaacggccagttggtcaaaaagaaacttccaaaagtcggcataccgtttgtcttgtttggtattgattgacgaatgctcaaaaataatctcattaatgcttagcgcagtctctctatcgcttctgaaccccggtgcacctgtgccgaaacgcaaatggggaaacacccgctttttggatgattatgcattgtctccacattgtatgcttccaagattctggtgggaatactgctgatagcctaacgttcatgatcaaaatttaactgttctaacccctacttgacagcaatatataaacagaaggaagctgccctgtcttaaacctttttttttatcatcattattagcttactttcataattgcgactggttccaattgacaagcttttgattttaacgacttttaacgacaacttgagaagatcaaaaaacaactaattattcgaaacg

SEQ ID NO: 6 - DNA, 1612 bp, Artificial Sequence
  Bovine P4HA cDNA Optimized (Sequence 4)
atgatttggtatatcctagtcgttggtattttgttgccacagtcactggctcacccaggcttcttcacttctataggacagatgactgatttgattcacacagaaaaagacctagttacaagccttaaagactatatcaaagctgaagaggataagttggagcaaatcaaaaagtgggcagagaaactcgatagattgactagtactgcaacaaaagatcctgagggttttgtgggtcacccagtgaatgctttcaagctgatgaagagacttaatacagagtggtcagaattggaaaacttggtacttaaagatatgagtgatggattcatttctaacttaacaattcaaagacaatactttccaaacgatgaggaccaagtaggagcagcaaaagctttgttgcgattgcaggacacatacaatttggacaccgacacgatatcgaagggtgatttacctggtgtgaagcataagtccttcctcactgtggaagattgttttgaattgggaaaagtcgcatatacagaagccgactactatcacacagaattatggatggagcaagctctgcgtcagttggacgaaggtgaagtttctaccgttgataaggtttcagttttggattacttatcatacgctgtttaccagcaaggtgatctggacaaagctctacttttaactaaaaagttgttggagctggacccggagcatcaaagagctaacggtaatctgaaatactttgaatacatcatggctaaggaaaaggacgcaaataagtcctcgtccgatgaccaatccgatcaaaagaccactctgaaaaaaaaaggtgcagctgttgactacctcccagagagacaaaagtatgaaatgctgtgtagaggagagggtatcaagatgactccaaggagacagaaaaagctgttctgtagatatcatgatgggaaccgtaacccaaaattcattcttgctccagcgaaacaggaagatgaatgggacaagcctagaatcattcgttttcatgacatcatctccgatgcagaaatagaggttgtgaaagacttggccaaaccaagattgagtagggctaccgtccatgaccctgagactggaaaattgactaccgcacaatatcgtgtctctaaatcagcatggttgtccggttacgagaatcccgtggtcagccgtatcaatatgcgtattcaagatttgactggtcttgacgtaagcactgctgaggaactacaagttgccaactatggtgtgggcggtcagtatgaaccccactttgatttcgccagaaaggacgagcctgatgcttttaaggagctaggtactggaaatagaatcgcaacgtggttgttctatatgtccgatgtgcttgctggaggagccacagttttccctgaggtaggtgcttctgtttggcctaaaaagggcacggccgtattttggtacaatctgtttgcatctggagaaggtgattacagcactagacatgctgcttgtcccgtcttagtcggtaataagtgggtttccaataagtggctgcatgagagaggtcaagagtttaggaggccatgcacattgtcagaattagaatgataatttt

SEQ ID NO: 7 - DNA, 1750 bp, Artificial Sequence
  Bovine P4HB (PDI) sequence, with Alpha pre-pro signal sequence (Sequence 5)
aaaatgagattcccatctattttcaccgctgtcttgttcgctgcctcctctgcattggctgcccctgttaacactaccactgaagacgagactgctcaaattccagctgaagcagttatcggttactctgaccttgagggtgatttcgacgtcgctgttttgcctttctctaactccactaacaacggtttgttgttcattaacaccactatcgcttccattgctgctaaggaagagggtgtctctctcgagaaaagagaggccgaagctgcacccgatgaggaagatcatgttttagtattgcataaaggaaatttcgatgaagctttggccgctcacaaatatctgctcgtcgagttttacgctccctggtgcggtcattgtaaggcccttgcaccagagtacgccaaggcagctggtaagttaaaggccgaaggttcagagatcagattagcaaaagttgatgctacagaagagtccgatcttgctcaacaatacggggttcgaggatacccaacaattaagtttttcaaaaatggtgatactgcttccccaaaggaatatactgctggtagagaggcagacgacatagtcaactggctcaaaaagagaacgggcccagctgcgtctacattaagcgacggagcagcagccgaagctcttgtggaatctagtgaagttgctgtaatcggtttctttaaggacatggaatctgattcagctaaacagttccttttagcagctgaagcaatcgatgacatccctttcggaatcacctcaaatagtgacgtgttcagcaagtaccaacttgacaaagatggagtggtcttgttcaaaaagtttgacgaaggcagaaacaatttcgagggtgaggttacaaaggagaaactgcttgatttcattaaacataaccaactacccttagttatcgaattcactgaacaaactgctcctaagattttcggtggagaaatcaaaacacatatcttgttgtttttgccaaagtccgtatcggattatgaaggtaaactctccaatttcaaaaaggccgctgagagctttaagggcaagattttgttcatctttattgactcagaccacacagacaatcagaggattttggagtttttcggtttgaaaaaggaggaatgtccagcagtccgtttgatcaccttggaggaggagatgaccaaatacaaaccagagtcggatgagttgactgccgagaagataacagaattttgtcacagatttctggaaggtaagatcaagcctcatcttatgtctcaagagttgcctgatgactgggataagcaaccagttaaagtattggtgggtaaaaactttgaggaagtggccttcgacgagaaaaaaaatgtctttgttgaattctatgctccgtggtgtggtcactgtaagcagctggcaccaatttgggataaactgggtgaaacttacaaagatcacgaaaacattgttattgcaaagatggacagtactgctaacgaagtggaggctgtgaaagttcactccttccctacgctgaagttctttcctgcatctgctgacagaactgttatcgactataatggagagaggacattggatggttttaaaaagtttcttgaatccggaggtcaagacggagctggtgacgacgatgatttggaagatctggaggaggctgaggaacctgatcttgaggaggatgacgaccagaaggcagtcaaagatgaactgtgataagggg

SEQ ID NO: 8 - DNA, 7479 bp, Artificial Sequence
  Collagen expression vectors - pDF-Col3A1 (Sequence 6)
ggatccttcagtaatgtcttgtttcttttgttgcagtggtgagccattttgacttcgtgaaagtttctttagaatagttgtttccagaggccaaacattccacccgtagtaaagtgcaagcgtaggaagaccaagactggcataaatcaggtataagtgtcgagcactggcaggtgatcttctgaaagtttctactagcagataagatccagtagtcatgcatatggcaacaatgtaccgtgtggatctaagaacgcgtcctactaaccttcgcattcgttggtccagtttgttgttatcgatcaacgtgacaaggttgtcgattccgcgtaagcatgcatacccaaggacgcctgttgcaattccaagtgagccagttccaacaatctttgtaatattagagcacttcattgtgttgcgcttgaaagtaaaatgcgaacaaattaagagataatctcgaaaccgcgacttcaaacgccaatatgatgtgcggcacacaataagcgttcatatccgctgggtgactttctcgctttaaaaaattatccgaaaaaattttctagagtgttgttactttatacttccggctcgtataatacgacaaggtgtaaggaggactaaaccatggctaaactcacctctgctgttccagtcctgactgctcgtgatgttgctggtgctgttgagttctggactgataggctcggtttctcccgtgacttcgtagaggacgactttgccggtgttgtacgtgacgacgttaccctgttcatctccgcagttcaggaccaggttgtgccagacaacactctggcatgggtatgggttcgtggtctggacgaactgtacgctgagtggtctgaggtcgtgtctaccaacttccgtgatgcatctggtccagctatgaccgagatcggtgaacagccctggggtcgtgagtttgcactgcgtgatccagctggtaactgcgtgcatttcgtcgcagaagagcaggactaacaattgacaccttacgattatttagagagtatttattagttttattgtatgtatacggatgttttattatctatttatgcccttatattctgtaactatccaaaagtcctatcttatcaagccagcaatctatgtccgcgaacgtcaactaaaaataagctttttatgctcttctctctttttttcccttcggtataattataccttgcatccacagattctcctgccaaattttgcataatcctttacaacatggctatatgggagcacttagcgccctccaaaacccatattgcctacgcatgtataggtgttttttccacaatattttctctgtgctctctttttattaaagagaagctctatatcggagaagcttctgtggccgttatattcggccttatcgtgggaccacattgcctgaattggtttgccccggaagattggggaaacttggatctgattaccttagctgcagaaaagggtaccactgagcgtcagaccccgtagaaaagatcaaaggatcttcttgagatcctttttttctgcgcgtaatctgctgcttgcaaacaaaaaaaccaccgctaccagcggtggtttgtttgccggatcaagagctaccaactctttttccgaaggtaactggcttcagcagagcgcagataccaaatactgttcttctagtgtagccgtagttaggccaccacttcaagaactctgtagcaccgcctacatacctcgctctgctaatcctgttaccagtggctgctgccagtggcgataagtcgtgtcttaccgggttggacccaagacgatagttaccggataaggcgcagcggtcgggctgaacggggggttcgtgcacacagcccagcttggagcgaacgacctacaccgaactgagatacctacagcgtgagctatgagaaagcgccacgcttcccgaagggagaaaggcggacaggtatccggtaagcggcagggtcggaacaggagagcgcacgagggagcttccagggggaaacgcctggtatctttatagtcctgtcgggtttcgccacctctgacttgagcgtcgatttttgtgatgctcgtcaggggggcggagcctatggaaaaacgccagcaacgcggcctttttacggttcctggccttttgctggccttttgctcacatgtatttaaataatgtatctaaacgcaaactccgagctggaaaaatgttaccggcgatgcgcggacaatttagaggcggcgatcaagaaacacctgctgggcgagcagtctggagcacagtcttcgatgggcccgagatcccaccgcgttcctgggtaccgggacgtgaggcagcgcgacatccatcaaatataccaggcgccaaccgagtctctcggaaaacagcttctggatatcttccgctggcggcgcaacgacgaataatagtccctggaggtgacggaatatatatgtgtggagggtaaatctgacagggtgtagcaaaggtaatattttcctaaaacatgcaatcggctgccccgcaacgggaaaaagaatgactttggcactcttcaccagagtggggtgtcccgctcgtgtgtgcaaataggctcccactggtcaccccggattttgcagaaaaacagcaagttccggggtgtctcactggtgtccgccaataagaggagccggcaggcacggagtctacatcaagctgtctccgatacactcgactaccatccgggtctctcagagaggggaatggcactataaataccgcctccttgcgctctctgccttcatcaatcaaatcatgatgtcttttgtccaaaagggtacttggttactttttgctctgttgcacccaactgttattctcgcacaacaggaagcagtagatggtggttgctcacatttaggtcaatcttacgcagatagagatgtatggaaacctgaaccatgtcaaatttgcgtgtgtgactcaggttcagtgctctgcgacgatatcatatgtgacgaccaggaattggactgtccaaacccagagataccattcggtgaatgttgtgctgtttgtccacagccaccaactgctcctacaagacctccaaacggtcaaggtccacaaggtcctaaaggtgatccgggtccacctggtattcctggtagaaatggtgaccctggacctcccggttccccaggtagcccaggatcacctgggcctcctggaatatgtgaatcctgcccaactggtggtcagaactatagcccacaatacgaggcctacgacgtcaaatctggtgttgctggaggaggtattgcaggctaccctggtcccgcagggcccccaggtccgccgggtccgcccggaacatcaggtcatcccggagcccctggtgcaccaggttatcagggaccgcccggagagcctggacaagctggtcccgctggaccccctggtccaccaggtgctattggaccaagtggtcctgccggaaaagacggtgaatccggtagacctggtagacccggcgaaaggggtttcccaggtcctcccggaatgaagggtccagccggtatgcccggttttcctgggatgaagggtcacagaggatttgatggtagaaacggagagaaaggcgaaaccggtgctcccggactgaagggtgaaaacggtgtccctggtgagaacggcgctcctggacctatgggtccacgtggtgctccaggagaaagaggcagaccaggattgcctggtgcagctggtgctagaggtaacgatggtgcccgtggttccgatggacaacccgggccacccggccctccaggtaccgctggatttcctggaagccctggtgctaagggggaggttggtccggctggtagtcccggaagtagcggtgccccaggtcaaagaggcgaaccaggccctcagggtcacgcaggagcacctggaccgcctggtcctcctggttcgaatggttcgcctggaggaaaaggtgaaatggggcccgcaggaatccccggtgcgcctggtcttattggtgccaggggtcctccaggcccgccaggtacaaatggtgtacccggacagcgaggagcagctggtgaacctggtaaaaacggtgccaaaggagatccaggtcctcgtggagagcgtggtgaagctggctctcccggtatcgccggtccaaaaggtgaggacggtaaggacggttcccctggtgagccaggtgcgaacggactgccaggtgcagccggagagcgaggagtcccaggattcaggggaccagccggtgctaacggcttgcctggtgaaaaagggccccctggtgataggggaggacccggtccagcaggccctcgtggagttgctggtgagcctggacgtgacggtttaccaggagggccaggtttgaggggtattcccgggtcccctggcggtcctggatcggatggaaaaccagggccaccaggttcgcagggtgaaacaggacgtccaggcccacccggctcacctggtccaaggggtcagcctggtgtcatgggtttccccggtccaaagggtaatgacggagcaccgggtaaaaatggtgaacgtggtggcccaggtggtccaggaccccaaggtccagctggaaaaaacggtgagacaggtcctcaaggacctccaggacctaccggtcctagcggagataagggagatacgggaccgccaggacctcaaggattgcaaggtttgcctggtacatctggccctcccggagaaaatggtaagcctggagagccaggaccaaaaggcgaagctggagccccaggtatccccggaggtaagggagactcaggtgctccgggtgagcgtggtcctccgggtgccggtggtccacctggacctagaggtggtgccgggccgccaggtcctgaaggtggtaaaggtgctgctggtccaccgggaccgcctggctctgctggtactcctggcttgcagggaatgccaggagagagaggtggacctggaggtcccggtccgaagggtgataaaggggagccaggatcatccggtgttgacggcgcacctggtaaagacggaccaaggggaccaacgggtccaatcggaccaccaggacccgctggccagccaggagataaaggcgagtccggagcacccggtgttcctggtatagctggacccaggggtggtcccggtgaaagaggtgaacagggcccaccgggtcccgccggtttccctggcgcccctggtcaaaatggagaaccaggtgcaaagggcgagagaggagccccaggagaaaagggtgagggaggaccacccggtgctgccggtccagctgggggttcaggtcctgctggaccaccaggtccacagggcgttaaaggtgagagaggaagtccaggtggtcctggagctgctggattcccaggtggccgtggacctcctggtccccctggatcgaatggtaatcctggtccgccaggtagttcgggtgctcctgggaaggacggtccacctggccccccaggtagtaacggtgcacctggtagtccaggtatatccggacctaaaggagattccggtccaccaggcgaaagaggggccccaggcccacagggtccaccaggagcccccggtcctctgggtattgctggtcttactggtgcacgtggactggccggtccacccggaatgcctggagcaagaggttcacctggaccacaaggtattaaaggagagaacggtaaacctggaccttccggtcaaaacggagagcggggacccccaggcccccaaggtctgccaggactagctggtaccgcaggggaaccaggaagagatggaaatccaggttcagacggactacccggtagagatggtgcaccgggggccaagggcgacaggggtgagaatggatctcctggtgcgccaggggcaccaggccacccaggtcccccaggtcctgtgggccctgctggaaagtcaggtgacaggggagagacaggcccggctggtccatctggcgcacccggaccagctggttccagaggcccacctggtccgcaaggccctagaggtgacaagggagagactggagaacgaggtgctatgggtatcaagggtcatagaggttttccgggtaatcccggcgccccaggttctcctggtccagctggccatcaaggtgcagtcggatcgcccggcccagccggtcccaggggccctgttggtccatccggtcctccaggaaaggatggtgcttctggacacccaggacctatcggacctccgggtcctagaggtaatagaggagaacgtggatccgagggtagtcctggtcaccctggtcaacctggcccaccagggcctccaggtgcacccggtccatgttgtggtgcaggcggtgtggctgcaattgctggtgtgggtgctgaaaaggccggcggtttcgctccatattatggtgatgaaccgattgattttaagatcaatactgacgaaatcatgacttccttaaagtccgttaatggtcaaattgagtctctaatctccccagatggttcacgtaaaaatcctgctagaaattgtagagatttgaagttttgtcaccccgagttgcagtccggtgagtactgggtggaccccaatcaaggttgtaagttagacgctattaaagtttactgcaatatggagacaggagaaacttgcatcagcgcttctccattgactatcccacaaaaaaattggtggactgactctggagctgagaaaaagcatgtatggttcggggaatcgatggaaggtggtttccaattcagctacggtaaccctgaacttcctgaagatgttcttgacgttcaattggcatttctgagattgttgtccagtcgtgcaagccaaaacattacataccattgcaaaaattccatcgcatatatggatcatgctagcggaaatgtgaaaaaggcattgaagctgatgggatcaaatgaaggtgaatttaaagcagagggtaattctaagtttacttacactgtattggaggatggttgtacgaagcatacaggtgaatggggtaaaacagtgtttcaatatcaaacccgcaaagcagttagattgccaatcgtcgatatcgcaccatacgacattggaggaccagatcaagagttcggagctgacatcggtccggtgtgtttcctttgataatcaagaggatgtcagaatgccatttgcctgagagatgcaggcttcatttttgatacttttttatttgtaacctatatagtataggattttttttgtcattttgtttcttctcgtacgagcttgctcctgatcagcctatctcgcagctgatgaatatcttgtggtaggggtttgggaaaatcattcgagtttgatgtttttcttggtatttcccactcctcttcagagtacagaagattaagtgagacgttcgtttgtgctccgga

SEQ ID NO: 9 - DNA, 7356 bp, Artificial Sequence
  Collagen expression vectors - pCAT1-Col3A1 (Sequence 7)
ggatccttcagtaatgtcttgtttcttttgttgcagtggtgagccattttgacttcgtgaaagtttctttagaatagttgtttccagaggccaaacattccacccgtagtaaagtgcaagcgtaggaagaccaagactggcataaatcaggtataagtgtcgagcactggcaggtgatcttctgaaagtttctactagcagataagatccagtagtcatgcatatggcaacaatgtaccgtgtggatctaagaacgcgtcctactaaccttcgcattcgttggtccagtttgttgttatcgatcaacgtgacaaggttgtcgattccgcgtaagcatgcatacccaaggacgcctgttgcaattccaagtgagccagttccaacaatctttgtaatattagagcacttcattgtgttgcgcttgaaagtaaaatgcgaacaaattaagagataatctcgaaaccgcgacttcaaacgccaatatgatgtgcggcacacaataagcgttcatatccgctgggtgactttctcgctttaaaaaattatccgaaaaaattttctagagtgttgttactttatacttccggctcgtataatacgacaaggtgtaaggaggactaaaccatggctaaactcacctctgctgttccagtcctgactgctcgtgatgttgctggtgctgttgagttctggactgataggctcggtttctcccgtgacttcgtagaggacgactttgccggtgttgtacgtgacgacgttaccctgttcatctccgcagttcaggaccaggttgtgccagacaacactctggcatgggtatgggttcgtggtctggacgaactgtacgctgagtggtctgaggtcgtgtctaccaacttccgtgatgcatctggtccagctatgaccgagatcggtgaacagccctggggtcgtgagtttgcactgcgtgatccagctggtaactgcgtgcatttcgtcgcagaagagcaggactaacaattgacaccttacgattatttagagagtatttattagttttattgtatgtatacggatgttttattatctatttatgcccttatattctgtaactatccaaaagtcctatcttatcaagccagcaatctatgtccgcgaacgtcaactaaaaataagctttttatgctcttctctctttttttcccttcggtataattataccttgcatccacagattctcctgccaaattttgcataatcctttacaacatggctatatgggagcacttagcgccctccaaaacccatattgcctacgcatgtataggtgttttttccacaatattttctctgtgctctctttttattaaagagaagctctatatcggagaagcttctgtggccgttatattcggccttatcgtgggaccacattgcctgaattggtttgccccggaagattggggaaacttggatctgattaccttagctgcagaaaagggtaccactgagcgtcagaccccgtagaaaagatcaaaggatcttcttgagatcctttttttctgcgcgtaatctgctgcttgcaaacaaaaaaaccaccgctaccagcggtggtttgtttgccggatcaagagctaccaactctttttccgaaggtaactggcttcagcagagcgcagataccaaatactgttcttctagtgtagccgtagttaggccaccacttcaagaactctgtagcaccgcctacatacctcgctctgctaatcctgttaccagtggctgctgccagtggcgataagtcgtgtcttaccgggttggacccaagacgatagttaccggataaggcgcagcggtcgggctgaacggggggttcgtgcacacagcccagcttggagcgaacgacctacaccgaactgagatacctacagcgtgagctatgagaaagcgccacgcttcccgaagggagaaaggcggacaggtatccggtaagcggcagggtcggaacaggagagcgcacgagggagcttccagggggaaacgcctggtatctttatagtcctgtcgggtttcgccacctctgacttgagcgtcgatttttgtgatgctcgtcaggggggcggagcctatggaaaaacgccagcaacgcggcctttttacggttcctggccttttgctggccttttgctcacatgtatttaaattaatcgaactccgaatgcggttctcctgtaaccttaattgtagcatagatcacttaaataaactcatggcctgacatctgtacacgttcttattggtcttttagcaatcttgaagtctttctattgttccggtcggcattacctaataaattcgaatcgagattgctagtacctgatatcatatgaagtaatcatcacatgcaagttccatgataccctctactaatggaattgaacaaagtttaagcttctcgcacgagaccgaatccatactatgcacccctcaaagttgggattagtcaggaaagctgagcaattaacttccctcgattggcctggacttttcgcttagcctgccgcaatcggtaagtttcattatcccagcggggtgatagcctctgttgctcatcaggccaaaatcatatataagctgtagacccagcacttcaattacttgaaattcaccataacacttgctctagtcaagacttacaattaaaatgatgtcttttgtccaaaagggtacttggttactttttgctctgttgcacccaactgttattctcgcacaacaggaagcagtagatggtggttgctcacatttaggtcaatcttacgcagatagagatgtatggaaacctgaaccatgtcaaatttgcgtgtgtgactcaggttcagtgctctgcgacgatatcatatgtgacgaccaggaattggactgtccaaacccagagataccattcggtgaatgttgtgctgtttgtccacagccaccaactgctcctacaagacctccaaacggtcaaggtccacaaggtcctaaaggtgatccgggtccacctggtattcctggtagaaatggtgaccctggacctcccggttccccaggtagcccaggatcacctgggcctcctggaatatgtgaatcctgcccaactggtggtcagaactatagcccacaatacgaggcctacgacgtcaaatctggtgttgctggaggaggtattgcaggctaccctggtcccgcagggcccccaggtccgccgggtccgcccggaacatcaggtcatcccggagcccctggtgcaccaggttatcagggaccgcccggagagcctggacaagctggtcccgctggaccccctggtccaccaggtgctattggaccaagtggtcctgccggaaaagacggtgaatccggtagacctggtagacccggcgaaaggggtttcccaggtcctcccggaatgaagggtccagccggtatgcccggttttcctgggatgaagggtcacagaggatttgatggtagaaacggagagaaaggcgaaaccggtgctcccggactgaagggtgaaaacggtgtccctggtgagaacggcgctcctggacctatgggtccacgtggtgctccaggagaaagaggcagaccaggattgcctggtgcagctggtgctagaggtaacgatggtgcccgtggttccgatggacaacccgggccacccggccctccaggtaccgctggatttcctggaagccctggtgctaagggggaggttggtccggctggtagtcccggaagtagcggtgccccaggtcaaagaggcgaaccaggccctcagggtcacgcaggagcacctggaccgcctggtcctcctggttcgaatggttcgcctggaggaaaaggtgaaatggggcccgcaggaatccccggtgcgcctggtcttattggtgccaggggtcctccaggcccgccaggtacaaatggtgtacccggacagcgaggagcagctggtgaacctggtaaaaacggtgccaaaggagatccaggtcctcgtggagagcgtggtgaagctggctctcccggtatcgccggtccaaaaggtgaggacggtaaggacggttcccctggtgagccaggtgcgaacggactgccaggtgcagccggagagcgaggagtcccaggattcaggggaccagccggtgctaacggcttgcctggtgaaaaagggccccctggtgataggggaggacccggtccagcaggccctcgtggagttgctggtgagcctggacgtgacggtttaccaggagggccaggtttgaggggtattcccgggtcccctggcggtcctggatcggatggaaaaccagggccaccaggttcgcagggtgaaacaggacgtccaggcccacccggctcacctggtccaaggggtcagcctggtgtcatgggtttccccggtccaaagggtaatgacggagcaccgggtaaaaatggtgaacgtggtggcccaggtggtccaggaccccaaggtccagctggaaaaaacggtgagacaggtcctcaaggacctccaggacctaccggtcctagcggagataagggagatacgggaccgccaggacctcaaggattgcaaggtttgcctggtacatctggccctcccggagaaaatggtaagcctggagagccaggaccaaaaggcgaagctggagccccaggtatccccggaggtaagggagactcaggtgctccgggtgagcgtggtcctccgggtgccggtggtccacctggacctagaggtggtgccgggccgccaggtcctgaaggtggtaaaggtgctgctggtccaccgggaccgcctggctctgctggtactcctggcttgcagggaatgccaggagagagaggtggacctggaggtcccggtccgaagggtgataaaggggagccaggatcatccggtgttgacggcgcacctggtaaagacggaccaaggggaccaacgggtccaatcggaccaccaggacccgctggccagccaggagataaaggcgagtccggagcacccggtgttcctggtatagctggacccaggggtggtcccggtgaaagaggtgaacagggcccaccgggtcccgccggtttccctggcgcccctggtcaaaatggagaaccaggtgcaaagggcgagagaggagccccaggagaaaagggtgagggaggaccacccggtgctgccggtccagctgggggttcaggtcctgctggaccaccaggtccacagggcgttaaaggtgagagaggaagtccaggtggtcctggagctgctggattcccaggtggccgtggacctcctggtccccctggatcgaatggtaatcctggtccgccaggtagttcgggtgctcctgggaaggacggtccacctggccccccaggtagtaacggtgcacctggtagtccaggtatatccggacctaaaggagattccggtccaccaggcgaaagaggggccccaggcccacagggtccaccaggagcccccggtcctctgggtattgctggtcttactggtgcacgtggactggccggtccacccggaatgcctggagcaagaggttcacctggaccacaaggtattaaaggagagaacggtaaacctggaccttccggtcaaaacggagagcggggacccccaggcccccaaggtctgccaggactagctggtaccgcaggggaaccaggaagagatggaaatccaggttcagacggactacccggtagagatggtgcaccgggggccaagggcgacaggggtgagaatggatctcctggtgcgccaggggcaccaggccacccaggtcccccaggtcctgtgggccctgctggaaagtcaggtgacaggggagagacaggcccggctggtccatctggcgcacccggaccagctggttccagaggcccacctggtccgcaaggccctagaggtgacaagggagagactggagaacgaggtgctatgggtatcaagggtcatagaggttttccgggtaatcccggcgccccaggttctcctggtccagctggccatcaaggtgcagtcggatcgcccggcccagccggtcccaggggccctgttggtccatccggtcctccaggaaaggatggtgcttctggacacccaggacctatcggacctccgggtcctagaggtaatagaggagaacgtggatccgagggtagtcctggtcaccctggtcaacctggcccaccagggcctccaggtgcacccggtccatgttgtggtgcaggcggtgtggctgcaattgctggtgtgggtgctgaaaaggccggcggtttcgctccatattatggtgatgaaccgattgattttaagatcaatactgacgaaatcatgacttccttaaagtccgttaatggtcaaattgagtctctaatctccccagatggttcacgtaaaaatcctgctagaaattgtagagatttgaagttttgtcaccccgagttgcagtccggtgagtactgggtggaccccaatcaaggttgtaagttagacgctattaaagtttactgcaatatggagacaggagaaacttgcatcagcgcttctccattgactatcccacaaaaaaattggtggactgactctggagctgagaaaaagcatgtatggttcggggaatcgatggaaggtggtttccaattcagctacggtaaccctgaacttcctgaagatgttcttgacgttcaattggcatttctgagattgttgtccagtcgtgcaagccaaaacattacataccattgcaaaaattccatcgcatatatggatcatgctagcggaaatgtgaaaaaggcattgaagctgatgggatcaaatgaaggtgaatttaaagcagagggtaattctaagtttacttacactgtattggaggatggttgtacgaagcatacaggtgaatggggtaaaacagtgtttcaatatcaaacccgcaaagcagttagattgccaatcgtcgatatcgcaccatacgacattggaggaccagatcaagagttcggagctgacatcggtccggtgtgtttcctttgataatcaagaggatgtcagaatgccatttgcctgagagatgcaggcttcatttttgatacttttttatttgtaacctatatagtataggattttttttgtcattttgtttcttctcgtacgagcttgctcctgatcagcctatctcgcagctgatgaatatcttgtggtaggggtttgggaaaatcattcgagtttgatgtttttcttggtatttcccactcctcttcagagtacagaagattaagtgagacgttcgtttgtgctccgga

SEQ ID NO: 10 - DNA, 404 bp, Artificial Sequence
  AOX1 landing pad (Sequence 8)
agaagcgatagagagactgcgctaagcattaatgagattatttttgagcattcgtcaatcaataccaaacaagacaaacggtatgccgacttttggaagtttctttttgaccaactggccgttagcatttcaacgaaccaaacttagttcatcttggatgagatcacgcttttgtcatattaggttccaagacagcgtttaaactgtcagttttgggccatttggggaacatgaaactatttgaccccacactcagaaagccctcatctggagtgatgttcgggtgtaatgcggagcttgttgcattcggaaataaacaaacatgaacctcgccaggggggccaggatagacaggctaataaagtcatggtgttagtagcctaatagaaggaattggaatgagc

SEQ ID NO: 11 - DNA, 7942 bp, Artificial Sequence
  MMV63 (Sequence 9)
ttctttcctgcggtacccagatccaattcccgctttgactgcctgaaatctccatcgcctacaatgatgacatttggatttggttgactcatgttggtattgtgaaatagacgcagatcgggaacactgaaaaatacacagttattattcatttaaataacatccaaagacgaaaggttgaatgaaacctttttgccatccgacatccacaggtccattctcacacataagtgccaaacgcaacaggaggggatacactagcagcagaccgttgcaaacgcaggacctccactcctcttctcctcaacacccacttttgccatcgaaaaaccagcccagttattgggcttgattggagctcgctcattccaattccttctattaggctactaacaccatgactttattagcctgtctatcctggcccccctggcgaggttcatgtttgtttatttccgaatgcaacaagctccgcattacacccgaacatcactccagatgagggctttctgagtgtggggtcaaatagtttcatgttccccaaatggcccaaaactgacagtttaaacgctgtcttggaacctaatatgacaaaagcgtgatctcatccaagatgaactaagtttggttcgttgaaatgctaacggccagttggtcaaaaagaaacttccaaaagtcggcataccgtttgtcttgtttggtattgattgacgaatgctcaaaaataatctcattaatgcttagcgcagtctctctatcgcttctgaaccccggtgcacctgtgccgaaacgcaaatggggaaacacccgctttttggatgattatgcattgtctccacattgtatgcttccaagattctggtgggaatactgctgatagcctaacgttcatgatcaaaatttaactgttctaacccctacttgacagcaatatataaacagaaggaagctgccctgtcttaaacctttttttttatcatcattattagcttactttcataattgcgactggttccaattgacaagcttttgattttaacgacttttaacgacaacttgagaagatcaaaaaacaactaattattgaaagaattcaaaacgatgagctttgtgcaaaaggggacctggttacttttcgctctgcttcatcccactgttattttggcacaacaggaagctgttgacggaggatgctcccatctcggtcagtcttatgcagatagagatgtatggaaaccagaaccgtgccaaatatgcgtctgtgactcaggatccgttctctgtgatgacataatatgtgacgaccaagaattagactgccccaaccctgaaatcccgtttggagaatgttgtgcagtttgcccacagcctccaacagctcccactcgccctcctaatggtcaaggacctcaaggccccaagggagatccaggtcctcctggtattcctgggcgaaatggcgatcctggtcctccaggatcaccaggctccccaggttctcccggccctcctggaatctgtgaatcatgtcctactggtggccagaactattctccccagtacgaagcatatgatgtcaagtctggagtagcaggaggaggaatcgcaggctatcctgggccagctggtcctcctggcccacccggaccccctggcacatctggccatcctggtgcccctggcgctccaggataccaaggtccccccggtgaacctgggcaagctggtccggcaggtcctccaggacctcctggtgctataggtccatctggccctgctggaaaagatggggaatcaggaagacccggacgacctggagagcgaggatttcctggccctcctggtatgaaaggcccagctggtatgcctggattccctggtatgaaaggacacagaggctttgatggacgaaatggagagaaaggcgaaactggtgctcctggattaaagggggaaaatggcgttccaggtgaaaatggagctcctggacccatgggtccaagaggggctcccggtgagagaggacggccaggacttcctggagccgcaggggctcgaggtaatgatggagctcgaggaagtgatggacaaccgggcccccctggtcctcctggaactgcaggattccctggttcccctggtgctaagggtgaagttggacctgcaggatctcctggttcaagtggcgcccctggacaaagaggagaacctggacctcagggacatgctggtgctccaggtccccctgggcctcctgggagtaatggtagtcctggtggcaaaggtgaaatgggtcctgctggcattcctggggctcctgggctgataggagctcgtggtcctccagggccacctggcaccaatggtgttcccgggcaacgaggtgctgcaggtgaacccggtaagaatggagccaaaggagacccaggaccacgtggggaacgcggagaagctggttctccaggtatcgcaggacctaagggtgaagatggcaaagatggttctcctggagaacctggtgcaaatggacttcctggagctgcaggagaaaggggtgtgcctggattccgaggacctgctggagcaaatggccttccaggagaaaagggtcctcctggggaccgtggtggcccaggccctgcagggcccagaggtgttgctggagagcccggcagagatggtctccctggaggtccaggattgaggggtattcctggtagccccggaggaccaggcagtgatgggaaaccagggcctcctggaagccaaggagagacgggtcgacccggtcctccaggttcacctggtccgcgaggccagcctggtgtcatgggcttccctggtcccaaaggaaacgatggtgctcctggaaaaaatggagaacgaggtggccctggaggtcctggccctcagggtcctgctggaaagaatggtgagaccggacctcagggtcctccaggacctactggcccttctggtgacaaaggagacacaggaccccctggtccacaaggactacaaggcttgcctggaacgagtggtcccccaggagaaaacggaaaacctggtgaacctggtccaaagggtgaggctggtgcacctggaattccaggaggcaagggtgattctggtgctcccggtgaacgcggacctcctggagcaggagggccccctggacctagaggtggagctggcccccctggtcccgaaggaggaaagggtgctgctggtccccctgggccacctggttctgctggtacacctggtctgcaaggaatgcctggagaaagagggggtcctggaggccctggtccaaagggtgataagggtgagcctggcagctcaggtgtcgatggtgctccagggaaagatggtccacggggtcccactggtcccattggtcctcctggcccagctggtcagcctggagataagggtgaaagtggtgcccctggagttccgggtatagctggtcctcgcggtggccctggtgagagaggcgaacaggggcccccaggacctgctggcttccctggtgctcctggccagaatggtgagcctggtgctaaaggagaaagaggcgctcctggtgagaaaggtgaaggaggccctcccggagccgcaggacccgccggaggttctgggcctgccggtcccccaggcccccaaggtgtcaaaggcgaacgtggcagtcctggtggtcctggtgctgctggcttccccggtggtcgtggtcctcctggccctcctggcagtaatggtaacccaggccccccaggctccagtggtgctccaggcaaagatggtcccccaggtccacctggcagtaatggtgctcctggcagccccgggatctctggaccaaagggtgattctggtccaccaggtgagaggggagcacctggcccccagggccctccgggagctccaggcccactaggaattgcaggacttactggagcacgaggtcttgcaggcccaccaggcatgccaggtgctaggggcagccccggcccacagggcatcaagggtgaaaatggtaaaccaggacctagtggtcagaatggagaacgtggtcctcctggcccccagggtcttcctggtctggctggtacagctggtgagcctggaagagatggaaaccctggatcagatggtctgccaggccgagatggagctccaggtgccaagggtgaccgtggtgaaaatggctctcctggtgcccctggagctcctggtcacccaggccctcctggtcctgtcggtccagctggaaagagcggtgacagaggagaaactggccctgctggtccttctggggcccccggtcctgccggatcaagaggtcctcctggtccccaaggcccacgcggtgacaaaggggaaaccggtgagcgtggtgctatgggcatcaaaggacatcgcggattccctggcaacccaggggcccccggatctccgggtcccgctggtcatcaaggtgcagttggcagtccaggccctgcaggccccagaggacctgttggacctagcgggccccctggaaaggacggagcaagtggacaccctggtcccattggaccaccggggccccgaggtaacagaggtgaaagaggatctgagggctccccaggccacccaggacaaccaggccctcctggacctcctggtgcccctggtccatgttgtggtgctggcggggttgctgccattgctggtgttggagccgaaaaagctggtggttttgccccatattatggagatgaaccgatagatttcaaaatcaacaccgatgagattatgacctcactcaaatcagtcaatggacaaatagaaagcctcattagtcctgatggttcccgtaaaaaccctgcacggaactgcagggacctgaaattctgccatcctgaactccagagtggagaatattgggttgatcctaaccaaggttgcaaattggatgctattaaagtctactgtaacatggaaactggggaaacgtgcataagtgccagtcctttgactatcccacagaagaactggtggacagattctggtgctgagaagaaacatgtttggtttggagaatccatggagggtggttttcagtttagctatggcaatcctgaacttcccgaagacgtcctcgatgtccagctggcattcctccgacttctctccagccgggcctctcagaacatcacatatcactgcaagaatagcattgcatacatggatcatgccagtgggaatgtaaagaaagccttgaagctgatggggtcaaatgaaggtgaattcaaggctgaaggaaatagcaaattcacatacacagttctggaggatggttgcacaaaacacactggggaatggggcaaaacagtcttccagtatcaaacacgcaaggccgtcagactacctattgtagatattgcaccctatgatatcggtggtcctgatcaagaatttggtgcggacattggccctgtttgctttttataaaggggcggccgctcaagaggatgtcagaatgccatttgcctgagagatgcaggcttcatttttgatacttttttatttgtaacctatatagtataggattttttttgtcattttgtttcttctcgtacgagcttgctcctgatcagcctatctcgcagcagatgaatatcttgtggtaggggtttgggaaaatcattcgagtttgatgtttttcttggtatttcccactcctcttcagagtacagaagattaagtgaaaccttcgtttgtgcggatccttcagtaatgtcttgtttcttttgttgcagtggtgagccattttgacttcgtgaaagtttctttagaatagttgtttccagaggccaaacattccacccgtagtaaagtgcaagcgtaggaagaccaagactggcataaatcaggtataagtgtcgagcactggcaggtgatcttctgaaagtttctactagcagataagatccagtagtcatgcatatggcaacaatgtaccgtgtggatctaagaacgcgtcctactaaccttcgcattcgttggtccagtttgttgttatcgatcaacgtgacaaggttgtcgattccgcgtaagcatgcatacccaaggacgcctgttgcaattccaagtgagccagttccaacaatctttgtaatattagagcacttcattgtgttgcgcttgaaagtaaaatgcgaacaaattaagagataatctcgaaaccgcgacttcaaacgccaatatgatgtgcggcacacaataagcgttcatatccgctgggtgactttctcgctttaaaaaattatccgaaaaaattttctagagtgttgttactttatacttccggctcgtataatacgacaaggtgtaaggaggactaaaccatggctaaactcacctctgctgttccagtcctgactgctcgtgatgttgctggtgctgttgagttctggactgatagactcggtttctcccgtgacttcgtagaggacgactttgccggtgttgtacgtgacgacgttaccctgttcatctccgcagttcaggaccaggttgtgccagacaacactctggcatgggtatgggttcgtggtctggacgaactgtacgctgagtggtctgaggtcgtgtctaccaacttccgtgatgcatctggtccagctatgaccgagatcggtgaacagccctggggtcgtgagtttgcactgcgtgatccagctggtaactgcgtgcatttcgtcgcagaagagcaggactaacaattgacaccttacgattatttagagagtatttattagttttattgtatgtatacggatgttttattatctatttatgcccttatattctgtaactatccaaaagtcctatcttatcaagccagcaatctatgtccgcgaacgtcaactaaaaataagctttttatgctcttctctctttttttcccttcggtataattataccttgcatccacagattctcctgccaaattttgcataatcctttacaacatggctatatgggagcacttagcgccctccaaaacccatattgcctacgcatgtataggtgttttttccacaatattttctctgtgctctctttttattaaagagaagctctatatcggagaagcttctgtggccgttatattcggccttatcgtgggaccacattgcctgaattggtttgccccggaagattggggaaacttggatctgattaccttagctgcaggtaccactgagcgtcagaccccgtagaaaagatcaaaggatcttcttgagatcctttttttctgcgcgtaatctgctgcttgcaaacaaaaaaaccaccgctaccagcggtggtttgtttgccggatcaagagctaccaactctttttccgaaggtaactggcttcagcagagcgcagataccaaatactgttcttctagtgtagccgtagttaggccaccacttcaagaactctgtagcaccgcctacatacctcgctctgctaatcctgttaccagtggctgctgccagtggcgataagtcgtgtcttaccgggttggactcaagacgatagttaccggataaggcgcagcggtcgggctgaacggggggttcgtgcacacagcccagcttggagcgaacgacctacaccgaactgagatacctacagcgtgagctatgagaaagcgccacgcttcccgaagggagaaaggcggacaggtatccggtaagcggcagggtcggaacaggagagcgcacgagggagcttccagggggaaacgcctggtatctttatagtcctgtcgggtttcgccacctctgacttgagcgtcgatttttgtgatgctcgtcaggggggcggagcctatggaaaaacgccagcaacgcggcctttttacggttcctggccttttgctggccttttgctcacatg

SEQ ID NO: 12 - DNA, 7954 bp, Artificial Sequence
  MMV77 (Sequence 10)
ccgtagaaaagatcaaaggatcttcttgagatcctttttttctgcgcgtaatctgctgcttgcaaacaaaaaaaccaccgctaccagcggtggtttgtttgccggatcaagagctaccaactctttttccgaaggtaactggcttcagcagagcgcagataccaaatactgttcttctagtgtagccgtagttaggccaccacttcaagaactctgtagcaccgcctacatacctcgctctgctaatcctgttaccagtggctgctgccagtggcgataagtcgtgtcttaccgggttggactcaagacgatagttaccggataaggcgcagcggtcgggctgaacggggggttcgtgcacacagcccagcttggagcgaacgacctacaccgaactgagatacctacagcgtgagctatgagaaagcgccacgcttcccgaagggagaaaggcggacaggtatccggtaagcggcagggtcggaacaggagagcgcacgagggagcttccagggggaaacgcctggtatctttatagtcctgtcgggtttcgccacctctgacttgagcgtcgatttttgtgatgctcgtcaggggggcggagcctatggaaaaacgccagcaacgcggcctttttacggttcctggccttttgctggccttttgctcacatgttctttcctgcggtacccagatccaattcccgctttgactgcctgaaatctccatcgcctacaatgatgacatttggatttggttgactcatgttggtattgtgaaatagacgcagatcgggaacactgaaaaatacacagttattattcatttaaataacatccaaagacgaaaggttgaatgaaacctttttgccatccgacatccacaggtccattctcacacataagtgccaaacgcaacaggaggggatacactagcagcagaccgttgcaaacgcaggacctccactcctcttctcctcaacacccacttttgccatcgaaaaaccagcccagttattgggcttgattggagctcgctcattccaattccttctattaggctactaacaccatgactttattagcctgtctatcctggcccccctggcgaggttcatgtttgtttatttccgaatgcaacaagctccgcattacacccgaacatcactccagatgagggctttctgagtgtggggtcaaatagtttcatgttccccaaatggcccaaaactgacagtttaaacgctgtcttggaacctaatatgacaaaagcgtgatctcatccaagatgaactaagtttggttcgttgaaatgctaacggccagttggtcaaaaagaaacttccaaaagtcggcataccgtttgtcttgtttggtattgattgacgaatgctcaaaaataatctcattaatgcttagcgcagtctctctatcgcttctgaaccccggtgcacctgtgccgaaacgcaaatggggaaacacccgctttttggatgattatgcattgtctccacattgtatgcttccaagattctggtgggaatactgctgatagcctaacgttcatgatcaaaatttaactgttctaacccctacttgacagcaatatataaacagaaggaagctgccctgtcttaaacctttttttttatcatcattattagcttactttcataattgcgactggttccaattgacaagcttttgattttaacgacttttaacgacaacttgagaagatcaaaaaacaactaattattgaaagaattcaaaacgatgatgtcttttgtccaaaagggtacttggttactttttgctctgttgcacccaactgttattctcgcacaacaggaagcagtagatggtggttgctcacatttaggtcaatcttacgcagatagagatgtatggaaacctgaaccatgtcaaatttgcgtgtgtgactcaggttcagtgctctgcgacgatatcatatgtgacgaccaggaattggactgtccaaacccagagataccattcggtgaatgttgtgctgtttgtccacagccaccaactgctcctacaagacctccaaacggtcaaggtccacaaggtcctaaaggtgatccgggtccacctggtattcctggtagaaatggtgaccctggacctcccggttccccaggtagcccaggatcacctgggcctcctggaatatgtgaatcctgcccaactggtggtcagaactatagcccacaatacgaggcctacgacgtcaaatctggtgttgctggaggaggtattgcaggctaccctggtcccgcagggcccccaggtccgccgggtccgcccggaacatcaggtcatcccggagcccctggtgcaccaggttatcagggaccgcccggagagcctggacaagctggtcccgctggaccccctggtccaccaggtgctattggaccaagtggtcctgccggaaaagacggtgaatccggtagacctggtagacccggcgaaaggggtttcccaggtcctcccggaatgaagggtccagccggtatgcccggttttcctgggatgaagggtcacagaggatttgatggtagaaacggagagaaaggcgaaaccggtgctcccggactgaagggtgaaaacggtgtccctggtgagaacggcgctcctggacctatgggtccacgtggtgctccaggagaaagaggcagaccaggattgcctggtgcagctggtgctagaggtaacgatggtgcccgtggttccgatggacaacccgggccacccggccctccaggtaccgctggatttcctggaagccctggtgctaagggggaggttggtccggctggtagtcccggaagtagcggtgccccaggtcaaagaggcgaaccaggccctcagggtcacgcaggagcacctggaccgcctggtcctcctggttcgaatggttcgcctggaggaaaaggtgaaatggggcccgcaggaatccccggtgcgcctggtcttattggtgccaggggtcctccaggcccgccaggtacaaatggtgtacccggacagcgaggagcagctggtgaacctggtaaaaacggtgccaaaggagatccaggtcctcgtggagagcgtggtgaagctggctctcccggtatcgccggtccaaaaggtgaggacggtaaggacggttcccctggtgagccaggtgcgaacggactgccaggtgcagccggagagcgaggagtcccaggattcaggggaccagccggtgctaacggcttgcctggtgaaaaagggccccctggtgataggggaggacccggtccagcaggccctcgtggagttgctggtgagcctggacgtgacggtttaccaggagggccaggtttgaggggtattcccgggtcccctggcggtcctggatcggatggaaaaccagggccaccaggttcgcagggtgaaacaggacgtccaggcccacccggctcacctggtccaaggggtcagcctggtgtcatgggtttccccggtccaaagggtaatgacggagcaccgggtaaaaatggtgaacgtggtggcccaggtggtccaggaccccaaggtccagctggaaaaaacggtgagacaggtcctcaaggacctccaggacctaccggtcctagcggagataagggagatacgggaccgccaggacctcaaggattgcaaggtttgcctggtacatctggccctcccggagaaaatggtaagcctggagagccaggaccaaaaggcgaagctggagccccaggtatccccggaggtaagggagactcaggtgctccgggtgagcgtggtcctccgggtgccggtggtccacctggacctagaggtggtgccgggccgccaggtcctgaaggtggtaaaggtgctgctggtccaccgggaccgcctggctctgctggtactcctggcttgcagggaatgccaggagagagaggtggacctggaggtcccggtccgaagggtgataaaggggagccaggatcatccggtgttgacggcgcacctggtaaagacggaccaaggggaccaacgggtccaatcggaccaccaggacccgctggccagccaggagataaaggcgagtccggagcacccggtgttcctggtatagctggacccaggggtggtcccggtgaaagaggtgaacagggcccaccgggtcccgccggtttccctggcgcccctggtcaaaatggagaaccaggtgcaaagggcgagagaggagccccaggagaaaagggtgagggaggaccacccggtgctgccggtccagctgggggttcaggtcctgctggaccaccaggtccacagggcgttaaaggtgagagaggaagtccaggtggtcctggagctgctggattcccaggtggccgtggacctcctggtccccctggatcgaatggtaatcctggtccgccaggtagttcgggtgctcctgggaaggacggtccacctggccccccaggtagtaacggtgcacctggtagtccaggtatatccggacctaaaggagattccggtccaccaggcgaaagaggggccccaggcccacagggtccaccaggagcccccggtcctctgggtattgctggtcttactggtgcacgtggactggccggtccacccggaatgcctggagcaagaggttcacctggaccacaaggtattaaaggagagaacggtaaacctggaccttccggtcaaaacggagagcggggacccccaggcccccaaggtctgccaggactagctggtaccgcaggggaaccaggaagagatggaaatccaggttcagacggactacccggtagagatggtgcaccgggggccaagggcgacaggggtgagaatggatctcctggtgcgccaggggcaccaggccacccaggtcccccaggtcctgtgggccctgctggaaagtcaggtgacaggggagagacaggcccggctggtccatctggcgcacccggaccagctggttccagaggcccacctggtccgcaaggccctagaggtgacaagggagagactggagaacgaggtgctatgggtatcaagggtcatagaggttttccgggtaatcccggcgccccaggttctcctggtccagctggccatcaaggtgcagtcggatcgcccggcccagccggtcccaggggccctgttggtccatccggtcctccaggaaaggatggtgcttctggacacccaggacctatcggacctccgggtcctagaggtaatagaggagaacgtggatccgagggtagtcctggtcaccctggtcaacctggcccaccagggcctccaggtgcacccggtccatgttgtggtgcaggcggtgtggctgcaattgctggtgtgggtgctgaaaaggccggcggtttcgctccatattatggtgatgaaccgattgattttaagatcaatactgacgaaatcatgacttccttaaagtccgttaatggtcaaattgagtctctaatctccccagatggttcacgtaaaaatcctgctagaaattgtagagatttgaagttttgtcaccccgagttgcagtccggtgagtactgggtggaccccaatcaaggttgtaagttagacgctattaaagtttactgcaatatggagacaggagaaacttgcatcagcgcttctccattgactatcccacaaaaaaattggtggactgactctggagctgagaaaaagcatgtatggttcggggaatcgatggaaggtggtttccaattcagctacggtaaccctgaacttcctgaagatgttcttgacgttcaattggcatttctgagattgttgtccagtcgtgcaagccaaaacattacataccattgcaaaaattccatcgcatatatggatcatgctagcggaaatgtgaaaaaggcattgaagctgatgggatcaaatgaaggtgaatttaaagcagagggtaattctaagtttacttacactgtattggaggatggttgtacgaagcatacaggtgaatggggtaaaacagtgtttcaatatcaaacccgcaaagcagttagattgccaatcgtcgatatcgcaccatacgacattggaggaccagatcaagagttcggagctgacatcggtccggtgtgtttcctttgataaggttaaaggggcggccgctcaagaggatgtcagaatgccatttgcctgagagatgcaggcttcatttttgatacttttttatttgtaacctatatagtataggattttttttgtcattttgtttcttctcgtacgagcttgctcctgatcagcctatctcgcagcagatgaatatcttgtggtaggggtttgggaaaatcattcgagtttgatgtttttcttggtatttcccactcctcttcagagtacagaagattaagtgaaaccttcgtttgtgcggatccttcagtaatgtcttgtttcttttgttgcagtggtgagccattttgacttcgtgaaagtttctttagaatagttgtttccagaggccaaacattccacccgtagtaaagtgcaagcgtaggaagaccaagactggcataaatcaggtataagtgtcgagcactggcaggtgatcttctgaaagtttctactagcagataagatccagtagtcatgcatatggcaacaatgtaccgtgtggatctaagaacgcgtcctactaaccttcgcattcgttggtccagtttgttgttatcgatcaacgtgacaaggttgtcgattccgcgtaagcatgcatacccaaggacgcctgttgcaattccaagtgagccagttccaacaatctttgtaatattagagcacttcattgtgttgcgcttgaaagtaaaatgcgaacaaattaagagataatctcgaaaccgcgacttcaaacgccaatatgatgtgcggcacacaataagcgttcatatccgctgggtgactttctcgctttaaaaaattatccgaaaaaattttctagagtgttgttactttatacttccggctcgtataatacgacaaggtgtaaggaggactaaaccatggctaaactcacctctgctgttccagtcctgactgctcgtgatgttgctggtgctgttgagttctggactgatagactcggtttctcccgtgacttcgtagaggacgactttgccggtgttgtacgtgacgacgttaccctgttcatctccgcagttcaggaccaggttgtgccagacaacactctggcatgggtatgggttcgtggtctggacgaactgtacgctgagtggtctgaggtcgtgtctaccaacttccgtgatgcatctggtccagctatgaccgagatcggtgaacagccctggggtcgtgagtttgcactgcgtgatccagctggtaactgcgtgcatttcgtcgcagaagaacaggactaacaattgacaccttacgattatttagagagtatttattagttttattgtatgtatacggatgttttattatctatttatgcccttatattctgtaactatccaaaagtcctatcttatcaagccagcaatctatgtccgcgaacgtcaactaaaaataagctttttatgctgttctctctttttttcccttcggtataattataccttgcatccacagattctcctgccaaattttgcataatcctttacaacatggctatatgggagcacttagcgccctccaaaacccatattgcctacgcatgtataggtgttttttccacaatattttctctgtgctctctttttattaaagagaagctctatatcggagaagcttctgtggccgttatattcggccttatcgtgggaccacattgcctgaattggtttgccccggaagattggggaaacttggatctgattaccttagctgcaggtaccactgagcgtcagacc

SEQ ID NO: 13 - DNA, 7356 bp, Artificial Sequence; identical to SEQ ID NO: 9
  MMV129 (Sequence 11)

SEQ ID NO: 14 - DNA, 7879 bp, Artificial Sequence
  MMV130 (Sequence 12)
ggatccttcagtaatgtcttgtttcttttgttgcagtggtgagccattttgacttcgtgaaagtttctttagaatagttgtttccagaggccaaacattccacccgtagtaaagtgcaagcgtaggaagaccaagactggcataaatcaggtataagtgtcgagcactggcaggtgatcttctgaaagtttctactagcagataagatccagtagtcatgcatatggcaacaatgtaccgtgtggatctaagaacgcgtcctactaaccttcgcattcgttggtccagtttgttgttatcgatcaacgtgacaaggttgtcgattccgcgtaagcatgcatacccaaggacgcctgttgcaattccaagtgagccagttccaacaatctttgtaatattagagcacttcattgtgttgcgcttgaaagtaaaatgcgaacaaattaagagataatctcgaaaccgcgacttcaaacgccaatatgatgtgcggcacacaataagcgttcatatccgctgggtgactttctcgctttaaaaaattatccgaaaaaattttctagagtgttgttactttatacttccggctcgtataatacgacaaggtgtaaggaggactaaaccatggctaaactcacctctgctgttccagtcctgactgctcgtgatgttgctggtgctgttgagttctggactgataggctcggtttctcccgtgacttcgtagaggacgactttgccggtgttgtacgtgacgacgttaccctgttcatctccgcagttcaggaccaggttgtgccagacaacactctggcatgggtatgggttcgtggtctggacgaactgtacgctgagtggtctgaggtcgtgtctaccaacttccgtgatgcatctggtccagctatgaccgagatcggtgaacagccctggggtcgtgagtttgcactgcgtgatccagctggtaactgcgtgcatttcgtcgcagaagagcaggactaacaattgacaccttacgattatttagagagtatttattagttttattgtatgtatacggatgttttattatctatttatgcccttatattctgtaactatccaaaagtcctatcttatcaagccagcaatctatgtccgcgaacgtcaactaaaaataagctttttatgctcttctctctttttttcccttcggtataattataccttgcatccacagattctcctgccaaattttgcataatcctttacaacatggctatatgggagcacttagcgccctccaaaacccatattgcctacgcatgtataggtgttttttccacaatattttctctgtgctctctttttattaaagagaagctctatatcggagaagcttctgtggccgttatattcggccttatcgtgggaccacattgcctgaattggtttgccccggaagattggggaaacttggatctgattaccttagctgcagaaaagggtaccactgagcgtcagaccccgtagaaaagatcaaaggatcttcttgagatcctttttttctgcgcgtaatctgctgcttgcaaacaaaaaaaccaccgctaccagcggtggtttgtttgccggatcaagagctaccaactctttttccgaaggtaactggcttcagcagagcgcagataccaaatactgttcttctagtgtagccgtagttaggccaccacttcaagaactctgtagcaccgcctacatacctcgctctgctaatcctgttaccagtggctgctgccagtggcgataagtcgtgtcttaccgggttggacccaagacgatagttaccggataaggcgcagcggtcgggctgaacggggggttcgtgcacacagcccagcttggagcgaacgacctacaccgaactgagatacctacagcgtgagctatgagaaagcgccacgcttcccgaagggagaaaggcggacaggtatccggtaagcggcagggtcggaacaggagagcgcacgagggagcttccagggggaaacgcctggtatctttatagtcctgtcgggtttcgccacctctgacttgagcgtcgatttttgtgatgctcgtcaggggggcggagcctatggaaaaacgccagcaacgcggcctttttacggttcctggccttttgctggccttttgctcacatgtatttcagaagcgatagagagactgcgctaagcattaatgagattatttttgagcattcgtcaatcaataccaaacaagacaaacggtatgccgacttttggaagtttctttttgaccaactggccgttagcatttcaacgaaccaaacttagttcatcttggatgagatcacgcttttgtcatattaggttccaagacagcgtttaaactgtcagttttgggccatttggggaacatgaaactatttgaccccacactcagaaagccctcatctgagtgatgttcgggtgtaatgcggagcttgttgcattcggaaataaacaaacatgaacctcgccaggggggccaggatagacaggctaataaagtcatggtgttagtagcctaatagaaggaattggaataaataatgtatctaaacgcaaactccgagctggaaaaatgttaccggcgatgcgcggacaatttagaggcggcgatcaagaaacacctgctgggcgagcagtctggagcacagtcttcgatgggcccgagatcccaccgcgttcctgggtaccgggacgtgaggcagcgcgacatccatcaaatataccaggcgccaaccgagtctctcggaaaacagcttctggatatcttccgctggcggcgcaacgacgaataatagtccctggaggtgacggaatatatatgtgtggagggtaaatctgacagggtgtagcaaaggtaatattttcctaaaacatgcaatcggctgccccgcaacgggaaaaagaatgactttggcactcttcaccagagtggggtgtcccgctcgtgtgtgcaaataggctcccactggtcaccccggattttgcagaaaaacagcaagttccggggtgtctcactggtgtccgccaataagaggagccggcaggcacggagtctacatcaagctgtctccgatacactcgactaccatccgggtctctcagagaggggaatggcactataaataccgcctccttgcgctctctgccttcatcaatcaaatcatgatgtcttttgtccaaaagggtacttggttactttttgctctgttgcacccaactgttattctcgcacaacaggaagcagtagatggtggttgctcacatttaggtcaatcttacgcagatagagatgtatggaaacctgaaccatgtcaaatttgcgtgtgtgactcaggttcagtgctctgcgacgatatcatatgtgacgaccaggaattggactgtccaaacccagagataccattcggtgaatgttgtgctgtttgtccacagccaccaactgctcctacaagacctccaaacggtcaaggtccacaaggtcctaaaggtgatccgggtccacctggtattcctggtagaaatggtgaccctggacctcccggttccccaggtagcccaggatcacctgggcctcctggaatatgtgaatcctgcccaactggtggtcagaactatagcccacaatacgaggcctacgacgtcaaatctggtgttgctggaggaggtattgcaggctaccctggtcccgcagggcccccaggtccgccgggtccgcccggaacatcaggtcatcccggagcccctggtgcaccaggttatcagggaccgcccggagagcctggacaagctggtcccgctggaccccctggtccaccaggtgctattggaccaagtggtcctgccggaaaagacggtgaatccggtagacctggtagacccggcgaaaggggtttcccaggtcctcccggaatgaagggtccagccggtatgcccggttttcctgggatgaagggtcacagaggatttgatggtagaaacggagagaaaggcgaaaccggtgctcccggactgaagggtgaaaacggtgtccctggtgagaacggcgctcctggacctatgggtccacgtggtgctccaggagaaagaggcagaccaggattgcctggtgcagctggtgctagaggtaacgatggtgcccgtggttccgatggacaacccgggccacccggccctccaggtaccgctggatttcctggaagccctggtgctaagggggaggttggtccggctggtagtcccggaagtagcggtgccccaggtcaaagaggcgaaccaggccctcagggtcacgcaggagcacctggaccgcctggtcctcctggttcgaatggttcgcctggaggaaaaggtgaaatggggcccgcaggaatccccggtgcgcctggtcttattggtgccaggggtcctccaggcccgccaggtacaaatggtgtacccggacagcgaggagcagctggtgaacctggtaaaaacggtgccaaaggagatccaggtcctcgtggagagcgtggtgaagctggctctcccggtatcgccggtccaaaaggtgaggacggtaaggacggttcccctggtgagccaggtgcgaacggactgccaggtgcagccggagagcgaggagtcccaggattcaggggaccagccggtgctaacggcttgcctggtgaaaaagggccccctggtgataggggaggacccggtccagcaggccctcgtggagttgctggtgagcctggacgtgacggtttaccaggagggccaggtttgaggggtattcccgggtcccctggcggtcctggatcggatggaaaaccagggccaccaggttcgcagggtgaaacaggacgtccaggcccacccggctcacctggtccaaggggtcagcctggtgtcatgggtttccccggtccaaagggtaatgacggagcaccgggtaaaaatggtgaacgtggtggcccaggtggtccaggaccccaaggtccagctggaaaaaacggtgagacaggtcctcaaggacctccaggacctaccggtcctagcggagataagggagatacgggaccgccaggacctcaaggattgcaaggtttgcctggtacatctggccctcccggagaaaatggtaagcctggagagccaggaccaaaaggcgaagctggagccccaggtatccccggaggtaagggagactcaggtgctccgggtgagcgtggtcctccgggtgccggtggtccacctggacctagaggtggtgccgggccgccaggtcctgaaggtggtaaaggtgctgctggtccaccgggaccgcctggctctgctggtactcctggcttgcagggaatgccaggagagagaggtggacctggaggtcccggtccgaagggtgataaaggggagccaggatcatccggtgttgacggcgcacctggtaaagacggaccaaggggaccaacgggtccaatcggaccaccaggacccgctggccagccaggagataaaggcgagtccggagcacccggtgttcctggtatagctggacccaggggtggtcccggtgaaagaggtgaacagggcccaccgggtcccgccggtttccctggcgcccctggtcaaaatggagaaccaggtgcaaagggcgagagaggagccccaggagaaaagggtgagggaggaccacccggtgctgccggtccagctgggggttcaggtcctgctggaccaccaggtccacagggcgttaaaggtgagagaggaagtccaggtggtcctggagctgctggattcccaggtggccgtggacctcctggtccccctggatcgaatggtaatcctggtccgccaggtagttcgggtgctcctgggaaggacggtccacctggccccccaggtagtaacggtgcacctggtagtccaggtatatccggacctaaaggagattccggtccaccaggcgaaagaggggccccaggcccacagggtccaccaggagcccccggtcctctgggtattgctggtcttactggtgcacgtggactggccggtccacccggaatgcctggagcaagaggttcacctggaccacaaggtattaaaggagagaacggtaaacctggaccttccggtcaaaacggagagcggggacccccaggcccccaaggtctgccaggactagctggtaccgcaggggaaccaggaagagatggaaatccaggttcagacggactacccggtagagatggtgcaccgggggccaagggcgacaggggtgagaatggatctcctggtgcgccaggggcaccaggccacccaggtcccccaggtcctgtgggccctgctggaaagtcaggtgacaggggagagacaggcccggctggtccatctggcgcacccggaccagctggttccagaggcccacctggtccgcaaggccctagaggtgacaagggagagactggagaacgaggtgctatgggtatcaagggtcatagaggttttccgggtaatcccggcgccccaggttctcctggtccagctggccatcaaggtgcagtcggatcgcccggcccagccggtcccaggggccctgttggtccatccggtcctccaggaaaggatggtgcttctggacacccaggacctatcggacctccgggtcctagaggtaatagaggagaacgtggatccgagggtagtcctggtcaccctggtcaacctggcccaccagggcctccaggtgcacccggtccatgttgtggtgcaggcggtgtggctgcaattgctggtgtgggtgctgaaaaggccggcggtttcgctccatattatggtgatgaaccgattgattttaagatcaatactgacgaaatcatgacttccttaaagtccgttaatggtcaaattgagtctctaatctccccagatggttcacgtaaaaatcctgctagaaattgtagagatttgaagttttgtcaccccgagttgcagtccggtgagtactgggtggaccccaatcaaggttgtaagttagacgctattaaagtttactgcaatatggagacaggagaaacttgcatcagcgcttctccattgactatcccacaaaaaaattggtggactgactctggagctgagaaaaagcatgtatggttcggggaatcgatggaaggtggtttccaattcagctacggtaaccctgaacttcctgaagatgttcttgacgttcaattggcatttctgagattgttgtccagtcgtgcaagccaaaacattacataccattgcaaaaattccatcgcatatatggatcatgctagcggaaatgtgaaaaaggcattgaagctgatgggatcaaatgaaggtgaatttaaagcagagggtaattctaagtttacttacactgtattggaggatggttgtacgaagcatacaggtgaatggggtaaaacagtgtttcaatatcaaacccgcaaagcagttagattgccaatcgtcgatatcgcaccatacgacattggaggaccagatcaagagttcggagctgacatcggtccggtgtgtttcctttgataatcaagaggatgtcagaatgccatttgcctgagagatgcaggcttcatttttgatacttttttatttgtaacctatatagtataggattttttttgtcattttgtttcttctcgtacgagcttgctcctgatcagcctatctcgcagctgatgaatatcttgtggtaggggtttgggaaaatcattcgagtttgatgtttttcttggtatttcccactcctcttcagagtacagaagattaagtgagacgttcgtttgtgctccgga

SEQ ID NO: 15 - DNA, 7963 bp, Artificial Sequence
  MMV78 (Sequence 13)
aattgacaccttacgattatttagagagtatttattagttttattgtatgtatacggatgttttattatctatttatgcccttatattctgtaactatccaaaagtcctatcttatcaagccagcaatctatgtccgcgaacgtcaactaaaaataagctttttatgctgttctctctttttttcccttcggtataattataccttgcatccacagattctcctgccaaattttgcataatcctttacaacatggctatatgggagcacttagcgccctccaaaacccatattgcctacgcatgtataggtgttttttccacaatattttctctgtgctctctttttattaaagagaagctctatatcggagaagcttctgtggccgttatattcggccttatcgtgggaccacattgcctgaattggtttgccccggaagattggggaaacttggatctgattaccttagctgcaggtaccactgagcgtcagaccccgtagaaaagatcaaaggatcttcttgagatcctttttttctgcgcgtaatctgctgcttgcaaacaaaaaaaccaccgctaccagcggtggtttgtttgccggatcaagagctaccaactctttttccgaaggtaactggcttcagcagagcgcagataccaaatactgttcttctagtgtagccgtagttaggccaccacttcaagaactctgtagcaccgcctacatacctcgctctgctaatcctgttaccagtggctgctgccagtggcgataagtcgtgtcttaccgggttggactcaagacgatagttaccggataaggcgcagcggtcgggctgaacggggggttcgtgcacacagcccagcttggagcgaacgacctacaccgaactgagatacctacagcgtgagctatgagaaagcgccacgcttcccgaagggagaaaggcggacaggtatccggtaagcggcagggtcggaacaggagagcgcacgagggagcttccagggggaaacgcctggtatctttatagtcctgtcgggtttcgccacctctgacttgagcgtcgatttttgtgatgctcgtcaggggggcggagcctatggaaaaacgccagcaacgcggcctttttacggttcctggccttttgctggccttttgctcacatgtcgcacaaacgaaggtttcacttaatcttctgtactctgaagaggagtgggaaataccaagaaaaacatcaaactcgaatgattttcccaaacccctaccacaagatattcatctgctgcgagataggctgatcaggagcaagctcgtacgagaagaaacaaaatgacaaaaaaaatcctatactatataggttacaaataaaaaagtatcaaaaatgaagcctgcatctctcaggcaaatggcattctgacatcctcttgaaaattatcattctaattctgacaatgtgcatggcctcctaaactcttgacctctctcatgcagccacttattggaaacccacttattaccgactaagacgggacaagcagcatgtctagtgctgtaatcaccttctccagatgcaaacagattgtaccaaaatacggccgtgccctttttaggccaaacagaagcacctacctcagggaaaactgtggctcctccagcaagcacatcggacatatagaacaaccacgttgcgattctatttccagtacctagctccttaaaagcatcaggctcgtcctttctggcgaaatcaaagtggggttcatactgaccgcccacaccatagttggcaacttgtagttcctcagcagtgcttacgtcaagaccagtcaaatcttgaatacgcatattgatacggctgaccacgggattctcgtaaccggacaaccatgctgatttagagacacgatattgtgcggtagtcaattttccagtctcagggtcatggacggtagccctactcaatcttggtttggccaagtctttcacaacctctatttctgcatcggagatgatgtcatgaaaacgaatgattctaggcttgtcccattcatcttcctgtttcgctggagcaagaatgaattttgggttacggttcccatcatgatatctacagaacagctttttctgtctccttggagtcatcttgataccctctcctctacacagcatttcatacttttgtctctctgggaggtagtcaacagctgcacctttttttttcagagtggtcttttgatcggattggtcatcggacgaggacttatttgcgtccttttccttagccatgatgtattcaaagtatttcagattaccgttagctctttgatgctccgggtccagctccaacaactttttagttaaaagtagagctttgtccagatcaccttgctggtaaacagcgtatgataagtaatccaaaactgaaaccttatcaacggtagaaacttcaccttcgtccaactgacgcagagcttgctccatccataattctgtgtgatagtagtcggcttctgtatatgcgacttttcccaattcaaaacaatcttccacagtgaggaaggacttatgcttcacaccaggtaaatcacccttcgatatcgtgtcggtgtccaaattgtatgtgtcctgcaatcgcaacaaagcttttgctgctcctacttggtcctcatcgtttggaaagtattgtctttgaattgttaagttagaaatgaatccatcactcatatctttaagtaccaagttttccaattctgaccactctgtattaagtctcttcatcagcttgaaagcattcactgggtgacccacaaaaccctcaggatcttttgttgcagtactagtcaatctatcgagtttctctgcccactttttgatttgctccaacttatcctcttcagctttgatatagtctttaaggcttgtaactaggtctttttctgtgtgaatcaaatcagtcatctgtcctatagaagtgaagaagcctgggtgagccagtgactgtggcaacaaaataccaacgactaggatataccaaatcatttttgatgtttgatagtttgataagagtgaactttagtgtttagaggggttataatttgttgtaactggttttggtcttaagttaaaacgaacttgttatattaaacacaacggtcactcaggatacaagaataggaaagaaaaactttaaactggggacatgttgtctttatataatttggcggttaacccttaatgcccgtttccgtctcttcatgataacaaagctgcccatctatgactgaatgtggagaagtatcggaacaacccttcactaaggatatctaggctaaactcattcgcgccttagatttctccaaggtatcggttaagtttcctctttcgtactggctaacgatggtgttgctcaacaaagggatggaacggcagctaaagggagtgcatggaatgactttaattggctgagaaagtgttctatttgtccgaatttcttttttctattatctgttcgtttgggcggatctctccagtggggggtaaatggaagatttctgttcatggggtaaggaagctgaaatccttcgtttcttataggggcaagtatactaaatctcggaacattgaatggggtttactttcattggctacagaaattattaagtttgttatggggtgaagttaccagtaattttcattttttcacttcaacttttggggtatttctgtggggtagcatagagcaatgatataaacaacaattgagtgacaggtctactttgttctcaaaaggccataaccatctgtttgcatctcttatcaccacaccatcctcctcatctggccttcaattgtggggaacaactagcatcccaacaccagactaactccacccagatgaaaccagttgtcgcttaccagtcaatgaatgttgagctaacgttccttgaaactcgaatgatcccagccttgctgcgtatcatccctccgctattccgccgcttgctccaaccatgtttccgcctttttcgaacaagttcaaatacctatctttggcaggacttttcctcctgccttttttagcctcagctctcggttagcctctaggcaaattctggtcttcatacctatatcaacttttcatcagatagcctttgggttcaaaaaagaactaaagcaggatgcctgatatataaatcccagatgatctgcttttgaaactattttcagtatcttgattcgtttacttacaaacaactattgttgattttatctggagaataatcgaacaaaatgagattcccatctattttcaccgctgtcttgttcgctgcctcctctgcattggctgcccctgttaacactaccactgaagacgagactgctcaaattccagctgaagcagttatcggttactctgaccttgagggtgatttcgacgtcgctgttttgcctttctctaactccactaacaacggtttgttgttcattaacaccactatcgcttccattgctgctaaggaagagggtgtctctctcgagaaaagagaggccgaagctgcacccgatgaggaagatcatgttttagtattgcataaaggaaatttcgatgaagctttggccgctcacaaatatctgctcgtcgagttttacgctccctggtgcggtcattgtaaggcccttgcaccagagtacgccaaggcagctggtaagttaaaggccgaaggttcagagatcagattagcaaaagttgatgctacagaagagtccgatcttgctcaacaatacggggttcgaggatacccaacaattaagtttttcaaaaatggtgatactgcttccccaaaggaatatactgctggtagagaggcagacgacatagtcaactggctcaaaaagagaacgggcccagctgcgtctacattaagcgacggagcagcagccgaagctcttgtggaatctagtgaagttgctgtaatcggtttctttaaggacatggaatctgattcagctaaacagttccttttagcagctgaagcaatcgatgacatccctttcggaatcacctcaaatagtgacgtgttcagcaagtaccaacttgacaaagatggagtggtcttgttcaaaaagtttgacgaaggcagaaacaatttcgagggtgaggttacaaaggagaaactgcttgatttcattaaacataaccaactacccttagttatcgaattcactgaacaaactgctcctaagattttcggtggagaaatcaaaacacatatcttgttgtttttgccaaagtccgtatcggattatgaaggtaaactctccaatttcaaaaaggccgctgagagctttaagggcaagattttgttcatctttattgactcagaccacacagacaatcagaggattttggagtttttcggtttgaaaaaggaggaatgtccagcagtccgtttgatcaccttggaggaggagatgaccaaatacaaaccagagtcggatgagttgactgccgagaagataacagaattttgtcacagatttctggaaggtaagatcaagcctcatcttatgtctcaagagttgcctgatgactgggataagcaaccagttaaagtattggtgggtaaaaactttgaggaagtggccttcgacgagaaaaaaaatgtctttgttgaattctatgctccgtggtgtggtcactgtaagcagctggcaccaatttgggataaactgggtgaaacttacaaagatcacgaaaacattgttattgcaaagatggacagtactgctaacgaagtggaggctgtgaaagttcactccttccctacgctgaagttctttcctgcatctgctgacagaactgttatcgactataatggagagaggacattggatggttttaaaaagtttcttgaatccggaggtcaagacggagctggtgacgacgatgatttggaagatctggaggaggctgaggaacctgatcttgaggaggatgacgaccagaaggcagtcaaagatgaactgtgataaggggcggccgctcaagaggatgtcagaatgccatttgcctgagagatgcaggcttcatttttgatacttttttatttgtaacctatatagtataggattttttttgtcattttgtttcttctcgtacgagcttgctcctgatcagcctatctcgcagcagatgaatatcttgtggtaggggtttgggaaaatcattcgagtttgatgtttttcttggtatttcccactcctcttcagagtacagaagattaagtgaaaccttcgtttgtgcggatccttcagtaatgtcttgtttcttttgttgcagtggtgagccattttgacttcgtgaaagtttctttagaatagttgtttccagaggccaaacattccacccgtagtaaagtgcaagcgtaggaagaccaagactggcataaatcaggtataagtgtcgagcactggcaggtgatcttctgaaagtttctactagcagataagatccagtagtcatgcatatggcaacaatgtaccgtgtggatctaagaacgcgtcctactaaccttcgcattcgttggtccagtttgttgttatcgatcaacgtgacaaggttgtcgattccgcgtaagcatgcatacccaaggacgcctgttgcaattccaagtgagccagttccaacaatctttgtaatattagagcacttcattgtgttgcgcttgaaagtaaaatgcgaacaaattaagagataatctcgaaaccgcgacttcaaacgccaatatgatgtgcggcacacaataagcgttcatatccgctgggtgactttctcgctttaaaaaattatccgaaaaaattttctagagtgttgacactttatacttccggctcgtataatacgacaaggtgtaaggaggactaaaccatgaaaaagccagagcttacagcaacgagcgttgagaaattcttgattgaaaagtttgattcagtttccgacctgatgcagttgtctgagggtgaagagtcaagagccttttcgttcgatgtgggtggtagaggttacgtccttagggtgaactcttgtgccgatggtttttacaaagatagatatgtttacagacatttcgcatccgcagcactccccatcccagaagtattggacattggagagttttccgaatccttgacctattgcatctctcgacgtgcccaaggtgtcactttacaagacttgccggagactgaacttccagcagttttacaacctgtagcagaggctatggacgctattgctgctgctgatttgtctcaaacaagtggattcggcccttttggtcctcagggtatcgggcaatacacaacttggagagactttatctgtgctatcgcagacccacatgtgtatcactggcaaaccgtcatggatgacactgtatcggctagtgtggcccaagctcttgatgagctaatgctgtgggctgaggactgtccagaagtgaggcacttggttcacgcagactttggatccaataatgttctgacagataacggacgtataacagctgtcattgactggtccgaagctatgttcggtgattcacaatatgaagtcgctaacatattcttttggcgtccctggttagcatgtatggagcaacaaactagatatttcgaacgtagacatcctgaactagctggatctccaagattgagagcttacatgctgaggatcggtttggatcagctgtaccagagcttggtagacggaaatttcgacgacgccgcatgggcgcaaggtagatgcgatgccattgtgagaagtggtgctggcactgttggtagaacccagattgcaagacgttcagctgctgtttggacggatggttgtgttgaggttttggcagattccggaaatcgtagacctagcactaggccaagagctaaggaataatagc

SEQ ID NO: 16 - DNA, 5508 bp, Artificial Sequence
  MMV94 (Sequence 14)
aacatccaaagacgaaaggttgaatgaaacctttttgccatccgacatccacaggtccattctcacacataagtgccaaacgcaacaggaggggatacactagcagcagaccgttgcaaacgcaggacctccactcctcttctcctcaacacccacttttgccatcgaaaaaccagcccagttattgggcttgattggagctcgctcattccaattccttctattaggctactaacaccatgactttattagcctgtctatcctggcccccctggcgaggttcatgtttgtttatttccgaatgcaacaagctccgcattacacccgaacatcactccagatgagggctttctgagtgtggggtcaaatagtttcatgttccccaaatggcccaaaactgacagtttaaacgctgtcttggaacctaatatgacaaaagcgtgatctcatccaagatgaactaagtttggttcgttgaaatgctaacggccagttggtcaaaaagaaacttccaaaagtcggcataccgtttgtcttgtttggtattgattgacgaatgctcaaaaataatctcattaatgcttagcgcagtctctctatcgcttctgaaccccggtgcacctgtgccgaaacgcaaatggggaaacacccgctttttggatgattatgcattgtctccacattgtatgcttccaagattctggtgggaatactgctgatagcctaacgttcatgatcaaaatttaactgttctaacccctacttgacagcaatatataaacagaaggaagctgccctgtcttaaacctttttttttatcatcattattagcttactttcataattgcgactggttccaattgacaagcttttgattttaacgacttttaacgacaacttgagaagatcaaaaaacaactaattattgaaagaattcatgttctctccaattttgtccttggaaattattttagctttggctactttgcaatctgtcttcgctgcccccgacgaggaggaccacgtcctggtgctccataagggcaacttcgacgaggcgctggcggcccacaagtacctgctggtggagttctacgccccatggtgcggccactgcaaggctctggccccggagtatgccaaagcagctgggaagctgaaggcagaaggttctgagatcagactggccaaggtggatgccactgaagagtctgacctggcccagcagtatggtgtccgaggctaccccaccatcaagttcttcaagaatggagacacagcttcccccaaagagtacacagctggccgagaagcggatgatatcgtgaactggctgaagaagcgcacgggccccgctgccagcacgctgtccgacggggctgctgcagaggccttggtggagtccagtgaggtggccgtcattggcttcttcaaggacatggagtcggactccgcaaagcagttcttgttggcagcagaggccattgatgacatccccttcgggatcacatctaacagcgatgtgttctccaaataccagctggacaaggatggggttgtcctctttaagaagtttgacgaaggccggaacaactttgagggggaggtcaccaaagaaaagcttctggacttcatcaagcacaaccagttgcccctggtcattgagttcaccgagcagacagccccgaagatcttcggaggggaaatcaagactcacatcctgctgttcctgccgaaaagcgtgtctgactatgagggcaagctgagcaacttcaaaaaagcggctgagagcttcaagggcaagatcctgtttatcttcatcgacagcgaccacactgacaaccagcgcatcctggaattcttcggcctaaagaaagaggagtgcccggccgtgcgcctcatcacgctggaggaggagatgaccaaatataagccagagtcagatgagctgacggcagagaagatcaccgagttctgccaccgcttcctggagggcaagattaagccccacctgatgagccaggagctgcctgacgactgggacaagcagcctgtcaaagtgctggttgggaagaactttgaagaggttgcttttgatgagaaaaagaacgtctttgtagagttctatgccccgtggtgcggtcactgcaagcagctggcccccatctgggataagctgggagagacgtacaaggaccacgagaacatagtcatcgccaagatggactccacggccaacgaggtggaggcggtgaaagtgcacagcttccccacgctcaagttcttccccgccagcgccgacaggacggtcatcgactacaatggggagcggacactggatggttttaagaagttcctggagagtggtggccaggatggggccggagatgatgacgatctagaagatcttgaagaagcagaagagcctgatctggaggaagatgatgatcaaaaagctgtgaaagatgaactgtaagcggccgctcaagaggatgtcagaatgccatttgcctgagagatgcaggcttcatttttgatacttttttatttgtaacctatatagtataggattttttttgtcattttgtttcttctcgtacgagcttgctcctgatcagcctatctcgcagcagatgaatatcttgtggtaggggtttgggaaaatcattcgagtttgatgtttttcttggtatttcccactcctcttcagagtacagaagattaagtgaaaccttcgtttgtgcggatccttcagtaatgtcttgtttcttttgttgcagtggtgagccattttgacttcgtgaaagtttctttagaatagttgtttccagaggccaaacattccacccgtagtaaagtgcaagcgtaggaagaccaagactggcataaatcaggtataagtgtcgagcactggcaggtgatcttctgaaagtttctactagcagataagatccagtagtcatgcatatggcaacaatgtaccgtgtggatctaagaacgcgtcctactaaccttcgcattcgttggtccagtttgttgttatcgatcaacgtgacaaggttgtcgattccgcgtaagcatgcatacccaaggacgcctgttgcaattccaagtgagccagttccaacaatctttgtaatattagagcacttcattgtgttgcgcttgaaagtaaaatgcgaacaaattaagagataatctcgaaaccgcgacttcaaacgccaatatgatgtgcggcacacaataagcgttcatatccgctgggtgactttctcgctttaaaaaattatccgaaaaaattttctagagtgttgacactttatacttccggctcgtataatacgacaaggtgtaaggaggactaaaccatgggtaaggaaaagactcacgtttcgaggccgcgattaaattccaacatggatgctgatttatatgggtataaatgggctcgcgataatgtcgggcaatcaggtgcgacaatctatcgattgtatgggaagcccgatgcgccagagttgtttctgaaacatggcaaaggtagcgttgccaatgatgttacagatgagatggtcagactaaactggctgacggaatttatgcctcttccgaccatcaagcattttatccgtactcctgatgatgcatggttactcaccactgcgatccccggcaaaacagcattccaggtattagaagaatatcctgattcaggtgaaaatattgttgatgcgctggcagtgttcctgcgccggttgcattcgattcctgtttgtaattgtccttttaacagcgatcgcgtatttcgtctcgctcaggcgcaatcacgaatgaataacggtttggttgatgcgagtgattttgatgacgagcgtaatggctggcctgttgaacaagtctggaaagaaatgcataagcttttgccattctcaccggattcagtcgtcactcatggtgatttctcacttgataaccttatttttgacgaggggaaattaataggttgtattgatgttggacgagtcggaatcgcagaccgataccaggatcttgccatcctatggaactgcctcggtgagttttctccttcattacagaaacggctttttcaaaaatatggtattgataatcctgatatgaataaattgcagtttcatttgatgctcgatgagtttttctaacaattgacaccttacgattatttagagagtatttattagttttattgtatgtatacggatgttttattatctatttatgcccttatattctgtaactatccaaaagtcctatcttatcaagccagcaatctatgtccgcgaacgtcaactaaaaataagctttttatgctgttctctctttttttcccttcggtataattataccttgcatccacagattctcctgccaaattttgcataatcctttacaacatggctatatgggagcacttagcgccctccaaaacccatattgcctacgcatgtataggtgttttttccacaatattttctctgtgctctctttttattaaagagaagctctatatcggagaagcttctgtggccgttatattcggccttatcgtgggaccacattgcctgaattggtttgccccggaagattggggaaacttggatctgattaccttagctgcaggtaccactgagcgtcagaccccgtagaaaagatcaaaggatcttcttgagatcctttttttctgcgcgtaatctgctgcttgcaaacaaaaaaaccaccgctaccagcggtggtttgtttgccggatcaagagctaccaactctttttccgaaggtaactggcttcagcagagcgcagataccaaatactgttcttctagtgtagccgtagttaggccaccacttcaagaactctgtagcaccgcctacatacctcgctctgctaatcctgttaccagtggctgctgccagtggcgataagtcgtgtcttaccgggttggactcaagacgatagttaccggataaggcgcagcggtcgggctgaacggggggttcgtgcacacagcccagcttggagcgaacgacctacaccgaactgagatacctacagcgtgagctatgagaaagcgccacgcttcccgaagggagaaaggcggacaggtatccggtaagcggcagggtcggaacaggagagcgcacgagggagcttccagggggaaacgcctggtatctttatagtcctgtcgggtttcgccacctctgacttgagcgtcgatttttgtgatgctcgtcaggggggcggagcctatggaaaaacgccagcaacgcggcctttttacggttcctggccttttgctggccttttgctcacatgttctttcctgcggtacccagatccaattcccgctttgactgcctgaaatctccatcgcctacaatgatgacatttggatttggttgactcatgttggtattgtgaaatagacgcagatcgggaacactgaaaaatacacagttattattcatttaaat

SEQ ID NO: 17 - DNA, 7605 bp, Artificial Sequence
  MMV156 (Sequence 15)
tgcaggtaccactgagcgtcagaccccgtagaaaagatcaaaggatcttcttgagatcctttttttctgcgcgtaatctgctgcttgcaaacaaaaaaaccaccgctaccagcggtggtttgtttgccggatcaagagctaccaactctttttccgaaggtaactggcttcagcagagcgcagataccaaatactgttcttctagtgtagccgtagttaggccaccacttcaagaactctgtagcaccgcctacatacctcgctctgctaatcctgttaccagtggctgctgccagtggcgataagtcgtgtcttaccgggttggactcaagacgatagttaccggataaggcgcagcggtcgggctgaacggggggttcgtgcacacagcccagcttggagcgaacgacctacaccgaactgagatacctacagcgtgagctatgagaaagcgccacgcttcccgaagggagaaaggcggacaggtatccggtaagcggcagggtcggaacaggagagcgcacgagggagcttccagggggaaacgcctggtatctttatagtcctgtcgggtttcgccacctctgacttgagcgtcgatttttgtgatgctcgtcaggggggcggagcctatggaaaaacgccagcaacgcggcctttttacggttcctggccttttgctggccttttgctcacatgttctttcctgcggtacccagatccaattcccgctttgactgcctgaaatctccatcgcctacaatgatgacatttggatttggttgactcatgttggtattgtgaaatagacgcagatcgggaacactgaaaaatacacagttattattcatttcagaagcgatagagagactgcgctaagcattaatgagattatttttgagcattcgtcaatcaataccaaacaagacaaacggtatgccgacttttggaagtttctttttgaccaactggccgttagcatttcaacgaaccaaacttagttcatcttggatgagatcacgcttttgtcatattaggttccaagacagcgtttaaactgtcagttttgggccatttggggaacatgaaactatttgaccccacactcagaaagccctcatctggagtgatgttcgggtgtaatgcggagcttgttgcattcggaaataaacaaacatgaacctcgccaggggggccaggatagacaggctaataaagtcatggtgttagtagcctaatagaaggaattggaataaatgacccttgtgactgacactttgggagtccctattctacttagtctcatatcgcatgaaacttttgataaattattttctgataggaatttttcatcagatattatcatcgcggcttacgtaataacaaaaaaaattgatggagtctatactaggctaacataaactaagttattaattaaacaaaacaaaacgtactagcattactgtcatatataagggctcctaactaaaactgtaaagacttcccgtaaaattatcattctaattctgacaatgtgcatggcctcctaaactcttgacctctctcatgcagccacttattggaaacccacttattaccgactaagacgggacaagcagcatgtctagtgctgtaatcaccttctccagatgcaaacagattgtaccaaaatacggccgtgccctttttaggccaaacagaagcacctacctcagggaaaactgtggctcctccagcaagcacatcggacatatagaacaaccacgttgcgattctatttccagtacctagctccttaaaagcatcaggctcgtcctttctggcgaaatcaaagtggggttcatactgaccgcccacaccatagttggcaacttgtagttcctcagcagtgcttacgtcaagaccagtcaaatcttgaatacgcatattgatacggctgaccacgggattctcgtaaccggacaaccatgctgatttagagacacgatattgtgcggtagtcaattttccagtctcagggtcatggacggtagccctactcaatcttggtttggccaagtctttcacaacctctatttctgcatcggagatgatgtcatgaaaacgaatgattctaggcttgtcccattcatcttcctgtttcgctggagcaagaatgaattttgggttacggttcccatcatgatatctacagaacagctttttctgtctccttggagtcatcttgataccctctcctctacacagcatttcatacttttgtctctctgggaggtagtcaacagctgcacctttttttttcagagtggtcttttgatcggattggtcatcggacgaggacttatttgcgtccttttccttagccatgatgtattcaaagtatttcagattaccgttagctctttgatgctccgggtccagctccaacaactttttagttaaaagtagagctttgtccagatcaccttgctggtaaacagcgtatgataagtaatccaaaactgaaaccttatcaacggtagaaacttcaccttcgtccaactgacgcagagcttgctccatccataattctgtgtgatagtagtcggcttctgtatatgcgacttttcccaattcaaaacaatcttccacagtgaggaaggacttatgcttcacaccaggtaaatcacccttcgatatcgtgtcggtgtccaaattgtatgtgtcctgcaatcgcaacaaagcttttgctgctcctacttggtcctcatcgtttggaaagtattgtctttgaattgttaagttagaaatgaatccatcactcatatctttaagtaccaagttttccaattctgaccactctgtattaagtctcttcatcagcttgaaagcattcactgggtgacccacaaaaccctcaggatcttttgttgcagtactagtcaatctatcgagtttctctgcccactttttgatttgctccaacttatcctcttcagctttgatatagtctttaaggcttgtaactaggtctttttctgtgtgaatcaaatcagtcatctgtcctatagaagtgaagaagcctgggtgagccagtgactgtggcaacaaaataccaacgactaggatataccaaatcatgcggcctgttgtagttttaatatagtttgagtatgagatggaactcagaacgaaggaattatcaccagtttatatattctgaggaaagggtgtgtcctaaattggacagtcacgatggcaataaacgctcagccaatcagaatgcaggagccataaattgttgtattattgctgcaagatttatgtgggttcacattccactgaatggttttcactgtagaattggtgtcctagttgttatgtttcgagatgttttcaagaaaaactaaaatgcacaaactgaccaataatgtgccgtcgcgcttggtacaaacgtcaggattgccaccacttttttcgcactctggtacaaaagttcgcacttcccactcgtatgtaacgaaaaacagagcagtctatccagaacgagacaaattagcgcgtactgtcccattccataaggtatcataggaaacgagagtcctccccccatcacgtatatataaacacactgatatcccacatccgcttgtcaccaaactaatacatccagttcaagttacctaaacaaatcaaagcatgagattcccatctattttcaccgctgtcttgttcgctgcctcctctgcattggctgcacccgatgaggaagatcatgttttagtattgcataaaggaaatttcgatgaagctttggccgctcacaaatatctgctcgtcgagttttacgctccctggtgcggtcattgtaaggcccttgcaccagagtacgccaaggcagctggtaagttaaaggccgaaggttcagagatcagattagcaaaagttgatgctacagaagagtccgatcttgctcaacaatacggggttcgaggatacccaacaattaagtttttcaaaaatggtgatactgcttccccaaaggaatatactgctggtagagaggcagacgacatagtcaactggctcaaaaagagaacgggcccagctgcgtctacattaagcgacggagcagcagccgaagctcttgtggaatctagtgaagttgctgtaatcggtttctttaaggacatggaatctgattcagctaaacagttccttttagcagctgaagcaatcgatgacatccctttcggaatcacctcaaatagtgacgtgttcagcaagtaccaacttgacaaagatggagtggtcttgttcaaaaagtttgacgaaggcagaaacaatttcgagggtgaggttacaaaggagaaactgcttgatttcattaaacataaccaactacccttagttatcgaattcactgaacaaactgctcctaagattttcggtggagaaatcaaaacacatatcttgttgtttttgccaaagtccgtatcggattatgaaggtaaactctccaatttcaaaaaggccgctgagagctttaagggcaagattttgttcatctttattgactcagaccacacagacaatcagaggattttggagtttttcggtttgaaaaaggaggaatgtccagcagtccgtttgatcaccttggaggaggagatgaccaaatacaaaccagagtcggatgagttgactgccgagaagataacagaattttgtcacagatttctggaaggtaagatcaagcctcatcttatgtctcaagagttgcctgatgactgggataagcaaccagttaaagtattggtgggtaaaaactttgaggaagtggccttcgacgagaaaaaaaatgtctttgttgaattctatgctccgtggtgtggtcactgtaagcagctggcaccaatttgggataaactgggtgaaacttacaaagatcacgaaaacattgttattgcaaagatggacagtactgctaacgaagtggaggctgtgaaagttcactccttccctacgctgaagttctttcctgcatctgctgacagaactgttatcgactataatggagagaggacattggatggttttaaaaagtttcttgaatccggaggtcaagacggagctggtgacgacgatgatttggaagatctggaggaggctgaggaacctgatcttgaggaggatgacgaccagaaggcagtcaaagatgaactgtgataaggggtcaagaggatgtcagaatgccatttgcctgagagatgcaggcttcatttttgatacttttttatttgtaacctatatagtataggattttttttgtcattttgtttcttctcgtacgagcttgctcctgatcagcctatctcgcagcagatgaatatcttgtggtaggggtttgggaaaatcattcgagtttgatgtttttcttggtatttcccactcctcttcagagtacagaagattaagtgagaccttcgtttgtgcggatccttcagtaatgtcttgtttcttttgttgcagtggtgagccattttgacttcgtgaaagtttctttagaatagttgtttccagaggccaaacattccacccgtagtaaagtgcaagcgtaggaagaccaagactggcataaatcaggtataagtgtcgagcactggcaggtgatcttctgaaagtttctactagcagataagatccagtagtcatgcatatggcaacaatgtaccgtgtggatctaagaacgcgtcctactaaccttcgcattcgttggtccagtttgttgttatcgatcaacgtgacaaggttgtcgattccgcgtaagcatgcatacccaaggacgcctgttgcaattccaagtgagccagttccaacaatctttgtaatattagagcacttcattgtgttgcgcttgaaagtaaaatgcgaacaaattaagagataatctcgaaaccgcgacttcaaacgccaatatgatgtgcggcacacaataagcgttcatatccgctgggtgactttctcgctttaaaaaattatccgaaaaaattttctagagtgttgacactttatacttccggctcgtataatacgacaaggtgtaaggaggactaaaccatgggtaaaaagcctgaactcaccgcgacgtctgtcgagaagtttctgatcgaaaagttcgacagcgtctccgacctgatgcagctctcggagggcgaagaatctcgtgctttcagcttcgatgtaggagggcgtggatatgtcctgcgggtaaatagctgcgccgatggtttctacaaagatcgttatgtttatcggcactttgcatcggccgcgctcccgattccggaagtgcttgacattggggaattcagcgagagcctgacctattgcatctcccgccgtgcacagggtgtcacgttgcaagacctgcctgaaaccgaactgcccgctgttctgcagccggtcgcggaggccatggatgcgatcgctgcggccgatcttagccagacgagcgggttcggcccattcggaccgcaaggaatcggtcaatacactacatggcgtgatttcatatgcgcgattgctgatccccatgtgtatcactggcaaactgtgatggacgacaccgtcagtgcgtccgtcgcgcaggctctcgatgagctgatgctttgggccgaggactgccccgaagtccggcacctcgtgcacgcggatttcggctccaacaatgtcctgacggacaatggccgcataacagcggtcattgactggagcgaggcgatgttcggggattcccaatacgaggtcgccaacatcttcttctggaggccgtggttggcttgtatggagcagcagacgcgctacttcgagcggaggcatccggagcttgcaggatcgccgcggctccgggcgtatatgctccgcattggtcttgaccaactctatcagagcttggttgacggcaatttcgatgatgcagcttgggcgcagggtcgatgcgacgcaatcgtccgatccggagccgggactgtcgggcgtacacaaatcgcccgcagaagcgcggccgtctggaccgatggctgtgtagaagtactcgccgatagtggaaaccgacgccccagcactcgtccgagggcaaaggaataacaattgacaccttacgattatttagagagtatttattagttttattgtatgtatacggatgttttattatctatttatgcccttatattctgtaactatccaaaagtcctatcttatcaagccagcaatctatgtccgcgaacgtcaactaaaaataagctttttatgctcttctctctttttttcccttcggtataattataccttgcatccacagattctcctgccaaattttgcataatcctttacaacatggctatatgggagcacttagcgccctccaaaacccatattgcctacgcatgtataggtgttttttccacaatattttctctgtgctctctttttattaaagagaagctctatatcggagaagcttctgtggccgttatattcggccttatcgtgggaccacattgcctgaattggtttgccccggaagattggggaaacttggatctgattaccttagctgca

SEQ ID NO: 18 - DNA, 8743 bp, Artificial Sequence
  MMV191 (Sequence 16)
ggatccttcagtaatgtcttgtttcttttgttgcagtggtgagccattttgacttcgtgaaagtttctttagaatagttgtttccagaggccaaacattccacccgtagtaaagtgcaagcgtaggaagaccaagactggcataaatcaggtataagtgtcgagcactggcaggtgatcttctgaaagtttctactagcagataagatccagtagtcatgcatatggcaacaatgtaccgtgtggatctaagaacgcgtcctactaaccttcgcattcgttggtccagtttgttgttatcgatcaacgtgacaaggttgtcgattccgcgtaagcatgcatacccaaggacgcctgttgcaattccaagtgagccagttccaacaatctttgtaatattagagcacttcattgtgttgcgcttgaaagtaaaatgcgaacaaattaagagataatctcgaaaccgcgacttcaaacgccaatatgatgtgcggcacacaataagcgttcatatccgctgggtgactttctcgctttaaaaaattatccgaaaaaattttctagacttctcttccaaatatcgtctccacaaaatgggtaaggaaaagactcacgtttcgaggccgcgattaaattccaacatggatgctgatttatatgggtataaatgggctcgcgataatgtcgggcaatcaggtgcgacaatctatcgattgtatgggaagcccgatgcgccagagttgtttctgaaacatggcaaaggtagcgttgccaatgatgttacagatgagatggtcagactaaactggctgacggaatttatgcctcttccgaccatcaagcattttatccgtactcctgatgatgcatggttactcaccactgcgatccccggcaaaacagcattccaggtattagaagaatatcctgattcaggtgaaaatattgttgatgcgctggcagtgttcctgcgccggttgcattcgattcctgtttgtaattgtccttttaacagcgatcgcgtatttcgtctcgctcaggcgcaatcacgaatgaataacggtttggttgatgcgagtgattttgatgacgagcgtaatggctggcctgttgaacaagtctggaaagaaatgcataagcttttgccattctcaccggattcagtcgtcactcatggtgatttctcacttgataaccttatttttgacgaggggaaattaataggttgtattgatgttggacgagtcggaatcgcagaccgataccaggatcttgccatcctatggaactgcctcggtgagttttctccttcattacagaaacggctttttcaaaaatatggtattgataatcctgatatgaataaattgcagtttcatttgatgctcgatgagtttttctaaaattgacaccttacgattatttagagagtatttattagttttattgtatgtatacggatgttttattatctatttatgcccttatattctgtaactatccaaaagtcctatcttatcaagccagcaatctatgtccgcgaacgtcaactaaaaataagctttttatgctgttctctctttttttcccttcggtataattataccttgcatccacagattctcctgccaaattttgcataatcctttacaacatggctatatgggagcacttagcgccctccaaaacccatattgcctacgcatgtataggtgttttttccacaatattttctctgtgctctctttttattaaagagaagctctatatcggagaagcttctgtggccgttatattcggccttatcgtgggaccacattgcctgaattggtttgccccggaagattggggaaacttggatctgattaccttagctgcatcagaattggttaattggttgtaacactgacccctatttgtttatttttctaaatacattcaaatatgtatccgctcatgagacaataaccctgataaatgcttcaataatattgaaaaaggaagaatatgagtattcaacatttccgtgtcgcccttattcccttttttgcggcattttgccttcctgtttttgctcacccagaaacgctggtgaaagtaaaagatgctgaagatcagttgggtgcacgagtgggttacatcgaactggatctcaacagcggtaagatccttgagagttttcgccccgaagaacgttttccaatgatgagcacttttaaagttctgctatgtggcgcggtattatcccgtattgacgccgggcaagagcaactcggtcgccgcatacactattctcagaatgacttggttgagtactcaccagtcacagaaaagcatcttacggatggcatgacagtaagagaattatgcagtgctgccataaccatgagtgataacactgcggccaacttacttctgacaacgatcggaggaccgaaggagctaaccgcttttttgcacaacatgggggatcatgtaactcgccttgatcgttgggaaccggagctgaatgaagccataccaaacgacgagcgtgacaccacgatgcctgtagcgatggcaacaacgttgcgcaaactattaactggcgaactacttactctagcttcccggcaacaattaatagactggatggaggcggataaagttgcaggaccacttctgcgctcggcccttccggctggctggtttattgctgataaatccggagccggtgagcgtggttctcgcggtatcatcgcagcgctggggccagatggtaagccctcccgtatcgtagttatctacacgacggggagtcaggcaactatggatgaacgaaatagacagatcgctgagataggtgcctcactgattaagcattggtaaggtaccactgagcgtcagaccccgtagaaaagatcaaaggatcttcttgagatcctttttttctgcgcgtaatctgctgcttgcaaacaaaaaaaccaccgctaccagcggtggtttgtttgccggatcaagagctaccaactctttttccgaaggtaactggcttcagcagagcgcagataccaaatactgttcttctagtgtagccgtagttaggccaccacttcaagaactctgtagcaccgcctacatacctcgctctgctaatcctgttaccagtggctgctgccagtggcgataagtcgtgtcttaccgggttggactcaagacgatagttaccggataaggcgcagcggtcgggctgaacggggggttcgtgcacacagcccagcttggagcgaacgacctacaccgaactgagatacctacagcgtgagctatgagaaagcgccacgcttcccgaagggagaaaggcggacaggtatccggtaagcggcagggtcggaacaggagagcgcacgagggagcttccagggggaaacgcctggtatctttatagtcctgtcgggtttcgccacctctgacttgagcgtcgatttttgtgatgctcgtcaggggggcggagcctatggaaaaacgccagcaacgcggcctttttacggttcctggccttttgctggccttttgctcacaatttaaatgacccttgtgactgacactttgggagtccctattctacttagtctcatatcgcatgaaacttttgataaattattttctgataggaatttttcatcagatattatcatcgcggcttacgtaataacaaaaaaaattgatggagtctatactaggctaacataaactaagttattaattaaacaaaacaaaacgtactagcattactgtcatatataagggctcctaactaaaactgtaaagacttcccgtaaaattatcattctaattctgacaatgtgcatggcctcctaaactcttgacctctctcatgcagccacttattggaaacccacttattaccgactaagacgggacaagcagcatgtctagtgctgtaatcaccttctccagatgcaaacagattgtaccaaaatacggccgtgccctttttaggccaaacagaagcacctacctcagggaaaactgtggctcctccagcaagcacatcggacatatagaacaaccacgttgcgattctatttccagtacctagctccttaaaagcatcaggctcgtcctttctggcgaaatcaaagtggggttcatactgaccgcccacaccatagttggcaacttgtagttcctcagcagtgcttacgtcaagaccagtcaaatcttgaatacgcatattgatacggctgaccacgggattctcgtaaccggacaaccatgctgatttagagacacgatattgtgcggtagtcaattttccagtctcagggtcatggacggtagccctactcaatcttggtttggccaagtctttcacaacctctatttctgcatcggagatgatgtcatgaaaacgaatgattctaggcttgtcccattcatcttcctgtttcgctggagcaagaatgaattttgggttacggttcccatcatgatatctacagaacagctttttctgtctccttggagtcatcttgataccctctcctctacacagcatttcatacttttgtctctctgggaggtagtcaacagctgcacctttttttttcagagtggtcttttgatcggattggtcatcggacgaggacttatttgcgtccttttccttagccatgatgtattcaaagtatttcagattaccgttagctctttgatgctccgggtccagctccaacaactttttagttaaaagtagagctttgtccagatcaccttgctggtaaacagcgtatgataagtaatccaaaactgaaaccttatcaacggtagaaacttcaccttcgtccaactgacgcagagcttgctccatccataattctgtgtgatagtagtcggcttctgtatatgcgacttttcccaattcaaaacaatcttccacagtgaggaaggacttatgcttcacaccaggtaaatcacccttcgatatcgtgtcggtgtccaaattgtatgtgtcctgcaatcgcaacaaagcttttgctgctcctacttggtcctcatcgtttggaaagtattgtctttgaattgttaagttagaaatgaatccatcactcatatctttaagtaccaagttttccaattctgaccactctgtattaagtctcttcatcagcttgaaagcattcactgggtgacccacaaaaccctcaggatcttttgttgcagtactagtcaatctatcgagtttctctgcccactttttgatttgctccaacttatcctcttcagctttgatatagtctttaaggcttgtaactaggtctttttctgtgtgaatcaaatcagtcatctgtcctatagaagtgaagaagcctgggtgagccagtgactgtggcaacaaaataccaacgactaggatataccaaatcatgcttttgttgttgagtgaagcgagtgacggaacggtaaaatgtaagtaacaaaagaaaaagagaaccaggggggggaggagagtatgtatttataccgtacggcaccaggcgaaaagctataaacaaacctttttcgcggtatatttgtttatatttcctattttaaactcaaaatctgccctaatctggacttttcatgcaaagttatgcacctgaggcaggaatgaagcaggctcgacgacgaaaaggctggaatgggtaactatggatcgattgatttgtctgttgaaatcttgatttggcactcgtttaaattaacattctgcatcatggtgaattgcggtcacaggtactggtttttcctgaagctctaggcggtgttactgttcccacaacttaaaacctaaaagaggtgggtgcttctttgcgtgggtgaccaaaaataaaaccgactgcctagtggcattgatacctttttttgggtgttgtcctggaaaccactgaacgtatctgcgagatacaaaagtatttttagataagtggcaaatgcaaaaaatctgattggtcagttaatgattgatgaacgactttaaggttaaaaagcaaaatagtgactgctgccatgtgcctgtatagcacatgaactgattattctgttcccacgctacgatgaaaacgccttctctgccgaaagattaaagctgcgcgggaaaaaaaaattaactttacggggcgagcacggttccccgaaacaaaagatggttggctttcacccagcgagctcactggatgccagttaaaaatagttaggtgggttcacctgtttttgtagaaatgtcttggtgtcctcgaccaatcaggtagccatccctgaaatacctggctccgtggcaacaccgaacgacctgctggcaacgttaaattctccggggtaaaacttaaatgtggagtaatagaaccagaaacgtctcttcccttctctctccttccaccgcccgttaccgtccctaggaaattttactctgctggagagcttcttctacggcccccttgcagcaatgctcttcccagcattacgttgcgggtaaaacggaggtcgtgtacccgacctagcagcccagggatggaaagtcccggccgtcgctggcaataactgcgggcggacgcatgtcttgagattattggaaaccaccagaatcgaatataaaaggcgaacacctttcccaattttggtttctcctgacccaaagactttaaatttaatttatttgtccctatttcaatcaattgaacaactatggccgcatgagattcccatctattttcaccgctgtcttgttcgctgcctcctctgcattggctgcccctgttaacactaccactgaagacgagactgctcaaattccagctgaagcagttatcggttactctgaccttgagggtgatttcgacgtcgctgttttgcctttctctaactccactaacaacggtttgttgttcattaacaccactatcgcttccattgctgctaaggaagagggtgtctctctcgagaaaagagaggccgaagctgcacccgatgaggaagatcatgttttagtattgcataaaggaaatttcgatgaagctttggccgctcacaaatatctgctcgtcgagttttacgctccctggtgcggtcattgtaaggcccttgcaccagagtacgccaaggcagctggtaagttaaaggccgaaggttcagagatcagattagcaaaagttgatgctacagaagagtccgatcttgctcaacaatacggggttcgaggatacccaacaattaagtttttcaaaaatggtgatactgcttccccaaaggaatatactgctggtagagaggcagacgacatagtcaactggctcaaaaagagaacgggcccagctgcgtctacattaagcgacggagcagcagccgaagctcttgtggaatctagtgaagttgctgtaatcggtttctttaaggacatggaatctgattcagctaaacagttccttttagcagctgaagcaatcgatgacatccctttcggaatcacctcaaatagtgacgtgttcagcaagtaccaacttgacaaagatggagtggtcttgttcaaaaagtttgacgaaggcagaaacaatttcgagggtgaggttacaaaggagaaactgcttgatttcattaaacataaccaactacccttagttatcgaattcactgaacaaactgctcctaagattttcggtggagaaatcaaaacacatatcttgttgtttttgccaaagtccgtatcggattatgaaggtaaactctccaatttcaaaaaggccgctgagagctttaagggcaagattttgttcatctttattgactcagaccacacagacaatcagaggattttggagtttttcggtttgaaaaaggaggaatgtccagcagtccgtttgatcaccttggaggaggagatgaccaaatacaaaccagagtcggatgagttgactgccgagaagataacagaattttgtcacagatttctggaaggtaagatcaagcctcatcttatgtctcaagagttgcctgatgactgggataagcaaccagttaaagtattggtgggtaaaaactttgaggaagtggccttcgacgagaaaaaaaatgtctttgttgaattctatgctccgtggtgtggtcactgtaagcagctggcaccaatttgggataaactgggtgaaacttacaaagatcacgaaaacattgttattgcaaagatggacagtactgctaacgaagtggaggctgtgaaagttcactccttccctacgctgaagttctttcctgcatctgctgacagaactgttatcgactataatggagagaggacattggatggttttaaaaagtttcttgaatccggaggtcaagacggagctggtgacgacgatgatttggaagatctggaggaggctgaggaacctgatcttgaggaggatgacgaccagaaggcagtcaaagatgaactgtgataaggggtcaagaggatgtcagaatgccatttgcctgagagatgcaggcttcatttttgatacttttttatttgtaacctatatagtataggattttttttgtcattttgtttcttctcgtacgagcttgctcctgatcagcctatctcgcagcagatgaatatcttgtggtaggggtttgggaaaatcattcgagtttgatgtttttcttggtatttcccactcctcttcagagtacagaagattaagtgagaccttcgtttgtgc

SEQ ID NO: 19 - DNA, 12068 bp, Artificial Sequence
  MMV208 (Sequence 17)
cggatgttttattatctatttatgcccttatattctgtaactatccaaaagtcctatcttatcaagccagcaatctatgtccgcgaacgtcaactaaaaataagctttttatgctcttctctctttttttcccttcggtataattataccttgcatccacagattctcctgccaaattttgcataatcctttacaacatggctatatgggagcacttagcgccctccaaaacccatattgcctacgcatgtataggtgttttttccacaatattttctctgtgctctctttttattaaagagaagctctatatcggagaagcttctgtggccgttatattcggccttatcgtgggaccacattgcctgaattggtttgccccggaagattggggaaacttggatctgattaccttagctgcagaaaagggtaccactgagcgtcagaccccgtagaaaagatcaaaggatcttcttgagatcctttttttctgcgcgtaatctgctgcttgcaaacaaaaaaaccaccgctaccagcggtggtttgtttgccggatcaagagctaccaactctttttccgaaggtaactggcttcagcagagcgcagataccaaatactgttcttctagtgtagccgtagttaggccaccacttcaagaactctgtagcaccgcctacatacctcgctctgctaatcctgttaccagtggctgctgccagtggcgataagtcgtgtcttaccgggttggacccaagacgatagttaccggataaggcgcagcggtcgggctgaacggggggttcgtgcacacagcccagcttggagcgaacgacctacaccgaactgagatacctacagcgtgagctatgagaaagcgccacgcttcccgaagggagaaaggcggacaggtatccggtaagcggcagggtcggaacaggagagcgcacgagggagcttccagggggaaacgcctggtatctttatagtcctgtcgggtttcgccacctctgacttgagcgtcgatttttgtgatgctcgtcaggggggcggagcctatggaaaaacgccagcaacgcggcctttttacggttcctggccttttgctggccttttgctcatatgtaagctttgaacacttatgtaagctcgaaaccagttaggtaagcagctttgtaagcaatctggacaatatgtaagcgggttacgtaaacagttatgtaagcagaaaaatttcaaacgacaaaacttggggtctacagacacagtagccagaagattgcactaccattcgactcctcatgacccactctttcgatccatgtagttaggttaccgtttttcctaatatttaaggatgttgaaaattcattttcattttttttcgtttttaagattttctcacaactcttccaaagattactagttgacttttcaaaatatttagggtatttttctcactttttcctagcaaactccaattggtgggttcagtgcaatggagtaccaccttgcaaccacaacgtaatagctaacttgtggccaccatgtctggttgtagagataattggattctaatgtggatcacatgactactcacgtgtcaaaaacccaacctgacttggcccagcttagcaagaatatttcgaatccactcttgtggcctagtggacaactgggacctagggacccttgtgactgacactttgggagtccctattctacttagtctcatatcgcatgaaacttttgataaattattttctgataggaatttttcatcagatattatcatcgcggcttacgtaataacaaaaaaaattgatggagtctatactaggctaacataaactaagttattaattaaacaaaacaaaacgtactagcattactgtcatatataagggctcctaactaaaactgtaaagacttcccgtaaaattatcattctaattctgacaatgtgcatggcctcctaaactcttgacctctctcatgcagccacttattggaaacccacttattaccgactaagacgggacaagcagcatgtctagtgctgtaatcaccttctccagatgcaaacagattgtaccaaaatacggccgtgccctttttaggccaaacagaagcaccaacctcagggaaaactgtggctcctccagcaagcacatcggacatatagaacaaccacgttgcgattctatttccagtacctagctccttaaaagcatcaggctcgtcctttctggcgaaatcaaagtggggttcatactgaccgcccacaccatagttggcaacttgtagttcttcagcagtgcttacgtcaagaccagtcaaatcttgaatacgcatattgatacggctgaccacgggattctcgtaaccggacaaccatgctgatttagagacacgatattgtgcggtagtcaattttccagtctcagggtcatggacggtagccctactcaatcttggtttggccaagtctttcacaacctctatttctgcatcggagatgatgtcatgaaaacgaatgattctaggcttgtcccattcatcttcctgtttcgctggagcaagaatgaattttgggttacggttcccatcatgatatctacagaacagctttttctgtctccttggagtcatcttgataccctctcctctacacagcatttcatacttttgtctctctgggaggtagtcaacagccgcacctttttttttcagagtggtcttttgatcggattggtcatcggacgaggacttatttgcgtccttttccttagccatgatgtattcaaagtatttcagattaccgttagctctttgatgctccgggtccagctccaacaactttttagttaaaagtagagctttgtccagatcaccttgctggtaaacagcgtatgataagtaatccaaaactgaaaccttatcaacggtagaaacttcaccttcgtccaactgacgtagagcttgctccatccataattctgtgtgatagtagtcggcttctgtatatgcgacttttcccaattcaaaacaatcttccacagtgaggaaggacttatgcttcacaccaggtaaatcacccttcgatatcgtgtcggtgtccaaattgtatgtgtcctgcaatcgcaacaaagcttttgctgctcctacttggtcctcatcgtttggaaagtattgtctttgaattgttaagttagaaatgaatccatcactcatatctttaagtaccaagttttccaattctgaccactctgtattaagtctcttcatcagcttgaaagcattcactgggtgacccacaaaaccctcaggatcttttgttgcagtacttgtcaatctatcgagtttctctgcccactttttgatttgctccaacttatcctcttcagctttgatatagtctttaaggcttgtaactaggtctttttctgtgtgaatcaaatcagtcatctgtcctatagaagtgaagaagcctgggtgagccagtgactgtggcaacaaaataccaacgactaggatataccaaatcatgcggccgcatggcccccgacgaggaggaccacgtcctggtgctccataagggcaacttcgacgaggcgctggcggcccacaagtacctgctggtggagttctacgccccatggtgcggccactgcaaggctctggccccggagtatgccaaagcagctgggaagctgaaggcagaaggttctgagatcagactggccaaggtggatgccactgaagagtctgacctggcccagcagtatggtgtccgaggctaccccaccatcaagttcttcaagaatggagacacagcttcccccaaagagtacacagctggccgggaagcggatgatatcgtgaactggctgaagaagcgcacgggccccgctgccagcacgctgtccgacggggctgctgcagaggctttggtggagtccagtgaggtggccgtcattggcttcttcaaggatatggagtcggactccgcaaagcagttcttcttggcagcagaggtcattgatgacatccccttcgggatcacatctaacagcgatgtgttctccaaataccagctggacaaggatggggttgtcctctttaagaagtttgacgaaggccggaacaactttgagggggaggtcaccaaagaaaagcttctggacttcatcaagcacaaccagttgcccctggtcattgagttcaccgagcagacagccccgaagatcttcggaggggaaatcaagactcacatcctgctgttcctgccgaaaagcgtgtctgactatgagggcaagctgagtaacttcaaaaaagcggctgagagcttcaagggcaagatcctgtttatcttcatcgacagcgaccacactgacaaccagcgcatcctggagttcttcggcctaaagaaagaggagtgcccggccgtgcgcctcatcacgctggaggaggagatgaccaaatataagccagagtcagatgagctgacggcagagaagatcaccgagttctgccaccgcttcctggagggcaagattaagccccacctgatgagccaggagctgcctgacgactgggacaagcagcctgtcaaagtgctggttgggaagaactttgaagaggttgcttttgatgagaaaaagaacgtctttgtagagttctatgccccgtggtgcggtcactgcaagcagctggcccccatctgggataagctgggagagacgtacaaggaccacgagaacatagtcatcgccaagatggactccacggccaacgaggtggaggcggtgaaagtgcacagcttccccacgctcaagttcttccccgccagcgccgacaggacggtcatcgactacaatggggaacggacactggatggttttaagaagttcctggagagtggtggccaggatggggccggagatgatgacgatcttgaagatcttgaagaagcagaagagcctgatctggaggaagatgatgatcaaaaagctgtgaaagatgaactgtaatcaagaggatgtcagaatgccatttgcctgagagatgcaggcttcatttttgatacttttttatttgtaacctatatagtataggattttttttgtcattttgtttcttctcgtacgagcttgctcctgatcagcctatctcgcagcagatgaatatcttgtggtaggggtttgggaaaatcattcgagtttgatgtttttcttggtatttcccactcctcttcagagtacagaagattaagtgagaccttcgtttgtgccgatcggttcagaagcgatagagagactgcgctaagcattaatgagattatttttgagcattcgtcaatcaataccaaacaagacaaacggtatgccgacttttggaagtttctttttgaccaactggccgttagcatttcaacgaaccaaacttagttcatcttggatgagatcacgcttttgtcatattaggttccaagacagcgtttaaactgtcagttttgggccatttggggaacatgaaactatttgaccccacactcagaaagccctcatctggagtgatgttcgggtgtaatgcggagcttgttgcattcggaaataaacaaacatgaacctcgccaggggggccaggatagacaggctaataaagtcatggtgttagtagcctaatagaaggaattggaatgagcggatccaatgtatctaaacgcaaactccgagctggaaaaatgttaccggcgatgcgcggacaatttagaggcggcgatcaagaaacacctgctgggcgagcagtctggagcacagtcttcgatgggcccgagatcccaccgcgttcctgggtaccgggacgtgaggcagcgcgacatccatcaaatataccaggcgccaaccgagtctctcggaaaacagcttctggatatcttccgctggcggcgcaacgacgaataatagtccctggaggtgacggaatatatatgtgtggagggtaaatctgacagggtgtagcaaaggtaatattttcctaaaacatgcaatcggctgccccgcaacgggaaaaagaatgactttggcactcttcaccagagtggggtgtcccgctcgtgtgtgcaaataggctcccactggtcaccccggattttgcagaaaaacagcaagttccggggtgtctcactggtgtccgccaataagaggagccggcaggcacggagtctacatcaagctgtctccgatacactcgactaccatccgggtctctcagagaggggaatggcactataaataccgcctccttgcgctctctgccttcatcaatcaaatcggatccatgtcttttgtccaaaagggtacttggttactttttgctctgttgcacccaactgttattctcgcacaacaggaagcagtagatggtggttgctcacatttaggtcaatcttacgcagatagagatgtatggaaacctgaaccatgtcaaatttgcgtgtgtgactcaggttcagtgctctgcgacgatatcatatgtgacgaccaggaattggactgtccaaacccagagataccattcggtgaatgttgtgctgtttgtccacagccaccaactgctcctacaagacctccaaacggtcaaggtccacaaggtcctaaaggtgatccgggtccacctggtattcctggtagaaatggtgaccctggacctcccggttccccaggtagcccaggatcacctgggcctcctggaatatgtgaatcctgcccaactggtggtcagaactatagcccacaatacgaggcctacgacgtcaaatctggtgttgctggaggaggtattgcaggctaccctggtcccgcagggcccccaggtccgccgggtccgcccggaacatcaggtcatcccggagcccctggtgcaccaggttatcagggaccgcccggagagcctggacaagctggtcccgctggaccccctggtccaccaggtgctattggaccaagtggtcctgccggaaaagacggtgaatccggtagacctggtagacccggcgaaaggggtttcccaggtcctcccggaatgaagggtccagccggtatgcccggttttcctgggatgaagggtcacagaggatttgatggtagaaacggagagaaaggcgaaaccggtgctcccggactgaagggtgaaaacggtgtccctggtgagaacggcgctcctggacctatgggtccacgtggtgctccaggagaaagaggcagaccaggattgcctggtgcagctggtgctagaggtaacgatggtgcccgtggttccgatggacaacccgggccacccggccctccaggtaccgctggatttcctggaagccctggtgctaagggggaggttggtccggctggtagtcccggaagtagcggtgccccaggtcaaagaggcgaaccaggccctcagggtcacgcaggagcacctggaccgcctggtcctcctggttcgaatggttcgcctggaggaaaaggtgaaatggggcccgcaggaatccccggtgcgcctggtcttattggtgccaggggtcctccaggcccgccaggtacaaatggtgtacccggacagcgaggagcagctggtgaacctggtaaaaacggtgccaaaggagatccaggtcctcgtggagagcgtggtgaagctggctctcccggtatcgccggtccaaaaggtgaggacggtaaggacggttcccctggtgagccaggtgcgaacggactgccaggtgcagccggagagcgaggagtcccaggattcaggggaccagccggtgctaacggcttgcctggtgaaaaagggccccctggtgataggggaggacccggtccagcaggccctcgtggagttgctggtgagcctggacgtgacggtttaccaggagggccaggtttgaggggtattcccgggtcccctggcggtcctggatcggatggaaaaccagggccaccaggttcgcagggtgaaacaggacgtccaggcccacccggctcacctggtccaaggggtcagcctggtgtcatgggtttccccggtccaaagggtaatgacggagcaccgggtaaaaatggtgaacgtggtggcccaggtggtccaggaccccaaggtccagctggaaaaaacggtgagacaggtcctcaaggacctccaggacctaccggtcctagcggagataagggagatacgggaccgccaggacctcaaggattgcaaggtttgcctggtacatctggccctcccggagaaaatggtaagcctggagagccaggaccaaaaggcgaagctggagccccaggtatccccggaggtaagggagactcaggtgctccgggtgagcgtggtcctccgggtgccggtggtccacctggacctagaggtggtgccgggccgccaggtcctgaaggtggtaaaggtgctgctggtccaccgggaccgcctggctctgctggtactcctggcttgcagggaatgccaggagagagaggtggacctggaggtcccggtccgaagggtgataaaggggagccaggatcatccggtgttgacggcgcacctggtaaagacggaccaaggggaccaacgggtccaatcggaccaccaggacccgctggccagccaggagataaaggcgagtccggagcacccggtgttcctggtatagctggacccaggggtggtcccggtgaaagaggtgaacagggcccaccgggtcccgccggtttccctggcgcccctggtcaaaatggagaaccaggtgcaaagggcgagagaggagccccaggagaaaagggtgagggaggaccacccggtgctgccggtccagctgggggttcaggtcctgctggaccaccaggtccacagggcgttaaaggtgagagaggaagtccaggtggtcctggagctgctggattcccaggtggccgtggacctcctggtccccctggatcgaatggtaatcctggtccgccaggtagttcgggtgctcctgggaaggacggtccacctggccccccaggtagtaacggtgcacctggtagtccaggtatatccggacctaaaggagattccggtccaccaggcgaaagaggggccccaggcccacagggtccaccaggagcccccggtcctctgggtattgctggtcttactggtgcacgtggactggccggtccacccggaatgcctggagcaagaggttcacctggaccacaaggtattaaaggagagaacggtaaacctggaccttccggtcaaaacggagagcggggacccccaggcccccaaggtctgccaggactagctggtaccgcaggggaaccaggaagagatggaaatccaggttcagacggactacccggtagagatggtgcaccgggggccaagggcgacaggggtgagaatggatctcctggtgcgccaggggcaccaggccacccaggtcccccaggtcctgtgggccctgctggaaagtcaggtgacaggggagagacaggcccggctggtccatctggcgcacccggaccagctggttccagaggcccacctggtccgcaaggccctagaggtgacaagggagagactggagaacgaggtgctatgggtatcaagggtcatagaggttttccgggtaatcccggcgccccaggttctcctggtccagctggccatcaaggtgcagtcggatcgcccggcccagccggtcccaggggccctgttggtccatccggtcctccaggaaaggatggtgcttctggacacccaggacctatcggacctccgggtcctagaggtaatagaggagaacgtggttccgagggtagtcctggtcaccctggtcaacctggcccaccagggcctccaggtgcacccggtccatgttgtggtgcaggcggtgtggctgcaattgctggtgtgggtgctgaaaaggccggcggtttcgctccatattatggtgatgaaccgattgattttaagatcaatactgacgaaatcatgacttccttaaagtccgttaatggtcaaattgagtctctaatctccccagatggttcacgtaaaaatcctgctagaaattgtagagatttgaagttttgtcaccccgagttgcagtccggtgagtactgggtggaccccaatcaaggttgtaagttagacgctattaaagtttactgcaatatggagacaggagaaacttgcatcagcgcttctccattgactatcccacaaaaaaattggtggactgactctggagctgagaaaaagcatgtatggttcggggaatcgatggaaggtggtttccaattcagctacggtaaccctgaacttcctgaagatgttcttgacgttcaattggcatttctgagattgttgtccagtcgtgcaagccaaaacattacataccattgcaaaaattccatcgcatatatggatcatgctagcggaaatgtgaaaaaggcattgaagctgatgggatcaaatgaaggtgaatttaaagcagagggtaattctaagtttacttacactgtattggaggatggttgtacgaagcatacaggtgaatggggtaaaacagtgtttcaatatcaaacccgcaaagcagttagattgccaatcgtcgatatcgcaccatacgacattggaggaccagatcaagagttcggagctgacatcggtccggtgtgtttcctttgataatcaagaggatgtcagaatgccatttgcctgagagatgcaggcttcatttttgatacttttttatttgtaacctatatagtataggattttttttgtcattttgtttcttctcgtacgagcttgctcctgatcagcctatctcgcagctgatgaatatcttgtggtaggggtttgggaaaatcattcgagtttgatgtttttcttggtatttcccactcctcttcagagtacagaagattaagtgagacgttcgtttgtgcccgcggatttaaatgatccttcagtaatgtcttgtttcttttgttgcagtggtgagccattttgacttcgtgaaagtttctttagaatagttgtttccagaggccaaacattccacccgtagtaaagtgcaagcgtaggaagaccaagactggcataaatcaggtataagtgtcgagcactggcaggtgatcttctgaaagtttctactagcagataagatccagtagtcatgcatatggcaacaatgtaccgtgtggatctaagaacgcgtcctactaaccttcgcattcgttggtccagtttgttgttatcgatcaacgtgacaaggttgtcgattccgcgtaagcatgcatacccaaggacgcctgttgcaattccaagtgagccagttccaacaatctttgtaatattagagcacttcattgtgttgcgcttgaaagtaaaatgcgaacaaattaagagataatctcgaaaccgcgacttcaaacgccaatatgatgtgcggcacacaataagcgttcatatccgctgggtgactttctcgctttaaaaaattatccgaaaaaattttctagagtgttgttactttatacttccggctcgtataatacgacaaggtgtaaggaggactaaaccatggctaaactcacctctgctgttccagtcctgactgctcgtgatgttgctggtgctgttgagttctggactgataggctcggtttctcccgtgacttcgtagaggacgactttgccggtgttgtacgtgacgacgttaccctgttcatctccgcagttcaggaccaggttgtgccagacaacactctggcatgggtatgggttcgtggtctggacgaactgtacgctgagtggtctgaggtcgtgtctaccaacttccgtgatgcatctggtccagctatgaccgagatcggtgaacagccctggggtcgtgagtttgcactgcgtgatccagctggtaactgcgtgcatttcgtcgcagaagagcaggactaacaattgacaccttacgattatttagagagtatttattagttttattgtatgtata

SEQ ID NO: 20 - DNA, 5735 bp, Artificial Sequence
  MMV84 (Sequence 18)
aacatccaaagacgaaaggttgaatgaaacctttttgccatccgacatccacaggtccattctcacacataagtgccaaacgcaacaggaggggatacactagcagcagaccgttgcaaacgcaggacctccactcctcttctcctcaacacccacttttgccatcgaaaaaccagcccagttattgggcttgattggagctcgctcattccaattccttctattaggctactaacaccatgactttattagcctgtctatcctggcccccctggcgaggttcatgtttgtttatttccgaatgcaacaagctccgcattacacccgaacatcactccagatgagggctttctgagtgtggggtcaaatagtttcatgttccccaaatggcccaaaactgacagtttaaacgctgtcttggaacctaatatgacaaaagcgtgatctcatccaagatgaactaagtttggttcgttgaaatgctaacggccagttggtcaaaaagaaacttccaaaagtcggcataccgtttgtcttgtttggtattgattgacgaatgctcaaaaataatctcattaatgcttagcgcagtctctctatcgcttctgaaccccggtgcacctgtgccgaaacgcaaatggggaaacacccgctttttggatgattatgcattgtctccacattgtatgcttccaagattctggtgggaatactgctgatagcctaacgttcatgatcaaaatttaactgttctaacccctacttgacagcaatatataaacagaaggaagctgccctgtcttaaacctttttttttatcatcattattagcttactttcataattgcgactggttccaattgacaagcttttgattttaacgacttttaacgacaacttgagaagatcaaaaaacaactaattattgaaagaattcaaaacgaaaatgagattcccatctattttcaccgctgtcttgttcgctgcctcctctgcattggctgcccctgttaacactaccactgaagacgagactgctcaaattccagctgaagcagttatcggttactctgaccttgagggtgatttcgacgtcgctgttttgcctttctctaactccactaacaacggtttgttgttcattaacaccactatcgcttccattgctgctaaggaagagggtgtctctctcgagaaaagagaggccgaagctgcacccgatgaggaagatcatgttttagtattgcataaaggaaatttcgatgaagctttggccgctcacaaatatctgctcgtcgagttttacgctccctggtgcggtcattgtaaggcccttgcaccagagtacgccaaggcagctggtaagttaaaggccgaaggttcagagatcagattagcaaaagttgatgctacagaagagtccgatcttgctcaacaatacggggttcgaggatacccaacaattaagtttttcaaaaatggtgatactgcttccccaaaggaatatactgctggtagagaggcagacgacatagtcaactggctcaaaaagagaacgggcccagctgcgtctacattaagcgacggagcagcagccgaagctcttgtggaatctagtgaagttgctgtaatcggtttctttaaggacatggaatctgattcagctaaacagttccttttagcagctgaagcaatcgatgacatccctttcggaatcacctcaaatagtgacgtgttcagcaagtaccaacttgacaaagatggagtggtcttgttcaaaaagtttgacgaaggcagaaacaatttcgagggtgaggttacaaaggagaaactgcttgatttcattaaacataaccaactacccttagttatcgaattcactgaacaaactgctcctaagattttcggtggagaaatcaaaacacatatcttgttgtttttgccaaagtccgtatcggattatgaaggtaaactctccaatttcaaaaaggccgctgagagctttaagggcaagattttgttcatctttattgactcagaccacacagacaatcagaggattttggagtttttcggtttgaaaaaggaggaatgtccagcagtccgtttgatcaccttggaggaggagatgaccaaatacaaaccagagtcggatgagttgactgccgagaagataacagaattttgtcacagatttctggaaggtaagatcaagcctcatcttatgtctcaagagttgcctgatgactgggataagcaaccagttaaagtattggtgggtaaaaactttgaggaagtggccttcgacgagaaaaaaaatgtctttgttgaattctatgctccgtggtgtggtcactgtaagcagctggcaccaatttgggataaactgggtgaaacttacaaagatcacgaaaacattgttattgcaaagatggacagtactgctaacgaagtggaggctgtgaaagttcactccttccctacgctgaagttctttcctgcatctgctgacagaactgttatcgactataatggagagaggacattggatggttttaaaaagtttcttgaatccggaggtcaagacggagctggtgacgacgatgatttggaagatctggaggaggctgaggaacctgatcttgaggaggatgacgaccagaaggcagtcaaagatgaactgtgataaggggggttaaaggggcggccgctcaagaggatgtcagaatgccatttgcctgagagatgcaggcttcatttttgatacttttttatttgtaacctatatagtataggattttttttgtcattttgtttcttctcgtacgagcttgctcctgatcagcctatctcgcagcagatgaatatcttgtggtaggggtttgggaaaatcattcgagtttgatgtttttcttggtatttcccactcctcttcagagtacagaagattaagtgaaaccttcgtttgtgcggatccttcagtaatgtcttgtttcttttgttgcagtggtgagccattttgacttcgtgaaagtttctttagaatagttgtttccagaggccaaacattccacccgtagtaaagtgcaagcgtaggaagaccaagactggcataaatcaggtataagtgtcgagcactggcaggtgatcttctgaaagtttctactagcagataagatccagtagtcatgcatatggcaacaatgtaccgtgtggatctaagaacgcgtcctactaaccttcgcattcgttggtccagtttgttgttatcgatcaacgtgacaaggttgtcgattccgcgtaagcatgcatacccaaggacgcctgttgcaattccaagtgagccagttccaacaatctttgtaatattagagcacttcattgtgttgcgcttgaaagtaaaatgcgaacaaattaagagataatctcgaaaccgcgacttcaaacgccaatatgatgtgcggcacacaataagcgttcatatccgctgggtgactttctcgctttaaaaaattatccgaaaaaattttctagagtgttgttactttatacttccggctcgtataatacgacaaggtgtaaggaggactaaaccatgggtaaggaaaagactcacgtttcgaggccgcgattaaattccaacatggatgctgatttatatgggtataaatgggctcgcgataatgtcgggcaatcaggtgcgacaatctatcgattgtatgggaagcccgatgcgccagagttgtttctgaaacatggcaaaggtagcgttgccaatgatgttacagatgagatggtcagactaaactggctgacggaatttatgcctcttccgaccatcaagcattttatccgtactcctgatgatgcatggttactcaccactgcgatccccggcaaaacagcattccaggtattagaagaatatcctgattcaggtgaaaatattgttgatgcgctggcagtgttcctgcgccggttgcattcgattcctgtttgtaattgtccttttaacagcgatcgcgtatttcgtctcgctcaggcgcaatcacgaatgaataacggtttggttgatgcgagtgattttgatgacgagcgtaatggctggcctgttgaacaagtctggaaagaaatgcataagcttttgccattctcaccggattcagtcgtcactcatggtgatttctcacttgataaccttatttttgacgaggggaaattaataggttgtattgatgttggacgagtcggaatcgcagaccgataccaggatcttgccatcctatggaactgcctcggtgagttttctccttcattacagaaacggctttttcaaaaatatggtattgataatcctgatatgaataaattgcagtttcatttgatgctcgatgagtttttctaacaattgacaccttacgattatttagagagtatttattagttttattgtatgtatacggatgttttattatctatttatgcccttatattctgtaactatccaaaagtcctatcttatcaagccagcaatctatgtccgcgaacgtcaactaaaaataagctttttatgctgttctctctttttttcccttcggtataattataccttgcatccacagattctcctgccaaattttgcataatcctttacaacatggctatatgggagcacttagcgccctccaaaacccatattgcctacgcatgtataggtgttttttccacaatattttctctgtgctctctttttattaaagagaagctctatatcggagaagcttctgtggccgttatattcggccttatcgtgggaccacattgcctgaattggtttgccccggaagattggggaaacttggatctgattaccttagctgcaggtaccactgagcgtcagaccccgtagaaaagatcaaaggatcttcttgagatcctttttttctgcgcgtaatctgctgcttgcaaacaaaaaaaccaccgctaccagcggtggtttgtttgccggatcaagagctaccaactctttttccgaaggtaactggcttcagcagagcgcagataccaaatactgttcttctagtgtagccgtagttaggccaccacttcaagaactctgtagcaccgcctacatacctcgctctgctaatcctgttaccagtggctgctgccagtggcgataagtcgtgtcttaccgggttggactcaagacgatagttaccggataaggcgcagcggtcgggctgaacggggggttcgtgcacacagcccagcttggagcgaacgacctacaccgaactgagatacctacagcgtgagctatgagaaagcgccacgcttcccgaagggagaaaggcggacaggtatccggtaagcggcagggtcggaacaggagagcgcacgagggagcttccagggggaaacgcctggtatctttatagtcctgtcgggtttcgccacctctgacttgagcgtcgatttttgtgatgctcgtcaggggggcggagcctatggaaaaacgccagcaacgcggcctttttacggttcctggccttttgctggccttttgctcacatgttctttcctgcggtacccagatccaattcccgctttgactgcctgaaatctccatcgcctacaatgatgacatttggatttggttgactcatgttggtattgtgaaatagacgcagatcgggaacactgaaaaatacacagttattattcatttaaat

SEQ ID NO: 21 - DNA, 7204 bp, Artificial Sequence
  MMV150 (Sequence 19)
aaaaataagctttttatgctcttctctctttttttcccttcggtataattataccttgcatccacagattctcctgccaaattttgcataatcctttacaacatggctatatgggagcacttagcgccctccaaaacccatattgcctacgcatgtataggtgttttttccacaatattttctctgtgctctctttttattaaagagaagctctatatcggagaagcttctgtggccgttatattcggccttatcgtgggaccacattgcctgaattggtttgccccggaagattggggaaacttggatctgattaccttagctgcagaaaagggtaccactgagcgtcagaccccgtagaaaagatcaaaggatcttcttgagatcctttttttctgcgcgtaatctgctgcttgcaaacaaaaaaaccaccgctaccagcggtggtttgtttgccggatcaagagctaccaactctttttccgaaggtaactggcttcagcagagcgcagataccaaatactgttcttctagtgtagccgtagttaggccaccacttcaagaactctgtagcaccgcctacatacctcgctctgctaatcctgttaccagtggctgctgccagtggcgataagtcgtgtcttaccgggttggacccaagacgatagttaccggataaggcgcagcggtcgggctgaacggggggttcgtgcacacagcccagcttggagcgaacgacctacaccgaactgagatacctacagcgtgagctatgagaaagcgccacgcttcccgaagggagaaaggcggacaggtatccggtaagcggcagggtcggaacaggagagcgcacgagggagcttccagggggaaacgcctggtatctttatagtcctgtcgggtttcgccacctctgacttgagcgtcgatttttgtgatgctcgtcaggggggcggagcctatggaaaaacgccagcaacgcggcctttttacggttcctggccttttgctggccttttgctcacatgtattttatgtaagctttgaacacttatgtaagctcgaaaccagttaggtaagcagctttgtaagcaatctggacaatatgtaagcgggttacgtaaacagttatgtaagcagaaaaatttcaaacgacaaaacttggggtctacagacacagtagccagaagattgcactaccattcgactcctcatgacccactctttcgatccatgtagttaggttaccgtttttcctaatatttaaggatgttgaaaattcattttcattttttttcgtttttaagattttctcacaactcttccaaagattactagttgacttttcaaaatatttagggtatttttctcactttttcctagcaaactccaattggtgggttcagtgcaatggagtaccaccttgcaaccacaacgtaatagctaacttgtggccaccatgtctggttgtagagataattggattctaatgtggatcacatgactactcacgtgtcaaaaacccaacctgacttggcccagcttagcaagaatatttcgaatccactcttgtggcctagtggacaactgggaaagcttgcgacgcagtcgtttttggcgatccaggcgtagtactaggaaataatgtatctaaacgcaaactccgagctggaaaaatgttaccggcgatgcgcggacaatttagaggcggcgatcaagaaacacctgctgggcgagcagtctggagcacagtcttcgatgggcccgagatcccaccgcgttcctgggtaccgggacgtgaggcagcgcgacatccatcaaatataccaggcgccaaccgagtgtctcggaaaacagcttctggatatcttccgctggcggcgcaacgacgaataatagtccctggaggtgacggaatatatatgtgtggagggtaaatctgacagggtgtagcaaaggtaatattttcctaaaacatgcaatcggctgccccgcaacgggaaaaagaatgactttggcactcttcaccagagtggggtgtcccgctcgtgtgtgcaaataggctcccactggtcaccccggattttgcagaaaaacagcaagttccggggtgtctcactggtgtccgccaataagaggagccggcaggcacggagtttacatcaagctgtctccgatacactcgactaccatccgggtctctcagagaggggaatggcactataaataccgcctccttgcgctctctgccttcatcaatcaaatcatgctgaggactcgaattccctaggatgttctctccaattttgtccttggaaattattttagctttggctactttgcaatctgtcttcgctcaacagtatccgtatgatgtgccggattatgcgtctccccagtacgaagcatatgatgtcaagtctggagtagcaggaggaggaatcgcaggctatcctgggccagctggtcctcctggcccacccggaccccctggcacatctggccatcctggtgcccctggcgctccaggataccaaggtccccccggtgaacctgggcaagctggtccggcaggtcctccaggacctcctggtgctataggtccatctggccctgctggaaaagatggggaatcaggaagacccggacgacctggagagcgaggatttcctggccctcctggtatgaaaggcccagctggtatgcctggattccctggtatgaaaggacacagaggctttgatggacgaaatggagagaaaggcgaaactggtgctcctggattaaagggggaaaatggcgttccaggtgaaaatggagctcctggacccatgggtccaagaggggctcccggtgagagaggacggccaggacttcctggagccgcaggggctcgaggtaatgatggagctcgaggaagtgatggacaaccgggcccccctggtcctcctggaactgcaggattccctggttcccctggtgctaagggtgaagttggacctgcaggatctcctggttcaagtggcgcccctggacaaagaggagaacctggacctcagggacatgctggtgctccaggtccccctgggcctcctgggagtaatggtagtcctggtggcaaaggtgaaatgggtcctgctggcattcctggggctcctgggctgataggagctcgtggtcctccagggccacctggcaccaatggtgttcccgggcaacgaggtgctgcaggtgaacccggtaagaatggagccaaaggagacccaggaccacgtggggaacgcggagaagctggttctccaggtatcgcaggacctaagggtgaagatggcaaagatggttctcctggagaacctggtgcaaatggacttcctggagctgcaggagaaaggggtgtgcctggattccgaggacctgctggagcaaatggccttccaggagaaaagggtcctcctggggaccgtggtggcccaggccctgcagggcccagaggtgttgctggagagcccggcagagatggtctccctggaggtccaggattgaggggtattcctggtagccccggaggaccaggcagtgatgggaaaccagggcctcctggaagccaaggagagacgggtcgacccggtcctccaggttcacctggtccgcgaggccagcctggtgtcatgggcttccctggtcccaaaggaaacgatggtgctcctggaaaaaatggagaacgaggtggccctggaggtcctggccctcagggtcctgctggaaagaatggtgagaccggacctcagggtcctccaggacctactggcccttctggtgacaaaggagacacaggaccccctggtccacaaggactacaaggcttgcctggaacgagtggtcccccaggagaaaacggaaaacctggtgaacctggtccaaagggtgaggctggtgcacctggaattccaggaggcaagggtgattctggtgctcccggtgaacgcggacctcctggagcaggagggccccctggacctagaggtggagctggcccccctggtcccgaaggaggaaagggtgctgctggtccccctgggccacctggttctgctggtacacctggtctgcaaggaatgcctggagaaagagggggtcctggaggccctggtccaaagggtgataagggtgagcctggcagctcaggtgtcgatggtgctccagggaaagatggtccacggggtcccactggtcccattggtcctcctggcccagctggtcagcctggagataagggtgaaagtggtgcccctggagttccgggtatagctggtcctcgcggtggccctggtgagagaggcgaacaggggcccccaggacctgctggcttccctggtgctcctggccagaatggtgagcctggtgctaaaggagaaagaggcgctcctggtgagaaaggtgaaggaggccctcccggagccgcaggacccgccggaggttctgggcctgccggtcccccaggcccccaaggtgtcaaaggcgaacgtggcagtcctggtggtcctggtgctgctggcttccccggtggtcgtggtcctcctggccctcctggcagtaatggtaacccaggccccccaggctccagtggtgctccaggcaaagatggtcccccaggtccacctggcagtaatggtgctcctggcagccccgggatctctggaccaaagggtgattctggtccaccaggtgagaggggagcacctggcccccagggccctccgggagctccaggcccactaggaattgcaggacttactggagcacgaggtcttgcaggcccaccaggcatgccaggtgctaggggcagccccggcccacagggcatcaagggtgaaaatggtaaaccaggacctagtggtcagaatggagaacgtggtcctcctggcccccagggtcttcctggtctggctggtacagctggtgagcctggaagagatggaaaccctggatcagatggtctgccaggccgagatggagctccaggtgccaagggtgaccgtggtgaaaatggctctcctggtgcccctggagctcctggtcacccaggccctcctggtcctgtcggtccagctggaaagagcggtgacagaggagaaactggccctgctggtccttctggggcccccggtcctgccggatcaagaggtcctcctggtccccaaggcccacgcggtgacaaaggggaaaccggtgagcgtggtgctatgggcatcaaaggacatcgcggattccctggcaacccaggggcccccggatctccgggtcccgctggtcatcaaggtgcagttggcagtccaggccctgcaggccccagaggacctgttggacctagcgggccccctggaaaggacggagcaagtggacaccctggtcccattggaccaccggggccccgaggtaacagaggtgaaagaggatctgagggctccccaggccacccaggacaaccaggccctcctggacctcctggtgcccctggtccatgttgtggtgctggcggggttgctgccattgctggtgttggagccgaaaaagctggtggttttgccccatattatggagctagcggttacattcctgaagctcctagagacggacaagcatacgttagaaaggacggtgagtgggtgttgctgtccaccttcttagctagcgattacaaggatgacgacgataagggatcgtgttgcccgggctgctgtcatcaccatcatcaccatagatcttaagcggccgcgagtcgtgagtaatcaagaggatgtcagaatgccatttgcctgagagatgcaggcttcatttttgatacttttttatttgtaacctatatagtataggattttttttgtcattttgtttcttctcgtacgagcttgctcctgatcagcctatctcgcagctgatgaatatcttgtggtaggggtttgggaaaatcattcgagtttgatgtttttcttggtatttcccactcctcttcagagtacagaagattaagtgagacgttcgtttgtgctccggaggatccttcagtaatgtcttgtttcttttgttgcagtggtgagccattttgacttcgtgaaagtttctttagaatagttgtttccagaggccaaacattccacccgtagtaaagtgcaagcgtaggaagaccaagactggcataaatcaggtataagtgtcgagcactggcaggtgatcttctgaaagtttctactagcagataagatccagtagtcatgcatatggcaacaatgtaccgtgtggatctaagaacgcgtcctactaaccttcgcattcgttggtccagtttgttgttatcgatcaacgtgacaaggttgtcgattccgcgtaagcatgcatacccaaggacgcctgttgcaattccaagtgagccagttccaacaatctttgtaatattagagcacttcattgtgttgcgcttgaaagtaaaatgcgaacaaattaagagataatctcgaaaccgcgacttcaaacgccaatatgatgtgcggcacacaataagcgttcatatccgctgggtgactttctcgctttaaaaaattatccgaaaaaattttctagagtgttgttactttatacttccggctcgtataatacgacaaggtgtaaggaggactaaaccatggctaaactcacctctgctgttccagtcctgactgctcgtgatgttgctggtgctgttgagttctggactgataggctcggtttctcccgtgacttcgtagaggacgactttgccggtgttgtacgtgacgacgttaccctgttcatctccgcagttcaggaccaggttgtgccagacaacactctggcatgggtatgggttcgtggtctggacgaactgtacgctgagtggtctgaggtcgtgtctaccaacttccgtgatgcatctggtccagctatgaccgagatcggtgaacagccctggggtcgtgagtttgcactgcgtgatccagctggtaactgcgtgcatttcgtcgcagaagagcaggactaacaattgacaccttacgattatttagagagtatttattagttttattgtatgtatacggatgttttattatctatttatgcccttatattctgtaactatccaaaagtcctatcttatcaagccagcaatctatgtccgcgaacgtcaact

SEQ ID NO: 22 - DNA, 6601 bp, Artificial Sequence
  MMV140 (Sequence 20)
gatcaaaggatcttcttgagatcctttttttctgcgcgtaatctgctgcttgcaaacaaaaaaaccaccgctaccagcggtggtttgtttgccggatcaagagctaccaactctttttccgaaggtaactggcttcagcagagcgcagataccaaatactgttcttctagtgtagccgtagttaggccaccacttcaagaactctgtagcaccgcctacatacctcgctctgctaatcctgttaccagtggctgctgccagtggcgataagtcgtgtcttaccgggttggacccaagacgatagttaccggataaggcgcagcggtcgggctgaacggggggttcgtgcacacagcccagcttggagcgaacgacctacaccgaactgagatacctacagcgtgagctatgagaaagcgccacgcttcccgaagggagaaaggcggacaggtatccggtaagcggcagggtcggaacaggagagcgcacgagggagcttccagggggaaacgcctggtatctttatagtcctgtcgggtttcgccacctctgacttgagcgtcgatttttgtgatgctcgtcaggggggcggagcctatggaaaaacgccagcaacgcggcctttttacggttcctggccttttgctggccttttgctcacatgtatttaaataatgtatctaaacgcaaactccgagctggaaaaatgttaccggcgatgcgcggacaatttagaggcggcgatcaagaaacacctgctgggcgagcagtctggagcacagtcttcgatgggcccgagatcccaccgcgttcctgggtaccgggacgtgaggcagcgcgacatccatcaaatataccaggcgccaaccgagtgtctcggaaaacagcttctggatatcttccgctggcggcgcaacgacgaataatagtccctggaggtgacggaatatatatgtgtggagggtaaatctgacagggtgtagcaaaggtaatattttcctaaaacatgcaatcggctgccccgcaacgggaaaaagaatgactttggcactcttcaccagagtggggtgtcccgctcgtgtgtgcaaataggctcccactggtcaccccggattttgcagaaaaacagcaagttccggggtgtctcactggtgtccgccaataagaggagccggcaggcacggagtttacatcaagctgtctccgatacactcgactaccatccgggtctctcagagaggggaatggcactataaataccgcctccttgcgctctctgccttcatcaatcaaatcatgctgaggactcgaattccctaggatgatgagctttgtgcaaaaggggacctggttacttttcgctctgcttcatcccactgttattttggcacaacagtatccgtatgatgtgccggattatgcgtctccccagtacgaagcatatgatgtcaagtctggagtagcaggaggaggaatcgcaggctatcctgggccagctggtcctcctggcccacccggaccccctggcacatctggccatcctggtgcccctggcgctccaggataccaaggtccccccggtgaacctgggcaagctggtccggcaggtcctccaggacctcctggtgctataggtccatctggccctgctggaaaagatggggaatcaggaagacccggacgacctggagagcgaggatttcctggccctcctggtatgaaaggcccagctggtatgcctggattccctggtatgaaaggacacagaggctttgatggacgaaatggagagaaaggcgaaactggtgctcctggattaaagggggaaaatggcgttccaggtgaaaatggagctcctggacccatgggtccaagaggggctcccggtgagagaggacggccaggacttcctggagccgcaggggctcgaggtaatgatggagctcgaggaagtgatggacaaccgggcccccctggtcctcctggaactgcaggattccctggttcccctggtgctaagggtgaagttggacctgcaggatctcctggttcaagtggcgcccctggacaaagaggagaacctggacctcagggacatgctggtgctccaggtccccctgggcctcctgggagtaatggtagtcctggtggcaaaggtgaaatgggtcctgctggcattcctggggctcctgggctgataggagctcgtggtcctccagggccacctggcaccaatggtgttcccgggcaacgaggtgctgcaggtgaacccggtaagaatggagccaaaggagacccaggaccacgtggggaacgcggagaagctggttctccaggtatcgcaggacctaagggtgaagatggcaaagatggttctcctggagaacctggtgcaaatggacttcctggagctgcaggagaaaggggtgtgcctggattccgaggacctgctggagcaaatggccttccaggagaaaagggtcctcctggggaccgtggtggcccaggccctgcagggcccagaggtgttgctggagagcccggcagagatggtctccctggaggtccaggattgaggggtattcctggtagccccggaggaccaggcagtgatgggaaaccagggcctcctggaagccaaggagagacgggtcgacccggtcctccaggttcacctggtccgcgaggccagcctggtgtcatgggcttccctggtcccaaaggaaacgatggtgctcctggaaaaaatggagaacgaggtggccctggaggtcctggccctcagggtcctgctggaaagaatggtgagaccggacctcagggtcctccaggacctactggcccttctggtgacaaaggagacacaggaccccctggtccacaaggactacaaggcttgcctggaacgagtggtcccccaggagaaaacggaaaacctggtgaacctggtccaaagggtgaggctggtgcacctggaattccaggaggcaagggtgattctggtgctcccggtgaacgcggacctcctggagcaggagggccccctggacctagaggtggagctggcccccctggtcccgaaggaggaaagggtgctgctggtccccctgggccacctggttctgctggtacacctggtctgcaaggaatgcctggagaaagagggggtcctggaggccctggtccaaagggtgataagggtgagcctggcagctcaggtgtcgatggtgctccagggaaagatggtccacggggtcccactggtcccattggtcctcctggcccagctggtcagcctggagataagggtgaaagtggtgcccctggagttccgggtatagctggtcctcgcggtggccctggtgagagaggcgaacaggggcccccaggacctgctggcttccctggtgctcctggccagaatggtgagcctggtgctaaaggagaaagaggcgctcctggtgagaaaggtgaaggaggccctcccggagccgcaggacccgccggaggttctgggcctgccggtcccccaggcccccaaggtgtcaaaggcgaacgtggcagtcctggtggtcctggtgctgctggcttccccggtggtcgtggtcctcctggccctcctggcagtaatggtaacccaggccccccaggctccagtggtgctccaggcaaagatggtcccccaggtccacctggcagtaatggtgctcctggcagccccgggatctctggaccaaagggtgattctggtccaccaggtgagaggggagcacctggcccccagggccctccgggagctccaggcccactaggaattgcaggacttactggagcacgaggtcttgcaggcccaccaggcatgccaggtgctaggggcagccccggcccacagggcatcaagggtgaaaatggtaaaccaggacctagtggtcagaatggagaacgtggtcctcctggcccccagggtcttcctggtctggctggtacagctggtgagcctggaagagatggaaaccctggatcagatggtctgccaggccgagatggagctccaggtgccaagggtgaccgtggtgaaaatggctctcctggtgcccctggagctcctggtcacccaggccctcctggtcctgtcggtccagctggaaagagcggtgacagaggagaaactggccctgctggtccttctggggcccccggtcctgccggatcaagaggtcctcctggtccccaaggcccacgcggtgacaaaggggaaaccggtgagcgtggtgctatgggcatcaaaggacatcgcggattccctggcaacccaggggcccccggatctccgggtcccgctggtcatcaaggtgcagttggcagtccaggccctgcaggccccagaggacctgttggacctagcgggccccctggaaaggacggagcaagtggacaccctggtcccattggaccaccggggccccgaggtaacagaggtgaaagaggatctgagggctccccaggccacccaggacaaccaggccctcctggacctcctggtgcccctggtccatgttgtggtgctggcggggttgctgccattgctggtgttggagccgaaaaagctggtggttttgccccatattatggagctagcggttacattcctgaagctcctagagacggacaagcatacgttagaaaggacggtgagtgggtgttgctgtccaccttcttagctagcgattacaaggatgacgacgataagggatcgtgttgcccgggctgctgtcatcaccatcatcaccatagatcttaagcggccgcgagtcgtgagtaatcaagaggatgtcagaatgccatttgcctgagagatgcaggcttcatttttgatacttttttatttgtaacctatatagtataggattttttttgtcattttgtttcttctcgtacgagcttgctcctgatcagcctatctcgcagctgatgaatatcttgtggtaggggtttgggaaaatcattcgagtttgatgtttttcttggtatttcccactcctcttcagagtacagaagattaagtgagacgttcgtttgtgctccggaggatccttcagtaatgtcttgtttcttttgttgcagtggtgagccattttgacttcgtgaaagtttctttagaatagttgtttccagaggccaaacattccacccgtagtaaagtgcaagcgtaggaagaccaagactggcataaatcaggtataagtgtcgagcactggcaggtgatcttctgaaagtttctactagcagataagatccagtagtcatgcatatggcaacaatgtaccgtgtggatctaagaacgcgtcctactaaccttcgcattcgttggtccagtttgttgttatcgatcaacgtgacaaggttgtcgattccgcgtaagcatgcatacccaaggacgcctgttgcaattccaagtgagccagttccaacaatctttgtaatattagagcacttcattgtgttgcgcttgaaagtaaaatgcgaacaaattaagagataatctcgaaaccgcgacttcaaacgccaatatgatgtgcggcacacaataagcgttcatatccgctgggtgactttctcgctttaaaaaattatccgaaaaaattttctagagtgttgttactttatacttccggctcgtataatacgacaaggtgtaaggaggactaaaccatggctaaactcacctctgctgttccagtcctgactgctcgtgatgttgctggtgctgttgagttctggactgataggctcggtttctcccgtgacttcgtagaggacgactttgccggtgttgtacgtgacgacgttaccctgttcatctccgcagttcaggaccaggttgtgccagacaacactctggcatgggtatgggttcgtggtctggacgaactgtacgctgagtggtctgaggtcgtgtctaccaacttccgtgatgcatctggtccagctatgaccgagatcggtgaacagccctggggtcgtgagtttgcactgcgtgatccagctggtaactgcgtgcatttcgtcgcagaagagcaggactaacaattgacaccttacgattatttagagagtatttattagttttattgtatgtatacggatgttttattatctatttatgcccttatattctgtaactatccaaaagtcctatcttatcaagccagcaatctatgtccgcgaacgtcaactaaaaataagctttttatgctcttctctctttttttcccttcggtataattataccttgcatccacagattctcctgccaaattttgcataatcctttacaacatggctatatgggagcacttagcgccctccaaaacccatattgcctacgcatgtataggtgttttttccacaatattttctctgtgctctctttttattaaagagaagctctatatcggagaagcttctgtggccgttatattcggccttatcgtgggaccacattgcctgaattggtttgccccggaagattggggaaacttggatctgattaccttagctgcagaaaagggtaccactgagcgtcagaccccgtagaaaa

SEQ ID NO: 23 - DNA, 57 bp, Artificial Sequence
  alpha-factor Pre (Sequence 21)
atgagattcccatctattttcaccgctgtcttgttcgctgcctcctctgcattggct

SEQ ID NO: 24 - DNA, 267 bp, Artificial Sequence
  Alpha-factor Pre pro (Sequence 22)
atgagattcccatctattttcaccgctgtcttgttcgctgcctcctctgcattggctgcccctgttaacactaccactgaagacgagactgctcaaattccagctgaagcagttatcggttactctgaccttgagggtgatttcgacgtcgctgttttgcctttctctaactccactaacaacggtttgttgttcattaacaccactatcgcttccattgctgctaaggaagagggtgtctctctcgagaaaagagaggccgaagct

SEQ ID NO: 25 - DNA, 1298 bp, Artificial Sequence
  pGCW14-GAP1 bidirectional promoter (Sequence 23)
ttttgttgttgagtgaagcgagtgacggaacggtaaaatgtaagtaacaaaagaaaaagagaaccaggggggggaggagagtatgtatttataccgtacggcaccaggcgaaaagctataaacaaacctttttcgcggtatatttgtttatatttcctattttaaactcaaaatctgccctaatctggacttttcatgcaaagttatgcacctgaggcaggaatgaagcaggctcgacgacgaaaaggctggaatgggtaactatggatcgattgatttgtctgttgaaatcttgatttggcactcgtttaaattaacattctgcatcatggtgaattgcggtcacaggtactggtttttcctgaagctctaggcggtgttactgttcccacaacttaaaacctaaaagaggtgggtgcttctttgcgtgggtgaccaaaaataaaaccgactgcctagtggcattgatacctttttttgggtgttgtcctggaaaccactgaacgtatctgcgagatacaaaagtatttttagataagtggcaaatgcaaaaaatctgattggtcagttaatgattgatgaacgactttaaggttaaaaagcaaaatagtgactgctgccatgtgcctgtatagcacatgaactgattattctgttcccacgctacgatgaaaacgccttctctgccgaaagattaaagctgcgcgggaaaaaaaaattaactttacggggcgagcacggttccccgaaacaaaagatggttggctttcacccagcgagctcactggatcccagttaaaaatagttaggtgggttcacctgtttttgtagaaatgtcttggtgtcctcgaccaatcaggtagccatccctgaaatacctggctccgtggcaacaccgaacgacctgctggcaacgttaaattctccggggtaaaacttaaatgtggagtaatagaaccagaaacgtctcttcccttctctctccttccaccgcccgttaccgtccctaggaaattttactctgctggagagcttcttctacggcccccttgcagcaatgctcttcccagcattacgttgcgggtaaaacggaggtcgtgtacccgacctagcagcccagggatggaaagtcccggccgtcgctggcaataactgcgggcggacgcatgtcttgagattattggaaaccaccagaatcgaatataaaaggcgaacacctttcccaattttggtttctcctgacccaaagactttaaatttaatttatttgtccctatttcaatcaattgaacaactat

SEQ ID NO: 26 - DNA, 550 bp, Artificial Sequence
  pHTX1 bi-directional promoter (Sequence 25)
tgttgtagttttaatatagtttgagtatgagatggaactcagaacgaaggaattatcaccagtttatatattctgaggaaagggtgtgtcctaaattggacagtcacgatggcaataaacgctcagccaatcagaatgcaggagccataaattgttgtattattgctgcaagatttatgtgggttcacattccactgaatggttttcactgtagaattggtgtcctagttgttatgtttcgagatgttttcaagaaaaactaaaatgcacaaactgaccaataatgtgccgtcgcgcttggtacaaacgtcaggattgccaccacttttttcgcactctggtacaaaagttcgcacttcccactcgtatgtaacgaaaaacagagcagtctatccagaacgagacaaattagcgcgtactgtcccattccataaggtatcataggaaacgagagtcctccccccatcacgtatatataaacacactgatatcccacatccgcttgtcaccaaactaatacatccagttcaagttacctaaacaaatcaaa

SEQ ID NO: 27 - DNA, 1251 bp, Artificial Sequence
  Das1-Das2 bi-directional promoter (Sequence 24)
ttttgatgtttgatagtttgataagagtgaactttagtgtttagaggggttataatttgttgtaactggttttggtcttaagttaaaacgaacttgttatattaaacacaacggtcactcaggatacaagaataggaaagaaaaactttaaactggggacatgttgtctttatataatttggcggttaacccttaatgcccgtttccgtctcttcatgataacaaagctgcccatctatgactgaatgtggagaagtatcggaacaacccttcactaaggatatctaggctaaactcattcgcgccttagatttctccaaggtatcggttaagtttcctctttcgtactggctaacgatggtgttgctcaacaaagggatggaacggcagctaaagggagtgcatggaatgactttaattggctgagaaagtgttctatttgtccgaatttcttttttctattatctgttcgtttgggcggatctctccagtggggggtaaatggaagatttctgttcatggggtaaggaagctgaaatccttcgtttcttataggggcaagtatactaaatctcggaacattgaatggggtttactttcattggctacagaaattattaagtttgttatggggtgaagttaccagtaattttcattttttcacttcaacttttggggtatttctgtggggtagcatagagcaatgatataaacaacaattgagtgacaggtctactttgttctcaaaaggccataaccatctgtttgcatctcttatcaccacaccatcctcctcatctggccttcaattgtggggaacaactagcatcccaacaccagactaactccacccagatgaaaccagttgtcgcttaccagtcaatgaatgttgagctaacgttccttgaaactcgaatgatcccagccttgctgcgtatcatccctccgctattccgccgcttgctccaaccatgtttccgcctttttcgaacaagttcaaatacctatctttggcaggacttttcctcctgccttttttagcctcagctctcggttagcctctaggcaaattctggtcttcatacctatatcaacttttcatcagatagcctttgggttcaaaaaagaactaaagcaggatgcctgatatataaatcccagatgatctgcttttgaaactattttcagtatcttgattcgtttacttacaaacaactattgttgattttatctggagaataatcgaacaaa

SEQ ID NO: 28 - DNA, 3908 bp, Artificial Sequence
  MMV132
ggatccttcagtaatgtcttgtttcttttgttgcagtggtgagccattttgacttcgtgaaagtttctttagaatagttgtttccagaggccaaacattccacccgtagtaaagtgcaagcgtaggaagaccaagactggcataaatcaggtataagtgtcgagcactggcaggtgatcttctgaaagtttctactagcagataagatccagtagtcatgcatatggcaacaatgtaccgtgtggatctaagaacgcgtcctactaaccttcgcattcgttggtccagtttgttgttatcgatcaacgtgacaaggttgtcgattccgcgtaagcatgcatacccaaggacgcctgttgcaattccaagtgagccagttccaacaatctttgtaatattagagcacttcattgtgttgcgcttgaaagtaaaatgcgaacaaattaagagataatctcgaaaccgcgacttcaaacgccaatatgatgtgcggcacacaataagcgttcatatccgctgggtgactttctcgctttaaaaaattatccgaaaaaattttctagagtgttgttactttatacttccggctcgtataatacgacaaggtgtaaggaggactaaaccatggctaaactcacctctgctgttccagtcctgactgctcgtgatgttgctggtgctgttgagttctggactgataggctcggtttctcccgtgacttcgtagaggacgactttgccggtgttgtacgtgacgacgttaccctgttcatctccgcagttcaggaccaggttgtgccagacaacactctggcatgggtatgggttcgtggtctggacgaactgtacgctgagtggtctgaggtcgtgtctaccaacttccgtgatgcatctggtccagctatgaccgagatcggtgaacagccctggggtcgtgagtttgcactgcgtgatccagctggtaactgcgtgcatttcgtcgcagaagagcaggactaacaattgacaccttacgattatttagagagtatttattagttttattgtatgtatacggatgttttattatctatttatgcccttatattctgtaactatccaaaagtcctatcttatcaagccagcaatctatgtccgcgaacgtcaactaaaaataagctttttatgctcttctctctttttttcccttcggtataattataccttgcatccacagattctcctgccaaattttgcataatcctttacaacatggctatatgggagcacttagcgccctccaaaacccatattgcctacgcatgtataggtgttttttccacaatattttctctgtgctctctttttattaaagagaagctctatatcggagaagcttctgtggccgttatattcggccttatcgtgggaccacattgcctgaattggtttgccccggaagattggggaaacttggatctgattaccttagctgcagaaaagggtaccactgagcgtcagaccccgtagaaaagatcaaaggatcttcttgagatcctttttttctgcgcgtaatctgctgcttgcaaacaaaaaaaccaccgctaccagcggtggtttgtttgccggatcaagagctaccaactctttttccgaaggtaactggcttcagcagagcgcagataccaaatactgttcttctagtgtagccgtagttaggccaccacttcaagaactctgtagcaccgcctacatacctcgctctgctaatcctgttaccagtggctgctgccagtggcgataagtcgtgtcttaccgggttggacccaagacgatagttaccggataaggcgcagcggtcgggctgaacggggggttcgtgcacacagcccagcttggagcgaacgacctacaccgaactgagatacctacagcgtgagctatgagaaagcgccacgcttcccgaagggagaaaggcggacaggtatccggtaagcggcagggtcggaacaggagagcgcacgagggagcttccagggggaaacgcctggtatctttatagtcctgtcgggtttcgccacctctgacttgagcgtcgatttttgtgatgctcgtcaggggggcggagcctatggaaaaacgccagcaacgcggcctttttacggttcctggccttttgctggccttttgctcacatgtatttaaataatgtatctaaacgcaaactccgagctggaaaaatgttaccggcgatgcgcggacaatttagaggcggcgatcaagaaacacctgctgggcgagcagtctggagcacagtcttcgatgggcccgagatcccaccgcgttcctgggtaccgggacgtgaggcagcgcgacatccatcaaatataccaggcgccaaccgagtgtctcggaaaacagcttctggatatcttccgctggcggcgcaacgacgaataatagtccctggaggtgacggaatatatatgtgtggagggtaaatctgacagggtgtagcaaaggtaatattttcctaaaacatgcaatcggctgccccgcaacgggaaaaagaatgactttggcactcttcaccagagtggggtgtcccgctcgtgtgtgcaaataggctcccactggtcaccccggattttgcagaaaaacagcaagttccggggtgtctcactggtgtccgccaataagaggagccggcaggcacggagtttacatcaagctgtctccgatacactcgactaccatccgggtctctcagagaggggaatggcactataaataccgcctccttgcgctctctgccttcatcaatcaaatcatgctgaggactcgaattcgacctctgttgcctctttgttggacgaaccattcaccggtgtcttgtacttaaagggcagtggtatcactgaagacttccagtccctaaagggtaagaagatcggttacgttggtgacttcggtaagatccaaatcgatgaattgaccaagcactacggtatgaagccagaagactacaccgccgtcagatgtggtatgaatgtcgccaagtacatcatcgaaggtaagattgatgccggtattggtatcgaatgtatgcaacaagtcgaattggaagagtacttggccaagcaaggcagaccagcttctgatgctaaaatgttgagaattgacaagttggcttgcttgggttgctgttgcttctgtaccgttctttacatctgcaacgatgaatttttgaagaagaaccctgaaaaggtcagaaagttcttgaaagccatcaagaaggcaaccgactacgttctagccgaccctgtgaaggcttggaaagaatacatcgacttcaagcctcaattgaacaacgatctatcctacaagcaataccaaagatgttacgcttacttctcttcatctttgtacaatgttcaccgtgactggaagaaggttaccggttacggtaagagattagccatcttgccaccagactatgtctcgaactacactaatgaatacttgtcctggccagaaccagaagaggtttctgatcctttggaagctcaaagattgatggctattcatcaagaaaaatgcagacaggaaggtactttcaagagattggctcttccagcttaagcggccgcgagtcgtgagtaatcaagaggatgtcagaatgccatttgcctgagagatgcaggcttcatttttgatacttttttatttgtaacctatatagtataggattttttttgtcattttgtttcttctcgtacgagcttgctcctgatcagcctatctcgcagctgatgaatatcttgtggtaggggtttgggaaaatcattcgagtttgatgtttttcttggtatttcccactcctcttcagagtacagaagattaagtgagacgttcgtttgtgctccgga

SEQ ID NO: 29 - DNA, 7476 bp, Artificial Sequence
  MMV193
ccgtagaaaagatcaaaggatcttcttgagatcctttttttctgcgcgtaatctgctgcttgcaaacaaaaaaaccaccgctaccagcggtggtttgtttgccggatcaagagctaccaactctttttccgaaggtaactggcttcagcagagcgcagataccaaatactgttcttctagtgtagccgtagttaggccaccacttcaagaactctgtagcaccgcctacatacctcgctctgctaatcctgttaccagtggctgctgccagtggcgataagtcgtgtcttaccgggttggacccaagacgatagttaccggataaggcgcagcggtcgggctgaacggggggttcgtgcacacagcccagcttggagcgaacgacctacaccgaactgagatacctacagcgtgagctatgagaaagcgccacgcttcccgaagggagaaaggcggacaggtatccggtaagcggcagggtcggaacaggagagcgcacgagggagcttccagggggaaacgcctggtatctttatagtcctgtcgggtttcgccacctctgacttgagcgtcgatttttgtgatgctcgtcaggggggcggagcctatggaaaaacgccagcaacgcggcctttttacggttcctggccttttgctggccttttgctcacatgtatttaaataatgtatctaaacgcaaactccgagctggaaaaatgttaccggcgatgcgcggacaatttagaggcggcgatcaagaaacacctgctgggcgagcagtctggagcacagtcttcgatgggcccgagatcccaccgcgttcctgggtaccgggacgtgaggcagcgcgacatccatcaaatataccaggcgccaaccgagtgtctcggaaaacagcttctggatatcttccgctggcggcgcaacgacgaataatagtccctggaggtgacggaatatatatgtgtggagggtaaatctgacagggtgtagcaaaggtaatattttcctaaaacatgcaatcggctgccccgcaacgggaaaaagaatgactttggcactcttcaccagagtggggtgtcccgctcgtgtgtgcaaataggctcccactggtcaccccggattttgcagaaaaacagcaagttccggggtgtctcactggtgtccgccaataagaggagccggcaggcacggagtttacatcaagctgtctccgatacactcgactaccatccgggtctctcagagaggggaatggcactataaataccgcctccttgcgctctctgccttcatcaatcaaatcatgatgtcttttgtccaaaagggtacttggttactttttgctctgttgcacccaactgttattctcgcacaacaggaagcagtagatggtggttgctcacatttaggtcaatcttacgcagatagagatgtatggaaacctgaaccatgtcaaatttgcgtgtgtgactcaggttcagtgctctgcgacgatatcatatgtgacgaccaggaattggactgtccaaacccagagataccattcggtgaatgttgtgctgtttgtccacagccaccaactgctcctacaagacctccaaacggtcaaggtccacaaggtcctaaaggtgatccgggtccacctggtattcctggtagaaatggtgaccctggacctcccggttccccaggtagcccaggatcacctgggcctcctggaatatgtgaatcctgcccaactggtggtcagaactatagcccacaatacgaggcctacgacgtcaaatctggtgttgctggaggaggtattgcaggctaccctggtcccgcagggcccccaggtccgccgggtccgcccggaacatcaggtcatcccggagcccctggtgcaccaggttatcagggaccgcccggagagcctggacaagctggtcccgctggaccccctggtccaccaggtgctattggaccaagtggtcctgccggaaaagacggtgaatccggtagacctggtagacccggcgaaaggggtttcccaggtcctcccggaatgaagggtccagccggtatgcccggttttcctgggatgaagggtcacagaggatttgatggtagaaacggagagaaaggcgaaaccggtgctcccggactgaagggtgaaaacggtgtccctggtgagaacggcgctcctggacctatgggtccacgtggtgctccaggagaaagaggcagaccaggattgcctggtgcagctggtgctagaggtaacgatggtgcccgtggttccgatggacaacccgggccacccggccctccaggtaccgctggatttcctggaagccctggtgctaagggggaggttggtccggctggtagtcccggaagtagcggtgccccaggtcaaagaggcgaaccaggccctcagggtcacgcaggagcacctggaccgcctggtcctcctggttcgaatggttcgcctggaggaaaaggtgaaatggggcccgcaggaatccccggtgcgcctggtcttattggtgccaggggtcctccaggcccgccaggtacaaatggtgtacccggacagcgaggagcagctggtgaacctggtaaaaacggtgccaaaggagatccaggtcctcgtggagagcgtggtgaagctggctctcccggtatcgccggtccaaaaggtgaggacggtaaggacggttcccctggtgagccaggtgcgaacggactgccaggtgcagccggagagcgaggagtcccaggattcaggggaccagccggtgctaacggcttgcctggtgaaaaagggccccctggtgataggggaggacccggtccagcaggccctcgtggagttgctggtgagcctggacgtgacggtttaccaggagggccaggtttgaggggtattcccgggtcccctggcggtcctggatcggatggaaaaccagggccaccaggttcgcagggtgaaacaggacgtccaggcccacccggctcacctggtccaaggggtcagcctggtgtcatgggtttccccggtccaaagggtaatgacggagcaccgggtaaaaatggtgaacgtggtggcccaggtggtccaggaccccaaggtccagctggaaaaaacggtgagacaggtcctcaaggacctccaggacctaccggtcctagcggagataagggagatacgggaccgccaggacctcaaggattgcaaggtttgcctggtacatctggccctcccggagaaaatggtaagcctggagagccaggaccaaaaggcgaagctggagccccaggtatccccggaggtaagggagactcaggtgctccgggtgagcgtggtcctccgggtgccggtggtccacctggacctagaggtggtgccgggccgccaggtcctgaaggtggtaaaggtgctgctggtccccctgggccacctggttctgctggtacacctggtctgcaaggaatgcctggagaaagagggggtcctggaggccctggtccaaagggtgataagggtgagcctggcagctcaggtgtcgatggtgctccagggaaagatggtccacggggtcccactggtcccattggtcctcctggcccagctggtcagcctggagataagggtgaaagtggtgcccctggagttccgggtatagctggtcctcgcggtggccctggtgagagaggcgaacaggggcccccaggacctgctggcttccctggtgctcctggccagaatggtgagcctggtgctaaaggagaaagaggcgctcctggtgagaaaggtgaaggaggccctcccggagccgcaggacccgccggaggttctgggcctgccggtcccccaggcccccaaggtgtcaaaggcgaacgtggcagtcctggtggtcctggtgctgctggcttccccggtggtcgtggtcctcctggccctcctggcagtaatggtaacccaggccccccaggctccagtggtgctccaggcaaagatggtcccccaggtccacctggcagtaatggtgctcctggcagccccgggatctctggaccaaagggtgattctggtccaccaggtgagaggggagcacctggcccccagggccctccgggagctccaggcccactaggaattgcaggacttactggagcacgaggtcttgcaggcccaccaggcatgccaggtgctaggggcagccccggcccacagggcatcaagggtgaaaatggtaaaccaggacctagtggtcagaatggagaacgtggtcctcctggcccccagggtcttcctggtctggctggtacagctggtgagcctggaagagatggaaaccctggatcagatggtctgccaggccgagatggagctccaggtgccaagggtgaccgtggtgaaaatggctctcctggtgcccctggagctcctggtcacccaggccctcctggtcctgtcggtccagctggaaagagcggtgacagaggagaaactggccctgctggtccttctggggcccccggtcctgccggatcaagaggtcctcctggtccccaaggcccacgcggtgacaaaggggaaaccggtgagcgtggtgctatgggcatcaaaggacatcgcggattccctggcaacccaggggcccccggatctccgggtcccgctggtcatcaaggtgcagttggcagtccaggccctgcaggccccagaggacctgttggacctagcgggccccctggaaaggacggagcaagtggacaccctggtcccattggaccaccggggccccgaggtaacagaggtgaaagaggatctgagggctccccaggccacccaggacaaccaggccctcctggacctcctggtgcccctggtccatgttgtggtgctggcggggttgctgccattgctggtgttggagccgaaaaagctggtggttttgccccatattatggagatgaaccgatagatttcaaaatcaacaccgatgagattatgacctcactcaaatcagtcaatggacaaatagaaagcctcattagtcctgatggttcccgtaaaaaccctgcacggaactgcagggacctgaaattctgccatcctgaactccagagtggagaatattgggttgatcctaaccaaggttgcaaattggatgctattaaagtctactgtaacatggaaactggggaaacgtgcataagtgccagtcctttgactatcccacagaagaactggtggacagattctggtgctgagaagaaacatgtttggtttggagaatccatggagggtggttttcagtttagctatggcaatcctgaacttcccgaagacgtcctcgatgtccagctggcattcctccgacttctctccagccgggcctctcagaacatcacatatcactgcaagaatagcattgcatacatggatcatgccagtgggaatgtaaagaaagccttgaagctgatggggtcaaatgaaggtgaattcaaggctgaaggaaatagcaaattcacatacacagttctggaggatggttgcacaaaacacactggggaatggggcaaaacagtcttccagtatcaaacacgcaaggccgtcagactacctattgtagatattgcaccctatgatatcggtggtcctgatcaagaatttggtgcggacattggccctgtttgctttttataatcaagaggatgtcagaatgccatttgcctgagagatgcaggcttcatttttgatacttttttatttgtaacctatatagtataggattttttttgtcattttgtttcttctcgtacgagcttgctcctgatcagcctatctcgcagctgatgaatatcttgtggtaggggtttgggaaaatcattcgagtttgatgtttttcttggtatttcccactcctcttcagagtacagaagattaagtgagacgttcgtttgtgctccggaggatccttcagtaatgtcttgtttcttttgttgcagtggtgagccattttgacttcgtgaaagtttctttagaatagttgtttccagaggccaaacattccacccgtagtaaagtgcaagcgtaggaagaccaagactggcataaatcaggtataagtgtcgagcactggcaggtgatcttctgaaagtttctactagcagataagatccagtagtcatgcatatggcaacaatgtaccgtgtggatctaagaacgcgtcctactaaccttcgcattcgttggtccagtttgttgttatcgatcaacgtgacaaggttgtcgattccgcgtaagcatgcatacccaaggacgcctgttgcaattccaagtgagccagttccaacaatctttgtaatattagagcacttcattgtgttgcgcttgaaagtaaaatgcgaacaaattaagagataatctcgaaaccgcgacttcaaacgccaatatgatgtgcggcacacaataagcgttcatatccgctgggtgactttctcgctttaaaaaattatccgaaaaaattttctagagtgttgttactttatacttccggctcgtataatacgacaaggtgtaaggaggactaaaccatggctaaactcacctctgctgttccagtcctgactgctcgtgatgttgctggtgctgttgagttctggactgataggctcggtttctcccgtgacttcgtagaggacgactttgccggtgttgtacgtgacgacgttaccctgttcatctccgcagttcaggaccaggttgtgccagacaacactctggcatgggtatgggttcgtggtctggacgaactgtacgctgagtggtctgaggtcgtgtctaccaacttccgtgatgcatctggtccagctatgaccgagatcggtgaacagccctggggtcgtgagtttgcactgcgtgatccagctggtaactgcgtgcatttcgtcgcagaagagcaggactaacaattgacaccttacgattatttagagagtatttattagttttattgtatgtatacggatgttttattatctatttatgcccttatattctgtaactatccaaaagtcctatcttatcaagccagcaatctatgtccgcgaacgtcaactaaaaataagctttttatgctcttctctctttttttcccttcggtataattataccttgcatccacagattctcctgccaaattttgcataatcctttacaacatggctatatgggagcacttagcgccctccaaaacccatattgcctacgcatgtataggtgttttttccacaatattttctctgtgctctctttttattaaagagaagctctatatcggagaagcttctgtggccgttatattcggccttatcgtgggaccacattgcctgaattggtttgccccggaagattggggaaacttggatctgattaccttagctgcagaaaagggtaccactgagcgtcagacc

SEQ ID NO: 30 - DNA, 7476 bp, Artificial Sequence
  MMV 194
acgcatgtataggtgttttttccacaatattttctctgtgctctctttttattaaagagaagctctatatcggagaagcttctgtggccgttatattcggccttatcgtgggaccacattgcctgaattggtttgccccggaagattggggaaacttggatctgattaccttagctgcagaaaagggtaccactgagcgtcagaccccgtagaaaagatcaaaggatcttcttgagatcctttttttctgcgcgtaatctgctgcttgcaaacaaaaaaaccaccgctaccagcggtggtttgtttgccggatcaagagctaccaactctttttccgaaggtaactggcttcagcagagcgcagataccaaatactgttcttctagtgtagccgtagttaggccaccacttcaagaactctgtagcaccgcctacatacctcgctctgctaatcctgttaccagtggctgctgccagtggcgataagtcgtgtcttaccgggttggacccaagacgatagttaccggataaggcgcagcggtcgggctgaacggggggttcgtgcacacagcccagcttggagcgaacgacctacaccgaactgagatacctacagcgtgagctatgagaaagcgccacgcttcccgaagggagaaaggcggacaggtatccggtaagcggcagggtcggaacaggagagcgcacgagggagcttccagggggaaacgcctggtatctttatagtcctgtcgggtttcgccacctctgacttgagcgtcgatttttgtgatgctcgtcaggggggcggagcctatggaaaaacgccagcaacgcggcctttttacggttcctggccttttgctggccttttgctcacatgtatttaaataatgtatctaaacgcaaactccgagctggaaaaatgttaccggcgatgcgcggacaatttagaggcggcgatcaagaaacacctgctgggcgagcagtctggagcacagtcttcgatgggcccgagatcccaccgcgttcctgggtaccgggacgtgaggcagcgcgacatccatcaaatataccaggcgccaaccgagtgtctcggaaaacagcttctggatatcttccgctggcggcgcaacgacgaataatagtccctggaggtgacggaatatatatgtgtggagggtaaatctgacagggtgtagcaaaggtaatattttcctaaaacatgcaatcggctgccccgcaacgggaaaaagaatgactttggcactcttcaccagagtggggtgtcccgctcgtgtgtgcaaataggctcccactggtcaccccggattttgcagaaaaacagcaagttccggggtgtctcactggtgtccgccaataagaggagccggcaggcacggagtttacatcaagctgtctccgatacactcgactaccatccgggtctctcagagaggggaatggcactataaataccgcctccttgcgctctctgccttcatcaatcaaatcatgatgtcttttgtccaaaagggtacttggttactttttgctctgttgcacccaactgttattctcgcacaacaggaagcagtagatggtggttgctcacatttaggtcaatcttacgcagatagagatgtatggaaacctgaaccatgtcaaatttgcgtgtgtgactcaggttcagtgctctgcgacgatatcatatgtgacgaccaggaattggactgtccaaacccagagataccattcggtgaatgttgtgctgtttgtccacagccaccaactgctcctacaagacctccaaacggtcaaggtccacaaggtcctaaaggtgatccgggtccacctggtattcctggtagaaatggtgaccctggacctcccggttccccaggtagcccaggatcacctgggcctcctggaatatgtgaatcctgcccaactggtggtcagaactatagcccacaatacgaggcctacgacgtcaaatctggtgttgctggaggaggtattgcaggctaccctggtcccgcagggcccccaggtccgccgggtccgcccggaacatcaggtcatcccggagcccctggtgcaccaggttatcagggaccgcccggagagcctggacaagctggtcccgctggaccccctggtccaccaggtgctattggaccaagtggtcctgccggaaaagacggtgaatccggtagacctggtagacccggcgaaaggggtttcccaggtcctcccggaatgaagggtccagccggtatgcccggttttcctgggatgaagggtcacagaggatttgatggtagaaacggagagaaaggcgaaaccggtgctcccggactgaagggtgaaaacggtgtccctggtgagaacggcgctcctggacctatgggtccacgtggtgctccaggagaaagaggcagaccaggattgcctggtgcagctggtgctagaggtaacgatggtgcccgtggttccgatggacaacccgggccacccggccctccaggtaccgctggatttcctggaagccctggtgctaagggggaggttggtccggctggtagtcccggaagtagcggtgccccaggtcaaagaggcgaaccaggccctcagggtcacgcaggagcacctggaccgcctggtcctcctggttcgaatggttcgcctggaggaaaaggtgaaatggggcccgcaggaatccccggtgcgcctggtcttattggtgccaggggtcctccaggcccgccaggtacaaatggtgtacccggacagcgaggagcagctggtgaacctggtaaaaacggtgccaaaggagatccaggtcctcgtggagagcgtggtgaagctggctctcccggtatcgccggtccaaaaggtgaggacggtaaggacggttcccctggtgagccaggtgcgaacggactgccaggtgcagccggagagcgaggagtcccaggattcaggggaccagccggtgctaacggcttgcctggtgaaaaagggccccctggtgataggggaggacccggtccagcaggccctcgtggagttgctggtgagcctggacgtgacggtttaccaggagggccaggtttgaggggtattcccgggtcccctggcggtcctggatcggatggaaaaccagggccaccaggttcgcagggtgaaacaggacgtccaggcccacccggctcacctggtccaaggggtcagcctggtgtcatgggtttccccggtccaaagggtaatgacggagcaccgggtaaaaatggtgaacgtggtggcccaggtggtccaggaccccaaggtccagctggaaaaaacggtgagacaggtcctcaaggacctccaggacctaccggtcctagcggagataagggagatacgggaccgccaggacctcaaggattgcaaggtttgcctggtacatctggccctcccggagaaaatggtaagcctggagagccaggaccaaaaggcgaagctggagccccaggtatccccggaggtaagggagactcaggtgctccgggtgagcgtggtcctccgggtgccggtggtccacctggacctagaggtggtgccgggccgccaggtcctgaaggtggtaaaggtgctgctggtccaccgggaccgcctggctctgctggtactcctggcttgcagggaatgccaggagagagaggtggacctggaggtcccggtccgaagggtgataaaggggagccaggatcatccggtgttgacggcgcacctggtaaagacggaccaaggggaccaacgggtccaatcggaccaccaggacccgctggccagccaggagataaaggcgagtccggagcacccggtgttcctggtatagctggacccaggggtggtcccggtgaaagaggtgaacagggcccaccgggtcccgccggtttccctggcgcccctggtcaaaatggagaaccaggtgcaaagggcgagagaggagccccaggagaaaagggtgagggaggaccacccggtgctgccggtccagctgggggttcaggtcctgctggaccaccaggtccacagggcgttaaaggtgagagaggaagtccaggtggtcctggagctgctggattcccaggtggccgtggacctcctggtccccctggatcgaatggtaatcctggtccgccaggtagttcgggtgctcctgggaaggacggtccacctggccccccaggtagtaacggtgcacctggtagtccaggtatatccggacctaaaggagattccggtccaccaggcgaaagaggggccccaggcccacagggtccaccaggagcccccggtcctctgggtattgctggtcttactggtgcacgtggactggccggtccacccggaatgcctggagcaagaggttcacctggaccacaaggtattaaaggagagaacggtaaacctggaccttccggtcaaaacggagagcggggacccccaggcccccaaggtctgccaggactagctggtaccgcaggggaaccaggaagagatggaaatccaggttcagacggactacccggtagagatggtgcaccgggggccaagggcgacaggggtgagaatggatctcctggtgcgccaggggcaccaggccacccaggtcccccaggtcctgtgggccctgctggaaagtcaggtgacaggggagagacaggcccggctggtccatctggcgcacccggaccagctggttccagaggcccacctggtccgcaaggccctagaggtgacaagggagagactggagaacgaggtgctatgggtatcaagggtcatagaggttttccgggtaatcccggcgccccaggttctcctggtccagctggccatcaaggtgcagtcggatcgcccggcccagccggtcccaggggccctgttggtccatccggtcctccaggaaaggatggtgcttctggacacccaggacctatcggacctccgggtcctagaggtaatagaggagaacgtggatccgagggtagtcctggtcaccctggtcaacctggcccaccagggcctccaggtgcacccggtccatgttgtggtgcaggcggggttgctgccattgctggtgttggagccgaaaaagctggtggttttgccccatattatggagatgaaccgatagatttcaaaatcaacaccgatgagattatgacctcactcaaatcagtcaatggacaaatagaaagcctcattagtcctgatggttcccgtaaaaaccctgcacggaactgcagggacctgaaattctgccatcctgaactccagagtggagaatattgggttgatcctaaccaaggttgcaaattggatgctattaaagtctactgtaacatggaaactggggaaacgtgcataagtgccagtcctttgactatcccacagaagaactggtggacagattctggtgctgagaagaaacatgtttggtttggagaatccatggagggtggttttcagtttagctatggcaatcctgaacttcccgaagacgtcctcgatgtccagctggcattcctccgacttctctccagccgggcctctcagaacatcacatatcactgcaagaatagcattgcatacatggatcatgccagtgggaatgtaaagaaagccttgaagctgatggggtcaaatgaaggtgaattcaaggctgaaggaaatagcaaattcacatacacagttctggaggatggttgcacaaaacacactggggaatggggcaaaacagtcttccagtatcaaacacgcaaggccgtcagactacctattgtagatattgcaccctatgatatcggtggtcctgatcaagaatttggtgcggacattggccctgtttgctttttataatcaagaggatgtcagaatgccatttgcctgagagatgcaggcttcatttttgatacttttttatttgtaacctatatagtataggattttttttgtcattttgtttcttctcgtacgagcttgctcctgatcagcctatctcgcagctgatgaatatcttgtggtaggggtttgggaaaatcattcgagtttgatgtttttcttggtatttcccactcctcttcagagtacagaagattaagtgagacgttcgtttgtgctccggaggatccttcagtaatgtcttgtttcttttgttgcagtggtgagccattttgacttcgtgaaagtttctttagaatagttgtttccagaggccaaacattccacccgtagtaaagtgcaagcgtaggaagaccaagactggcataaatcaggtataagtgtcgagcactggcaggtgatcttctgaaagtttctactagcagataagatccagtagtcatgcatatggcaacaatgtaccgtgtggatctaagaacgcgtcctactaaccttcgcattcgttggtccagtttgttgttatcgatcaacgtgacaaggttgtcgattccgcgtaagcatgcatacccaaggacgcctgttgcaattccaagtgagccagttccaacaatctttgtaatattagagcacttcattgtgttgcgcttgaaagtaaaatgcgaacaaattaagagataatctcgaaaccgcgacttcaaacgccaatatgatgtgcggcacacaataagcgttcatatccgctgggtgactttctcgctttaaaaaattatccgaaaaaattttctagagtgttgttactttatacttccggctcgtataatacgacaaggtgtaaggaggactaaaccatggctaaactcacctctgctgttccagtcctgactgctcgtgatgttgctggtgctgttgagttctggactgataggctcggtttctcccgtgacttcgtagaggacgactttgccggtgttgtacgtgacgacgttaccctgttcatctccgcagttcaggaccaggttgtgccagacaacactctggcatgggtatgggttcgtggtctggacgaactgtacgctgagtggtctgaggtcgtgtctaccaacttccgtgatgcatctggtccagctatgaccgagatcggtgaacagccctggggtcgtgagtttgcactgcgtgatccagctggtaactgcgtgcatttcgtcgcagaagagcaggactaacaattgacaccttacgattatttagagagtatttattagttttattgtatgtatacggatgttttattatctatttatgcccttatattctgtaactatccaaaagtcctatcttatcaagccagcaatctatgtccgcgaacgtcaactaaaaataagctttttatgctcttctctctttttttcccttcggtataattataccttgcatccacagattctcctgccaaattttgcataatcctttacaacatggctatatgggagcacttagcgccctccaaaacccatattgcct

SEQ ID NO: 31 - DNA, 7476 bp, Artificial Sequence
  MMV 195
cgcatgtataggtgttttttccacaatattttctctgtgctctctttttattaaagagaagctctatatcggagaagcttctgtggccgttatattcggccttatcgtgggaccacattgcctgaattggtttgccccggaagattggggaaacttggatctgattaccttagctgcagaaaagggtaccactgagcgtcagaccccgtagaaaagatcaaaggatcttcttgagatcctttttttctgcgcgtaatctgctgcttgcaaacaaaaaaaccaccgctaccagcggtggtttgtttgccggatcaagagctaccaactctttttccgaaggtaactggcttcagcagagcgcagataccaaatactgttcttctagtgtagccgtagttaggccaccacttcaagaactctgtagcaccgcctacatacctcgctctgctaatcctgttaccagtggctgctgccagtggcgataagtcgtgtcttaccgggttggacccaagacgatagttaccggataaggcgcagcggtcgggctgaacggggggttcgtgcacacagcccagcttggagcgaacgacctacaccgaactgagatacctacagcgtgagctatgagaaagcgccacgcttcccgaagggagaaaggcggacaggtatccggtaagcggcagggtcggaacaggagagcgcacgagggagcttccagggggaaacgcctggtatctttatagtcctgtcgggtttcgccacctctgacttgagcgtcgatttttgtgatgctcgtcaggggggcggagcctatggaaaaacgccagcaacgcggcctttttacggttcctggccttttgctggccttttgctcacatgtatttaaataatgtatctaaacgcaaactccgagctggaaaaatgttaccggcgatgcgcggacaatttagaggcggcgatcaagaaacacctgctgggcgagcagtctggagcacagtcttcgatgggcccgagatcccaccgcgttcctgggtaccgggacgtgaggcagcgcgacatccatcaaatataccaggcgccaaccgagtgtctcggaaaacagcttctggatatcttccgctggcggcgcaacgacgaataatagtccctggaggtgacggaatatatatgtgtggagggtaaatctgacagggtgtagcaaaggtaatattttcctaaaacatgcaatcggctgccccgcaacgggaaaaagaatgactttggcactcttcaccagagtggggtgtcccgctcgtgtgtgcaaataggctcccactggtcaccccggattttgcagaaaaacagcaagttccggggtgtctcactggtgtccgccaataagaggagccggcaggcacggagtttacatcaagctgtctccgatacactcgactaccatccgggtctctcagagaggggaatggcactataaataccgcctccttgcgctctctgccttcatcaatcaaatcatgatgtcttttgtccaaaagggtacttggttactttttgctctgttgcacccaactgttattctcgcacaacaggaagcagtagatggtggttgctcacatttaggtcaatcttacgcagatagagatgtatggaaacctgaaccatgtcaaatttgcgtgtgtgactcaggttcagtgctctgcgacgatatcatatgtgacgaccaggaattggactgtccaaacccagagataccattcggtgaatgttgtgctgtttgtccacagccaccaactgctcctacaagacctccaaacggtcaaggtccacaaggtcctaaaggtgatccgggtccacctggtattcctggtagaaatggtgaccctggacctcccggttccccaggtagcccaggatcacctgggcctcctggaatatgtgaatcctgcccaactggtggtcagaactatagcccacaatacgaggcctacgacgtcaaatctggtgttgctggaggaggtattgcaggctaccctggtcccgcagggcccccaggtccgccgggtccgcccggaacatcaggtcatcccggagcccctggtgcaccaggttatcagggaccgcccggagagcctggacaagctggtcccgctggaccccctggtccaccaggtgctattggaccaagtggtcctgccggaaaagacggtgaatccggtagacctggtagacccggcgaaaggggtttcccaggtcctcccggaatgaagggtccagccggtatgcccggttttcctgggatgaagggtcacagaggatttgatggtagaaacggagagaaaggcgaaaccggtgctcccggactgaagggtgaaaacggtgtccctggtgagaacggcgctcctggacctatgggtccacgtggtgctccaggagaaagaggcagaccaggattgcctggtgcagctggtgctagaggtaacgatggtgcccgtggttccgatggacaacccgggccacccggccctccaggtaccgctggatttcctggaagccctggtgctaagggggaggttggtccggctggtagtcccggaagtagcggtgccccaggtcaaagaggcgaaccaggccctcagggtcacgcaggagcacctggaccgcctggtcctcctggttcgaatggttcgcctggaggaaaaggtgaaatggggcccgcaggaatccccggtgcgcctggtcttattggtgccaggggtcctccaggcccgccaggtacaaatggtgtacccggacagcgaggagcagctggtgaacctggtaaaaacggtgccaaaggagatccaggtcctcgtggagagcgtggtgaagctggctctcccggtatcgccggtccaaaaggtgaggacggtaaggacggttcccctggtgagccaggtgcgaacggactgccaggtgcagccggagagcgaggagtcccaggattcaggggaccagccggtgctaacggcttgcctggtgaaaaagggccccctggtgataggggaggacccggtccagcaggccctcgtggagttgctggtgagcctggacgtgacggtttaccaggagggccaggtttgaggggtattcccgggtcccctggcggtcctggatcggatggaaaaccagggccaccaggttcgcagggtgaaacaggacgtccaggcccacccggctcacctggtccaaggggtcagcctggtgtcatgggtttccccggtccaaagggtaatgacggagcaccgggtaaaaatggtgaacgtggtggcccaggtggtccaggaccccaaggtccagctggaaaaaacggtgagacaggtcctcaaggacctccaggacctaccggtcctagcggagataagggagatacgggaccgccaggacctcaaggattgcaaggtttgcctggtacatctggccctcccggagaaaatggtaagcctggagagccaggaccaaaaggcgaagctggagccccaggtatccccggaggtaagggagactcaggtgctccgggtgagcgtggtcctccgggtgccggtggtccacctggacctagaggtggtgccgggccgccaggtcctgaaggtggtaaaggtgctgctggtccaccgggaccgcctggctctgctggtactcctggcttgcagggaatgccaggagagagaggtggacctggaggtcccggtccgaagggtgataaaggggagccaggatcatccggtgttgacggcgcacctggtaaagacggaccaaggggaccaacgggtccaatcggaccaccaggacccgctggccagccaggagataaaggcgagtccggagcacccggtgttcctggtatagctggacccaggggtggtcccggtgaaagaggtgaacagggcccaccgggtcccgccggtttccctggcgcccctggtcaaaatggagaaccaggtgcaaagggcgagagaggagccccaggagaaaagggtgagggaggaccacccggtgctgccggtccagctgggggttcaggtcctgctggaccaccaggtccacagggcgttaaaggtgagagaggaagtccaggtggtcctggagctgctggattcccaggtggccgtggacctcctggtccccctggatcgaatggtaatcctggtccgccaggtagttcgggtgctcctgggaaggacggtccacctggccccccaggtagtaacggtgcacctggtagtccaggtatatccggacctaaaggagattccggtccaccaggcgaaagaggggccccaggcccacagggtccaccaggagcccccggtcctctgggtattgctggtcttactggtgcacgtggactggccggtccacccggaatgcctggagcaagaggttcacctggaccacaaggtattaaaggagagaacggtaaacctggaccttccggtcaaaacggagagcggggacccccaggcccccaaggtctgccaggactagctggtaccgcaggggaaccaggaagagatggaaatccaggttcagacggactacccggtagagatggtgcaccgggggccaagggcgacaggggtgagaatggatctcctggtgcgccaggggcaccaggccacccaggtcccccaggtcctgtgggccctgctggaaagtcaggtgacaggggagagacaggcccggctggtccatctggcgcacccggaccagctggttccagaggcccacctggtccgcaaggccctagaggtgacaagggagagactggagaacgaggtgctatgggtatcaagggtcatagaggttttccgggtaatcccggcgccccaggttctcctggtccagctggccatcaaggtgcagtcggatcgcccggcccagccggtcccaggggccctgttggtccatccggtcctccaggaaaggatggtgcttctggacacccaggacctatcggacctccgggtcctagaggtaatagaggagaacgtggatccgagggtagtcctggtcaccctggtcaacctggcccaccagggcctccaggtgcacccggtccatgttgtggtgcaggcggtgtggctgcaattgctggtgtgggtgctgaaaaggccggcggtttcgctccatattatggtgatgaaccgattgattttaagatcaatactgacgaaatcatgacttccttaaagtccgttaatggtcaaattgagtctctaatctccccagatggttcacgtaaaaatcctgctagaaattgtagagatttgaagttttgtcaccccgagttgcagtccggtgagtactgggtggaccccaatcaaggttgtaagttagacgctattaaagtttactgcaatatggagacaggagaaacttgcatcagcgcttctccattgactatcccacaaaaaaattggtggactgactctggagctgagaaaaagcatgtatggttcggggaatcgatggagggtggttttcagtttagctatggcaatcctgaacttcccgaagacgtcctcgatgtccagctggcattcctccgacttctctccagccgggcctctcagaacatcacatatcactgcaagaatagcattgcatacatggatcatgccagtgggaatgtaaagaaagccttgaagctgatggggtcaaatgaaggtgaattcaaggctgaaggaaatagcaaattcacatacacagttctggaggatggttgcacaaaacacactggggaatggggcaaaacagtcttccagtatcaaacacgcaaggccgtcagactacctattgtagatattgcaccctatgatatcggtggtcctgatcaagaatttggtgcggacattggccctgtttgctttttataatcaagaggatgtcagaatgccatttgcctgagagatgcaggcttcatttttgatacttttttatttgtaacctatatagtataggattttttttgtcattttgtttcttctcgtacgagcttgctcctgatcagcctatctcgcagctgatgaatatcttgtggtaggggtttgggaaaatcattcgagtttgatgtttttcttggtatttcccactcctcttcagagtacagaagattaagtgagacgttcgtttgtgctccggaggatccttcagtaatgtcttgtttcttttgttgcagtggtgagccattttgacttcgtgaaagtttctttagaatagttgtttccagaggccaaacattccacccgtagtaaagtgcaagcgtaggaagaccaagactggcataaatcaggtataagtgtcgagcactggcaggtgatcttctgaaagtttctactagcagataagatccagtagtcatgcatatggcaacaatgtaccgtgtggatctaagaacgcgtcctactaaccttcgcattcgttggtccagtttgttgttatcgatcaacgtgacaaggttgtcgattccgcgtaagcatgcatacccaaggacgcctgttgcaattccaagtgagccagttccaacaatctttgtaatattagagcacttcattgtgttgcgcttgaaagtaaaatgcgaacaaattaagagataatctcgaaaccgcgacttcaaacgccaatatgatgtgcggcacacaataagcgttcatatccgctgggtgactttctcgctttaaaaaattatccgaaaaaattttctagagtgttgttactttatacttccggctcgtataatacgacaaggtgtaaggaggactaaaccatggctaaactcacctctgctgttccagtcctgactgctcgtgatgttgctggtgctgttgagttctggactgataggctcggtttctcccgtgacttcgtagaggacgactttgccggtgttgtacgtgacgacgttaccctgttcatctccgcagttcaggaccaggttgtgccagacaacactctggcatgggtatgggttcgtggtctggacgaactgtacgctgagtggtctgaggtcgtgtctaccaacttccgtgatgcatctggtccagctatgaccgagatcggtgaacagccctggggtcgtgagtttgcactgcgtgatccagctggtaactgcgtgcatttcgtcgcagaagagcaggactaacaattgacaccttacgattatttagagagtatttattagttttattgtatgtatacggatgttttattatctatttatgcccttatattctgtaactatccaaaagtcctatcttatcaagccagcaatctatgtccgcgaacgtcaactaaaaataagctttttatgctcttctctctttttttcccttcggtataattataccttgcatccacagattctcctgccaaattttgcataatcctttacaacatggctatatgggagcacttagcgccctccaaaacccatattgccta

SEQ ID NO: 32 - DNA, 7479 bp, Artificial Sequence
  MMV197
aaggggagccaggatcatccggtgttgacggcgcacctggtaaagacggaccaaggggaccaacgggtccaatcggaccaccaggacccgctggccagccaggagataaaggcgagtccggagcacccggtgttcctggtatagctggacccaggggtggtcccggtgaaagaggtgaacagggcccaccgggtcccgccggtttccctggcgcccctggtcaaaatggagaaccaggtgcaaagggcgagagaggagccccaggagaaaagggtgagggaggaccacccggtgctgccggtccagctgggggttcaggtcctgctggaccaccaggtccacagggcgttaaaggtgagagaggaagtccaggtggtcctggagctgctggattcccaggtggccgtggacctcctggtccccctggatcgaatggtaatcctggtccgccaggtagttcgggtgctcctgggaaggacggtccacctggccccccaggtagtaacggtgcacctggtagtccaggtatatccggacctaaaggagattccggtccaccaggcgaaagaggggccccaggcccacagggtccaccaggagcccccggtcctctgggtattgctggtcttactggtgcacgtggactggccggtccacccggaatgcctggagcaagaggttcacctggaccacaaggtattaaaggagagaacggtaaacctggaccttccggtcaaaacggagagcggggacccccaggcccccaaggtctgccaggactagctggtaccgcaggggaaccaggaagagatggaaatccaggttcagacggactacccggtagagatggtgcaccgggggccaagggcgacaggggtgagaatggatctcctggtgcgccaggggcaccaggccacccaggtcccccaggtcctgtgggccctgctggaaagtcaggtgacaggggagagacaggcccggctggtccatctggcgcacccggaccagctggttccagaggcccacctggtccgcaaggccctagaggtgacaagggagagactggagaacgaggtgctatgggtatcaagggtcatagaggttttccgggtaatcccggcgccccaggttctcctggtccagctggccatcaaggtgcagtcggatcgcccggcccagccggtcccaggggccctgttggtccatccggtcctccaggaaaggatggtgcttctggacacccaggacctatcggacctccgggtcctagaggtaatagaggagaacgtggatccgagggtagtcctggtcaccctggtcaacctggcccaccagggcctccaggtgcacccggtccatgttgtggtgcaggcggtgtggctgcaattgctggtgtgggtgctgaaaaggccggcggtttcgctccatattatggtgatgaaccgattgattttaagatcaatactgacgaaatcatgacttccttaaagtccgttaatggtcaaattgagtctctaatctccccagatggttcacgtaaaaatcctgctagaaattgtagagatttgaagttttgtcaccccgagttgcagtccggtgagtactgggtggaccccaatcaaggttgtaagttagacgctattaaagtttactgcaatatggagacaggagaaacttgcatcagcgcttctccattgactatcccacaaaaaaattggtggactgactctggagctgagaaaaagcatgtatggttcggggaatcgatggaaggtggtttccaattcagctacggtaaccctgaacttcctgaagatgttcttgacgttcaattggcatttctgagattgttgtccagtcgtgcaagccaaaacattacataccattgcaaaaattccatcgcatatatggatcatgctagcggaaatgtgaaaaaggcattgaagctgatgggatcaaatgaaggtgaatttaaagcagagggtaattctaagtttacttacactgtattggaggatggttgtacgaagcatacaggtgaatggggtaaaacagtgtttcaatatcaaacccgcaaagcagttagattgccaatcgtcgatatcgcaccatacgacattggaggaccagatcaagagttcggagctgacatcggtccggtgtgtttcctttgataatcaagaggatgtcagaatgccatttgcctgagagatgcaggcttcatttttgatacttttttatttgtaacctatatagtataggattttttttgtcattttgtttcttctcgtacgagcttgctcctgatcagcctatctcgcagctgatgaatatcttgtggtaggggtttgggaaaatcattcgagtttgatgtttttcttggtatttcccactcctcttcagagtacagaagattaagtgagacgttcgtttgtgctccggaggatccttcagtaatgtcttgtttcttttgttgcagtggtgagccattttgacttcgtgaaagtttctttagaatagttgtttccagaggccaaacattccacccgtagtaaagtgcaagcgtaggaagaccaagactggcataaatcaggtataagtgtcgagcactggcaggtgatcttctgaaagtttctactagcagataagatccagtagtcatgcatatggcaacaatgtaccgtgtggatctaagaacgcgtcctactaaccttcgcattcgttggtccagtttgttgttatcgatcaacgtgacaaggttgtcgattccgcgtaagcatgcatacccaaggacgcctgttgcaattccaagtgagccagttccaacaatctttgtaatattagagcacttcattgtgttgcgcttgaaagtaaaatgcgaacaaattaagagataatctcgaaaccgcgacttcaaacgccaatatgatgtgcggcacacaataagcgttcatatccgctgggtgactttctcgctttaaaaaattatccgaaaaaattttctagagtgttgttactttatacttccggctcgtataatacgacaaggtgtaaggaggactaaaccatggctaaactcacctctgctgttccagtcctgactgctcgtgatgttgctggtgctgttgagttctggactgataggctcggtttctcccgtgacttcgtagaggacgactttgccggtgttgtacgtgacgacgttaccctgttcatctccgcagttcaggaccaggttgtgccagacaacactctggcatgggtatgggttcgtggtctggacgaactgtacgctgagtggtctgaggtcgtgtctaccaacttccgtgatgcatctggtccagctatgaccgagatcggtgaacagccctggggtcgtgagtttgcactgcgtgatccagctggtaactgcgtgcatttcgtcgcagaagagcaggactaacaattgacaccttacgattatttagagagtatttattagttttattgtatgtatacggatgttttattatctatttatgcccttatattctgtaactatccaaaagtcctatcttatcaagccagcaatctatgtccgcgaacgtcaactaaaaataagctttttatgctcttctctctttttttcccttcggtataattataccttgcatccacagattctcctgccaaattttgcataatcctttacaacatggctatatgggagcacttagcgccctccaaaacccatattgcctacgcatgtataggtgttttttccacaatattttctctgtgctctctttttattaaagagaagctctatatcggagaagcttctgtggccgttatattcggccttatcgtgggaccacattgcctgaattggtttgccccggaagattggggaaacttggatctgattaccttagctgcagaaaagggtaccactgagcgtcagaccccgtagaaaagatcaaaggatcttcttgagatcctttttttctgcgcgtaatctgctgcttgcaaacaaaaaaaccaccgctaccagcggtggtttgtttgccggatcaagagctaccaactctttttccgaaggtaactggcttcagcagagcgcagataccaaatactgttcttctagtgtagccgtagttaggccaccacttcaagaactctgtagcaccgcctacatacctcgctctgctaatcctgttaccagtggctgctgccagtggcgataagtcgtgtcttaccgggttggacccaagacgatagttaccggataaggcgcagcggtcgggctgaacggggggttcgtgcacacagcccagcttggagcgaacgacctacaccgaactgagatacctacagcgtgagctatgagaaagcgccacgcttcccgaagggagaaaggcggacaggtatccggtaagcggcagggtcggaacaggagagcgcacgagggagcttccagggggaaacgcctggtatctttatagtcctgtcgggtttcgccacctctgacttgagcgtcgatttttgtgatgctcgtcaggggggcggagcctatggaaaaacgccagcaacgcggcctttttacggttcctggccttttgctggccttttgctcacatgtatttaaataatgtatctaaacgcaaactccgagctggaaaaatgttaccggcgatgcgcggacaatttagaggcggcgatcaagaaacacctgctgggcgagcagtctggagcacagtcttcgatgggcccgagatcccaccgcgttcctgggtaccgggacgtgaggcagcgcgacatccatcaaatataccaggcgccaaccgagtgtctcggaaaacagcttctggatatcttccgctggcggcgcaacgacgaataatagtccctggaggtgacggaatatatatgtgtggagggtaaatctgacagggtgtagcaaaggtaatattttcctaaaacatgcaatcggctgccccgcaacgggaaaaagaatgactttggcactcttcaccagagtggggtgtcccgctcgtgtgtgcaaataggctcccactggtcaccccggattttgcagaaaaacagcaagttccggggtgtctcactggtgtccgccaataagaggagccggcaggcacggagtttacatcaagctgtctccgatacactcgactaccatccgggtctctcagagaggggaatggcactataaataccgcctccttgcgctctctgccttcatcaatcaaatcatgatgagctttgtgcaaaaggggacctggttacttttcgctctgcttcatcccactgttattttggcacaacaggaagctgttgacggaggatgctcccatctcggtcagtcttatgcagatagagatgtatggaaaccagaaccgtgccaaatatgcgtctgtgactcaggatccgttctctgtgatgacataatatgtgacgaccaagaattagactgccccaaccctgaaatcccgtttggagaatgttgtgcagtttgcccacagcctccaacagctcccactcgccctcctaatggtcaaggacctcaaggccccaagggagatccaggtcctcctggtattcctgggcgaaatggcgatcctggtcctccaggatcaccaggctccccaggttctcccggccctcctggaatctgtgaatcatgtcctactggtggccagaactattctccccagtacgaagcatatgatgtcaagtctggagtagcaggaggaggaatcgcaggctatcctgggccagctggtcctcctggcccacccggaccccctggcacatctggccatcctggtgcccctggcgctccaggataccaaggtccccccggtgaacctgggcaagctggtccggcaggtcctccaggacctcctggtgctataggtccatctggccctgctggaaaagatggggaatcaggaagacccggacgacctggagagcgaggatttcctggccctcctggtatgaaaggcccagctggtatgcctggattccctggtatgaaaggacacagaggctttgatggacgaaatggagagaaaggcgaaactggtgctcctggattaaagggggaaaatggcgttccaggtgaaaatggagctcctggacccatgggtccaagaggggctcccggtgagagaggacggccaggacttcctggagccgcaggggctcgaggtaatgatggagctcgaggaagtgatggacaaccgggcccccctggtcctcctggaactgcaggattccctggttcccctggtgctaagggtgaagttggacctgcaggatctcctggttcaagtggcgcccctggacaaagaggagaacctggacctcagggacatgctggtgctccaggtccccctgggcctcctgggagtaatggtagtcctggtggcaaaggtgaaatgggtcctgctggcattcctggggctcctgggctgataggagctcgtggtcctccagggccacctggcaccaatggtgttcccgggcaacgaggtgctgcaggtgaacccggtaagaatggagccaaaggagacccaggaccacgtggggaacgcggagaagctggttctccaggtatcgcaggacctaagggtgaagatggcaaagatggttctcctggagaacctggtgcaaatggacttcctggagctgcaggagaaaggggtgtgcctggattccgaggacctgctggagcaaatggccttccaggagaaaagggtcctcctggggaccgtggtggcccaggccctgcagggcccagaggtgttgctggagagcccggcagagatggtctccctggaggtccaggattgaggggtattcctggtagccccggaggaccaggcagtgatgggaaaccagggcctcctggaagccaaggagagacgggtcgacccggtcctccaggttcacctggtccgcgaggccagcctggtgtcatgggcttccctggtcccaaaggaaacgatggtgctcctggaaaaaatggagaacgaggtggccctggaggtcctggccctcagggtcctgctggaaagaatggtgagaccggacctcagggtcctccaggacctactggcccttctggtgacaaaggagacacaggaccccctggtccacaaggactacaaggcttgcctggaacgagtggtcccccaggagaaaacggaaaacctggtgaacctggtccaaagggtgaggctggtgcacctggaattccaggaggcaagggtgattctggtgctcccggtgaacgcggacctcctggagcaggagggccccctggacctagaggtggagctggcccccctggtcccgaaggaggaaagggtgctgctggtccaccgggaccgcctggctctgctggtactcctggcttgcagggaatgccaggagagagaggtggacctggaggtcccggtccgaagggtgata

SEQ ID NO: 33 - DNA, 7479 bp, Artificial Sequence
  MMV198
tccgccaataagaggagccggcaggcacggagtttacatcaagctgtctccgatacactcgactaccatccgggtctctcagagaggggaatggcactataaataccgcctccttgcgctctctgccttcatcaatcaaatcatgatgagctttgtgcaaaaggggacctggttacttttcgctctgcttcatcccactgttattttggcacaacaggaagctgttgacggaggatgctcccatctcggtcagtcttatgcagatagagatgtatggaaaccagaaccgtgccaaatatgcgtctgtgactcaggatccgttctctgtgatgacataatatgtgacgaccaagaattagactgccccaaccctgaaatcccgtttggagaatgttgtgcagtttgcccacagcctccaacagctcccactcgccctcctaatggtcaaggacctcaaggccccaagggagatccaggtcctcctggtattcctgggcgaaatggcgatcctggtcctccaggatcaccaggctccccaggttctcccggccctcctggaatctgtgaatcatgtcctactggtggccagaactattctccccagtacgaagcatatgatgtcaagtctggagtagcaggaggaggaatcgcaggctatcctgggccagctggtcctcctggcccacccggaccccctggcacatctggccatcctggtgcccctggcgctccaggataccaaggtccccccggtgaacctgggcaagctggtccggcaggtcctccaggacctcctggtgctataggtccatctggccctgctggaaaagatggggaatcaggaagacccggacgacctggagagcgaggatttcctggccctcctggtatgaaaggcccagctggtatgcctggattccctggtatgaaaggacacagaggctttgatggacgaaatggagagaaaggcgaaactggtgctcctggattaaagggggaaaatggcgttccaggtgaaaatggagctcctggacccatgggtccaagaggggctcccggtgagagaggacggccaggacttcctggagccgcaggggctcgaggtaatgatggagctcgaggaagtgatggacaaccgggcccccctggtcctcctggaactgcaggattccctggttcccctggtgctaagggtgaagttggacctgcaggatctcctggttcaagtggcgcccctggacaaagaggagaacctggacctcagggacatgctggtgctccaggtccccctgggcctcctgggagtaatggtagtcctggtggcaaaggtgaaatgggtcctgctggcattcctggggctcctgggctgataggagctcgtggtcctccagggccacctggcaccaatggtgttcccgggcaacgaggtgctgcaggtgaacccggtaagaatggagccaaaggagacccaggaccacgtggggaacgcggagaagctggttctccaggtatcgcaggacctaagggtgaagatggcaaagatggttctcctggagaacctggtgcaaatggacttcctggagctgcaggagaaaggggtgtgcctggattccgaggacctgctggagcaaatggccttccaggagaaaagggtcctcctggggaccgtggtggcccaggccctgcagggcccagaggtgttgctggagagcccggcagagatggtctccctggaggtccaggattgaggggtattcctggtagccccggaggaccaggcagtgatgggaaaccagggcctcctggaagccaaggagagacgggtcgacccggtcctccaggttcacctggtccgcgaggccagcctggtgtcatgggcttccctggtcccaaaggaaacgatggtgctcctggaaaaaatggagaacgaggtggccctggaggtcctggccctcagggtcctgctggaaagaatggtgagaccggacctcagggtcctccaggacctactggcccttctggtgacaaaggagacacaggaccccctggtccacaaggactacaaggcttgcctggaacgagtggtcccccaggagaaaacggaaaacctggtgaacctggtccaaagggtgaggctggtgcacctggaattccaggaggcaagggtgattctggtgctcccggtgaacgcggacctcctggagcaggagggccccctggacctagaggtggagctggcccccctggtcccgaaggaggaaagggtgctgctggtccccctgggccacctggttctgctggtacacctggtctgcaaggaatgcctggagaaagagggggtcctggaggccctggtccaaagggtgataagggtgagcctggcagctcaggtgtcgatggtgctccagggaaagatggtccacggggtcccactggtcccattggtcctcctggcccagctggtcagcctggagataagggtgaaagtggtgcccctggagttccgggtatagctggtcctcgcggtggccctggtgagagaggcgaacaggggcccccaggacctgctggcttccctggtgctcctggccagaatggtgagcctggtgctaaaggagaaagaggcgctcctggtgagaaaggtgaaggaggccctcccggagccgcaggacccgccggaggttctgggcctgccggtcccccaggcccccaaggtgtcaaaggcgaacgtggcagtcctggtggtcctggtgctgctggcttccccggtggtcgtggtcctcctggccctcctggcagtaatggtaacccaggccccccaggctccagtggtgctccaggcaaagatggtcccccaggtccacctggcagtaatggtgctcctggcagccccgggatctctggaccaaagggtgattctggtccaccaggtgagaggggagcacctggcccccagggccctccgggagctccaggcccactaggaattgcaggacttactggagcacgaggtcttgcaggcccaccaggcatgccaggtgctaggggcagccccggcccacagggcatcaagggtgaaaatggtaaaccaggacctagtggtcagaatggagaacgtggtcctcctggcccccagggtcttcctggtctggctggtacagctggtgagcctggaagagatggaaaccctggatcagatggtctgccaggccgagatggagctccaggtgccaagggtgaccgtggtgaaaatggctctcctggtgcccctggagctcctggtcacccaggccctcctggtcctgtcggtccagctggaaagagcggtgacagaggagaaactggccctgctggtccttctggggcccccggtcctgccggatcaagaggtcctcctggtccccaaggcccacgcggtgacaaaggggaaaccggtgagcgtggtgctatgggcatcaaaggacatcgcggattccctggcaacccaggggcccccggatctccgggtcccgctggtcatcaaggtgcagttggcagtccaggccctgcaggccccagaggacctgttggacctagcgggccccctggaaaggacggagcaagtggacaccctggtcccattggaccaccggggccccgaggtaacagaggtgaaagaggatctgagggctccccaggccacccaggacaaccaggccctcctggacctcctggtgcccctggtccatgttgtggtgctggcggtgtggctgcaattgctggtgtgggtgctgaaaaggccggcggtttcgctccatattatggtgatgaaccgattgattttaagatcaatactgacgaaatcatgacttccttaaagtccgttaatggtcaaattgagtctctaatctccccagatggttcacgtaaaaatcctgctagaaattgtagagatttgaagttttgtcaccccgagttgcagtccggtgagtactgggtggaccccaatcaaggttgtaagttagacgctattaaagtttactgcaatatggagacaggagaaacttgcatcagcgcttctccattgactatcccacaaaaaaattggtggactgactctggagctgagaaaaagcatgtatggttcggggaatcgatggaaggtggtttccaattcagctacggtaaccctgaacttcctgaagatgttcttgacgttcaattggcatttctgagattgttgtccagtcgtgcaagccaaaacattacataccattgcaaaaattccatcgcatatatggatcatgctagcggaaatgtgaaaaaggcattgaagctgatgggatcaaatgaaggtgaatttaaagcagagggtaattctaagtttacttacactgtattggaggatggttgtacgaagcatacaggtgaatggggtaaaacagtgtttcaatatcaaacccgcaaagcagttagattgccaatcgtcgatatcgcaccatacgacattggaggaccagatcaagagttcggagctgacatcggtccggtgtgtttcctttgataatcaagaggatgtcagaatgccatttgcctgagagatgcaggcttcatttttgatacttttttatttgtaacctatatagtataggattttttttgtcattttgtttcttctcgtacgagcttgctcctgatcagcctatctcgcagctgatgaatatcttgtggtaggggtttgggaaaatcattcgagtttgatgtttttcttggtatttcccactcctcttcagagtacagaagattaagtgagacgttcgtttgtgctccggaggatccttcagtaatgtcttgtttcttttgttgcagtggtgagccattttgacttcgtgaaagtttctttagaatagttgtttccagaggccaaacattccacccgtagtaaagtgcaagcgtaggaagaccaagactggcataaatcaggtataagtgtcgagcactggcaggtgatcttctgaaagtttctactagcagataagatccagtagtcatgcatatggcaacaatgtaccgtgtggatctaagaacgcgtcctactaaccttcgcattcgttggtccagtttgttgttatcgatcaacgtgacaaggttgtcgattccgcgtaagcatgcatacccaaggacgcctgttgcaattccaagtgagccagttccaacaatctttgtaatattagagcacttcattgtgttgcgcttgaaagtaaaatgcgaacaaattaagagataatctcgaaaccgcgacttcaaacgccaatatgatgtgcggcacacaataagcgttcatatccgctgggtgactttctcgctttaaaaaattatccgaaaaaattttctagagtgttgttactttatacttccggctcgtataatacgacaaggtgtaaggaggactaaaccatggctaaactcacctctgctgttccagtcctgactgctcgtgatgttgctggtgctgttgagttctggactgataggctcggtttctcccgtgacttcgtagaggacgactttgccggtgttgtacgtgacgacgttaccctgttcatctccgcagttcaggaccaggttgtgccagacaacactctggcatgggtatgggttcgtggtctggacgaactgtacgctgagtggtctgaggtcgtgtctaccaacttccgtgatgcatctggtccagctatgaccgagatcggtgaacagccctggggtcgtgagtttgcactgcgtgatccagctggtaactgcgtgcatttcgtcgcagaagagcaggactaacaattgacaccttacgattatttagagagtatttattagttttattgtatgtatacggatgttttattatctatttatgcccttatattctgtaactatccaaaagtcctatcttatcaagccagcaatctatgtccgcgaacgtcaactaaaaataagctttttatgctcttctctctttttttcccttcggtataattataccttgcatccacagattctcctgccaaattttgcataatcctttacaacatggctatatgggagcacttagcgccctccaaaacccatattgcctacgcatgtataggtgttttttccacaatattttctctgtgctctctttttattaaagagaagctctatatcggagaagcttctgtggccgttatattcggccttatcgtgggaccacattgcctgaattggtttgccccggaagattggggaaacttggatctgattaccttagctgcagaaaagggtaccactgagcgtcagaccccgtagaaaagatcaaaggatcttcttgagatcctttttttctgcgcgtaatctgctgcttgcaaacaaaaaaaccaccgctaccagcggtggtttgtttgccggatcaagagctaccaactctttttccgaaggtaactggcttcagcagagcgcagataccaaatactgttcttctagtgtagccgtagttaggccaccacttcaagaactctgtagcaccgcctacatacctcgctctgctaatcctgttaccagtggctgctgccagtggcgataagtcgtgtcttaccgggttggacccaagacgatagttaccggataaggcgcagcggtcgggctgaacggggggttcgtgcacacagcccagcttggagcgaacgacctacaccgaactgagatacctacagcgtgagctatgagaaagcgccacgcttcccgaagggagaaaggcggacaggtatccggtaagcggcagggtcggaacaggagagcgcacgagggagcttccagggggaaacgcctggtatctttatagtcctgtcgggtttcgccacctctgacttgagcgtcgatttttgtgatgctcgtcaggggggcggagcctatggaaaaacgccagcaacgcggcctttttacggttcctggccttttgctggccttttgctcacatgtatttaaataatgtatctaaacgcaaactccgagctggaaaaatgttaccggcgatgcgcggacaatttagaggcggcgatcaagaaacacctgctgggcgagcagtctggagcacagtcttcgatgggcccgagatcccaccgcgttcctgggtaccgggacgtgaggcagcgcgacatccatcaaatataccaggcgccaaccgagtgtctcggaaaacagcttctggatatcttccgctggcggcgcaacgacgaataatagtccctggaggtgacggaatatatatgtgtggagggtaaatctgacagggtgtagcaaaggtaatattttcctaaaacatgcaatcggctgccccgcaacgggaaaaagaatgactttggcactcttcaccagagtggggtgtcccgctcgtgtgtgcaaataggctcccactggtcaccccggattttgcagaaaaacagcaagttccggggtgtctcactggtg

SEQ ID NO: 34 - DNA, 7479 bp, Artificial Sequence
  MMV199
gcatgtataggtgttttttccacaatattttctctgtgctctctttttattaaagagaagctctatatcggagaagcttctgtggccgttatattcggccttatcgtgggaccacattgcctgaattggtttgccccggaagattggggaaacttggatctgattaccttagctgcagaaaagggtaccactgagcgtcagaccccgtagaaaagatcaaaggatcttcttgagatcctttttttctgcgcgtaatctgctgcttgcaaacaaaaaaaccaccgctaccagcggtggtttgtttgccggatcaagagctaccaactctttttccgaaggtaactggcttcagcagagcgcagataccaaatactgttcttctagtgtagccgtagttaggccaccacttcaagaactctgtagcaccgcctacatacctcgctctgctaatcctgttaccagtggctgctgccagtggcgataagtcgtgtcttaccgggttggacccaagacgatagttaccggataaggcgcagcggtcgggctgaacggggggttcgtgcacacagcccagcttggagcgaacgacctacaccgaactgagatacctacagcgtgagctatgagaaagcgccacgcttcccgaagggagaaaggcggacaggtatccggtaagcggcagggtcggaacaggagagcgcacgagggagcttccagggggaaacgcctggtatctttatagtcctgtcgggtttcgccacctctgacttgagcgtcgatttttgtgatgctcgtcaggggggcggagcctatggaaaaacgccagcaacgcggcctttttacggttcctggccttttgctggccttttgctcacatgtatttaaataatgtatctaaacgcaaactccgagctggaaaaatgttaccggcgatgcgcggacaatttagaggcggcgatcaagaaacacctgctgggcgagcagtctggagcacagtcttcgatgggcccgagatcccaccgcgttcctgggtaccgggacgtgaggcagcgcgacatccatcaaatataccaggcgccaaccgagtgtctcggaaaacagcttctggatatcttccgctggcggcgcaacgacgaataatagtccctggaggtgacggaatatatatgtgtggagggtaaatctgacagggtgtagcaaaggtaatattttcctaaaacatgcaatcggctgccccgcaacgggaaaaagaatgactttggcactcttcaccagagtggggtgtcccgctcgtgtgtgcaaataggctcccactggtcaccccggattttgcagaaaaacagcaagttccggggtgtctcactggtgtccgccaataagaggagccggcaggcacggagtttacatcaagctgtctccgatacactcgactaccatccgggtctctcagagaggggaatggcactataaataccgcctccttgcgctctctgccttcatcaatcaaatcatgatgagctttgtgcaaaaggggacctggttacttttcgctctgcttcatcccactgttattttggcacaacaggaagctgttgacggaggatgctcccatctcggtcagtcttatgcagatagagatgtatggaaaccagaaccgtgccaaatatgcgtctgtgactcaggatccgttctctgtgatgacataatatgtgacgaccaagaattagactgccccaaccctgaaatcccgtttggagaatgttgtgcagtttgcccacagcctccaacagctcccactcgccctcctaatggtcaaggacctcaaggccccaagggagatccaggtcctcctggtattcctgggcgaaatggcgatcctggtcctccaggatcaccaggctccccaggttctcccggccctcctggaatctgtgaatcatgtcctactggtggccagaactattctccccagtacgaagcatatgatgtcaagtctggagtagcaggaggaggaatcgcaggctatcctgggccagctggtcctcctggcccacccggaccccctggcacatctggccatcctggtgcccctggcgctccaggataccaaggtccccccggtgaacctgggcaagctggtccggcaggtcctccaggacctcctggtgctataggtccatctggccctgctggaaaagatggggaatcaggaagacccggacgacctggagagcgaggatttcctggccctcctggtatgaaaggcccagctggtatgcctggattccctggtatgaaaggacacagaggctttgatggacgaaatggagagaaaggcgaaactggtgctcctggattaaagggggaaaatggcgttccaggtgaaaatggagctcctggacccatgggtccaagaggggctcccggtgagagaggacggccaggacttcctggagccgcaggggctcgaggtaatgatggagctcgaggaagtgatggacaaccgggcccccctggtcctcctggaactgcaggattccctggttcccctggtgctaagggtgaagttggacctgcaggatctcctggttcaagtggcgcccctggacaaagaggagaacctggacctcagggacatgctggtgctccaggtccccctgggcctcctgggagtaatggtagtcctggtggcaaaggtgaaatgggtcctgctggcattcctggggctcctgggctgataggagctcgtggtcctccagggccacctggcaccaatggtgttcccgggcaacgaggtgctgcaggtgaacccggtaagaatggagccaaaggagacccaggaccacgtggggaacgcggagaagctggttctccaggtatcgcaggacctaagggtgaagatggcaaagatggttctcctggagaacctggtgcaaatggacttcctggagctgcaggagaaaggggtgtgcctggattccgaggacctgctggagcaaatggccttccaggagaaaagggtcctcctggggaccgtggtggcccaggccctgcagggcccagaggtgttgctggagagcccggcagagatggtctccctggaggtccaggattgaggggtattcctggtagccccggaggaccaggcagtgatgggaaaccagggcctcctggaagccaaggagagacgggtcgacccggtcctccaggttcacctggtccgcgaggccagcctggtgtcatgggcttccctggtcccaaaggaaacgatggtgctcctggaaaaaatggagaacgaggtggccctggaggtcctggccctcagggtcctgctggaaagaatggtgagaccggacctcagggtcctccaggacctactggcccttctggtgacaaaggagacacaggaccccctggtccacaaggactacaaggcttgcctggaacgagtggtcccccaggagaaaacggaaaacctggtgaacctggtccaaagggtgaggctggtgcacctggaattccaggaggcaagggtgattctggtgctcccggtgaacgcggacctcctggagcaggagggccccctggacctagaggtggagctggcccccctggtcccgaaggaggaaagggtgctgctggtccccctgggccacctggttctgctggtacacctggtctgcaaggaatgcctggagaaagagggggtcctggaggccctggtccaaagggtgataagggtgagcctggcagctcaggtgtcgatggtgctccagggaaagatggtccacggggtcccactggtcccattggtcctcctggcccagctggtcagcctggagataagggtgaaagtggtgcccctggagttccgggtatagctggtcctcgcggtggccctggtgagagaggcgaacaggggcccccaggacctgctggcttccctggtgctcctggccagaatggtgagcctggtgctaaaggagaaagaggcgctcctggtgagaaaggtgaaggaggccctcccggagccgcaggacccgccggaggttctgggcctgccggtcccccaggcccccaaggtgtcaaaggcgaacgtggcagtcctggtggtcctggtgctgctggcttccccggtggtcgtggtcctcctggccctcctggcagtaatggtaacccaggccccccaggctccagtggtgctccaggcaaagatggtcccccaggtccacctggcagtaatggtgctcctggcagccccgggatctctggaccaaagggtgattctggtccaccaggtgagaggggagcacctggcccccagggccctccgggagctccaggcccactaggaattgcaggacttactggagcacgaggtcttgcaggcccaccaggcatgccaggtgctaggggcagccccggcccacagggcatcaagggtgaaaatggtaaaccaggacctagtggtcagaatggagaacgtggtcctcctggcccccagggtcttcctggtctggctggtacagctggtgagcctggaagagatggaaaccctggatcagatggtctgccaggccgagatggagctccaggtgccaagggtgaccgtggtgaaaatggctctcctggtgcccctggagctcctggtcacccaggccctcctggtcctgtcggtccagctggaaagagcggtgacagaggagaaactggccctgctggtccttctggggcccccggtcctgccggatcaagaggtcctcctggtccccaaggcccacgcggtgacaaaggggaaaccggtgagcgtggtgctatgggcatcaaaggacatcgcggattccctggcaacccaggggcccccggatctccgggtcccgctggtcatcaaggtgcagttggcagtccaggccctgcaggccccagaggacctgttggacctagcgggccccctggaaaggacggagcaagtggacaccctggtcccattggaccaccggggccccgaggtaacagaggtgaaagaggatctgagggctccccaggccacccaggacaaccaggccctcctggacctcctggtgcccctggtccatgttgtggtgctggcggggttgctgccattgctggtgttggagccgaaaaagctggtggttttgccccatattatggagatgaaccgatagatttcaaaatcaacaccgatgagattatgacctcactcaaatcagtcaatggacaaatagaaagcctcattagtcctgatggttcccgtaaaaaccctgcacggaactgcagggacctgaaattctgccatcctgaactccagagtggagaatattgggttgatcctaaccaaggttgcaaattggatgctattaaagtctactgtaacatggaaactggggaaacgtgcataagtgccagtcctttgactatcccacagaagaactggtggacagattctggtgctgagaagaaacatgtttggtttggagaatccatggaaggtggtttccaattcagctacggtaaccctgaacttcctgaagatgttcttgacgttcaattggcatttctgagattgttgtccagtcgtgcaagccaaaacattacataccattgcaaaaattccatcgcatatatggatcatgctagcggaaatgtgaaaaaggcattgaagctgatgggatcaaatgaaggtgaatttaaagcagagggtaattctaagtttacttacactgtattggaggatggttgtacgaagcatacaggtgaatggggtaaaacagtgtttcaatatcaaacccgcaaagcagttagattgccaatcgtcgatatcgcaccatacgacattggaggaccagatcaagagttcggagctgacatcggtccggtgtgtttcctttgataatcaagaggatgtcagaatgccatttgcctgagagatgcaggcttcatttttgatacttttttatttgtaacctatatagtataggattttttttgtcattttgtttcttctcgtacgagcttgctcctgatcagcctatctcgcagctgatgaatatcttgtggtaggggtttgggaaaatcattcgagtttgatgtttttcttggtatttcccactcctcttcagagtacagaagattaagtgagacgttcgtttgtgctccggaggatccttcagtaatgtcttgtttcttttgttgcagtggtgagccattttgacttcgtgaaagtttctttagaatagttgtttccagaggccaaacattccacccgtagtaaagtgcaagcgtaggaagaccaagactggcataaatcaggtataagtgtcgagcactggcaggtgatcttctgaaagtttctactagcagataagatccagtagtcatgcatatggcaacaatgtaccgtgtggatctaagaacgcgtcctactaaccttcgcattcgttggtccagtttgttgttatcgatcaacgtgacaaggttgtcgattccgcgtaagcatgcatacccaaggacgcctgttgcaattccaagtgagccagttccaacaatctttgtaatattagagcacttcattgtgttgcgcttgaaagtaaaatgcgaacaaattaagagataatctcgaaaccgcgacttcaaacgccaatatgatgtgcggcacacaataagcgttcatatccgctgggtgactttctcgctttaaaaaattatccgaaaaaattttctagagtgttgttactttatacttccggctcgtataatacgacaaggtgtaaggaggactaaaccatggctaaactcacctctgctgttccagtcctgactgctcgtgatgttgctggtgctgttgagttctggactgataggctcggtttctcccgtgacttcgtagaggacgactttgccggtgttgtacgtgacgacgttaccctgttcatctccgcagttcaggaccaggttgtgccagacaacactctggcatgggtatgggttcgtggtctggacgaactgtacgctgagtggtctgaggtcgtgtctaccaacttccgtgatgcatctggtccagctatgaccgagatcggtgaacagccctggggtcgtgagtttgcactgcgtgatccagctggtaactgcgtgcatttcgtcgcagaagagcaggactaacaattgacaccttacgattatttagagagtatttattagttttattgtatgtatacggatgttttattatctatttatgcccttatattctgtaactatccaaaagtcctatcttatcaagccagcaatctatgtccgcgaacgtcaactaaaaataagctttttatgctcttctctctttttttcccttcggtataattataccttgcatccacagattctcctgccaaattttgcataatcctttacaacatggctatatgggagcacttagcgccctccaaaacccatattgcctac

SEQ ID NO: 35 - DNA, 4751 bp, Bos taurus
  misc_feature (1)..(4751): Bos taurus collagen type I alpha 1 chain (COL1A1), mRNA;  NCBI Reference Sequence: NM_001034039.2
  CDS (119)..(4510)
gcagacgggagtttctcctcggggtcggagcaggaggcacgcggagtgtgaggccacgcatgagcggacgctaacccccaccccagccgcaaagagtctacatgtctagggtctagacatgttcagctttgtggacctccggctcctgctcctcttagcggccaccgccctcctgacgcacggccaagaggagggccaggaagaaggccaagaagaagacatcccaccagtcacctgcgtacagaacggcctcaggtaccatgaccgagacgtgtggaaacccgtgccctgccagatctgtgtctgcgacaacggcaacgtgctgtgcgatgacgtgatctgcgacgaacttaaggactgtcctaacgccaaagtccccacggacgaatgctgccccgtctgccccgaaggccaggaatcacccacggaccaagaaaccaccggagtcgagggaccgaaaggagacactggcccccgaggcccaaggggacccgccggcccccccggccgagatggcatccctggacaacctggacttcccggaccccctggaccccccggacctcccggaccccctggcctcggaggaaactttgctccccagttgtcttacggctatgatgagaaatcaacaggaatttccgtgcctggtcccatgggtccttctggtcctcgtggtctccctggcccccctggcgcacctggtccccaaggtttccaaggcccccctggtgagcctggcgagccaggagcctcaggtcccatgggtccccgtggtccccctggcccccctggcaagaacggagatgatggcgaagctggaaagcctggtcgtcctggtgagcgcgggcctcccggacctcagggtgctcggggattgcctggaacagctggcctccctggaatgaagggacacagaggtttcagtggtttggatggtgccaagggagatgctggtcctgctggccccaagggcgagcctggtagccccggtgaaaatggagctcctggtcagatgggcccccgtggtctgcctggtgagagaggtcgccctggagcccctggccctgctggtgctcgaggaaatgatggtgcgactggtgctgctgggccccctggtcccactggccccgctggtcctcctggtttccctggtgctgtgggtgctaagggtgaaggtggtccccaaggaccccgaggttctgaaggtccccagggtgtacgtggtgagcctggcccccctggccctgctggtgctgctggccctgctggcaaccctggtgctgatggacagcctggtgctaaaggagccaatggcgctcctggtattgctggtgctcctggcttccctggtgcccgaggcccctctggaccccagggccccagcggcccccctggccccaagggtaacagcggtgaacctggtgctcctggcagcaaaggagacactggcgccaagggagaacccggtcccactggtattcaaggcccccctggccccgctggggaagaaggaaagcgaggagcccgaggtgaacctggacctgctggcctgcctggaccccctggcgagcgtggtggacctggaagccgtggtttccctggcgccgacggtgttgctggtcccaagggtcctgctggtgaacgcggtgctcctggccctgctggccccaaaggttctcctggtgaagctggtcgccccggtgaagctggtctgcccggtgccaagggtctgactggaagccctggcagcccgggtcctgatggcaaaactggcccccctggtcccgccggtcaagatggccgccctggacctccaggccctcccggtgcccgtggtcaggctggcgtgatgggtttccctggacctaaaggtgctgctggagagcctggaaaagctggagagcgaggtgttcctggaccccctggcgctgttggtcctgctggcaaagacggagaagctggagctcagggacccccaggacctgctggccccgctggtgagagaggcgaacaaggccctgctggctcccctggattccagggtctccccggccctgctggtcctcctggtgaagcaggcaaacctggtgaacagggtgttcctggagatcttggtgcccccggcccctctggagcaagaggcgagagaggtttccccggcgagcgtggtgtgcaagggccgcccggtcctgcaggtccccgtggggccaatggtgcccctggcaacgatggtgctaagggtgatgctggtgcccctggagcccccggtagccagggtgcccctggccttcaaggaatgcctggtgaacgaggtgcagctggtcttccaggccctaagggtgacagaggggatgctggtcccaaaggtgctgatggtgctcctggcaaagatggcgtccgtggtctgactggtcccatcggtcctcctggccccgctggtgcccctggtgacaagggtgaagctggtcctagtggcccagccggtcccactggagctcgtggtgcccccggtgaccgtggtgagcctggtccccccggccctgctggcttcgctggcccccctggtgctgatggccaacctggtgctaaaggcgaacctggtgatgctggtgctaaaggtgacgctggtccccccggccctgctgggcccgctggaccccccggccccattggtaacgttggtgctcccggacccaaaggtgctcgtggcagcgctggtccccctggtgctactggtttcccaggtgctgctggccgagtcggtccccccggcccctctggaaatgctggaccccctggccctcctggccctgctggcaaagaaggcagcaaaggcccccgcggtgagactggccccgctgggcgtcccggtgaagtcggtccccctggtccccctggccccgctggtgagaaaggagcccctggtgctgacggacctgctggagctcctggcactcctggacctcaaggtattgctggacagcgtggtgtggtcggcctgcctggtcagagaggagaaagaggcttccctggtcttcctggcccctctggtgaacccggcaaacaaggtccttctggagcaagtggtgaacgtggcccccctggtcccatgggcccccctggattggctggaccccctggcgagtctggacgtgagggagctcctggtgctgaaggatcccctggacgagatggttctcctggcgccaagggtgaccgtggtgagaccggccctgctggacctcctggtgctcctggcgctcccggtgcccccggccctgtcggacctgccggcaagagcggtgatcgtggtgagaccggtcctgctggtcctgctggtcccattggccccgttggtgcccgtggccccgctggaccccaaggcccccgtggtgacaagggtgagacaggcgaacagggcgacagaggcattaagggtcaccgtggcttctctggtctccagggtccccccggccctcccggctctcctggtgagcaaggtccttccggagcctctggtcctgctggtccccgcggtccccctggctctgctggttctcccggcaaagatggactcaatggtctcccaggccccatcggtccccctgggcctcgaggtcgcactggtgatgctggtcctgctggtcctcccggccctcctggaccccctggtcccccaggtcctcccagcggcggctacgacttgagcttcctgccccagccacctcaagagaaggctcacgatggtggccgctactaccgggctgatgatgccaatgtggtccgtgaccgtgacctcgaggtggacaccaccctcaagagcctgagccagcagatcgagaacatccggagccctgaaggcagccgcaagaaccccgcccgcacctgccgtgacctcaagatgtgccactctgactggaagagcggagaatactggattgaccccaaccaaggctgcaacctggatgccattaaggtcttctgcaacatggaaaccggtgagacctgtgtataccccactcagcccagcgtggcccagaagaactggtatatcagcaagaaccccaaggaaaagaggcacgtctggtacggcgagagcatgaccggcggattccagttcgagtatggcggccaggggtccgatcctgccgatgtggccatccagctgactttcctgcgcctgatgtccaccgaggcctcccagaacatcacctaccactgcaagaacagcgtggcctacatggaccagcagactggcaacctcaagaaggccctgctcctccagggctccaacgagatcgagatccgggccgagggcaacagccgcttcacctacagcgtcacctacgatggctgcacgagtcacaccggagcctggggcaagacagtgatcgaatacaaaaccaccaagacctcccgcttgcccatcatcgatgtggcccccttggacgttggcgccccagaccaggaattcggcttcgacgttggccctgcctgcttcctgtaaactccttccaccccaacctggctccctcccacccaacccacttgcccctgactctggaaacagacaaacaacccaaactgaaacccccgaaaagccaaaaaatgggagacaatttcacatggactttggaaaatatttttttcctttgcattcatctctcaaacttagtttttatctttgaccaactgaacatgaccaaaaaccaaaagtgcattcaaccttaccaaaaaaaaaaaaaaaa

SEQ ID NO: 36 - protein, 1463 aa, Bos taurus
MFSFVDLRLLLLLAATALLTHGQEEGQEEGQEEDIPPVTCVQNGLRYHDRDVWKPVPCQICVCDNGNVLCDDVICDELKDCPNAKVPTDECCPVCPEGQESPTDQETTGVEGPKGDTGPRGPRGPAGPPGRDGIPGQPGLPGPPGPPGPPGPPGLGGNFAPQLSYGYDEKSTGISVPGPMGPSGPRGLPGPPGAPGPQGFQGPPGEPGEPGASGPMGPRGPPGPPGKNGDDGEAGKPGRPGERGPPGPQGARGLPGTAGLPGMKGHRGFSGLDGAKGDAGPAGPKGEPGSPGENGAPGQMGPRGLPGERGRPGAPGPAGARGNDGATGAAGPPGPTGPAGPPGFPGAVGAKGEGGPQGPRGSEGPQGVRGEPGPPGPAGAAGPAGNPGADGQPGAKGANGAPGIAGAPGFPGARGPSGPQGPSGPPGPKGNSGEPGAPGSKGDTGAKGEPGPTGIQGPPGPAGEEGKRGARGEPGPAGLPGPPGERGGPGSRGFPGADGVAGPKGPAGERGAPGPAGPKGSPGEAGRPGEAGLPGAKGLTGSPGSPGPDGKTGPPGPAGQDGRPGPPGPPGARGQAGVMGFPGPKGAAGEPGKAGERGVPGPPGAVGPAGKDGEAGAQGPPGPAGPAGERGEQGPAGSPGFQGLPGPAGPPGEAGKPGEQGVPGDLGAPGPSGARGERGFPGERGVQGPPGPAGPRGANGAPGNDGAKGDAGAPGAPGSQGAPGLQGMPGERGAAGLPGPKGDRGDAGPKGADGAPGKDGVRGLTGPIGPPGPAGAPGDKGEAGPSGPAGPTGARGAPGDRGEPGPPGPAGFAGPPGADGQPGAKGEPGDAGAKGDAGPPGPAGPAGPPGPIGNVGAPGPKGARGSAGPPGATGFPGAAGRVGPPGPSGNAGPPGPPGPAGKEGSKGPRGETGPAGRPGEVGPPGPPGPAGEKGAPGADGPAGAPGTPGPQGIAGQRGVVGLPGQRGERGFPGLPGPSGEPGKQGPSGASGERGPPGPMGPPGLAGPPGESGREGAPGAEGSPGRDGSPGAKGDRGETGPAGPPGAPGAPGAPGPVGPAGKSGDRGETGPAGPAGPIGPVGARGPAGPQGPRGDKGETGEQGDRGIKGHRGFSGLQGPPGPPGSPGEQGPSGASGPAGPRGPPGSAGSPGKDGLNGLPGPIGPPGPRGRTGDAGPAGPPGPPGPPGPPGPPSGGYDLSFLPQPPQEKAHDGGRYYRADDANVVRDRDLEVDTTLKSLSQQIENIRSPEGSRKNPARTCRDLKMCHSDWKSGEYWIDPNQGCNLDAIKVFCNMETGETCVYPTQPSVAQKNWYISKNPKEKRHVWYGESMTGGFQFEYGGQGSDPADVAIQLTFLRLMSTEASQNITYHCKNSVAYMDQQTGNLKKALLLQGSNEIEIRAEGNSRFTYSVTYDGCTSHTGAWGKTVIEYKTTKTSRLPIIDVAPLDVGAPDQEFGFDVGPACFL

SEQ ID NO: 37 - DNA, 4628 bp, Bos taurus
  misc_feature (1)..(4628): Bos taurus collagen type I alpha 2 chain (COL1A2), mRNA;  NCBI Reference Sequence: NM_174520.2
  CDS (111)..(4205)
taagttggaggtactggccacgactgcatgcctgcgcccgccaggtgatacctccgccggtgacccaggggctctgcgacacaaggagtctgcatgtctgagtggtagacatgctcagctttgtggatacgcggactttgttgctgcttgcagtaacttcgtgcctagcaacatgccaatccttacaagaggcaactgcaagaaagggcccaagtggagatagaggaccacgcggagaaaggggtccaccaggcccaccaggcagagatggtgatgacggcatcccaggccctcctggcccccctggccctcctggcccccctggtcttggcgggaactttgctgctcagtttgatgcaaaaggaggtggccctggaccaatggggctgatgggacctcgcggccctcctggggcttctggagcccctggccctcaaggtttccagggacctccgggtgagcctggtgaacctggtcagactggtcctgcaggtgctcgtggcccgcctggccctcctggcaaggctggtgaggatggtcaccctggaaaacctggacgacctggtgagagaggggttgttggaccacagggtgctcgtggctttcctggaactcctggactccctggcttcaagggcattaggggtcacaatggtctggatggattgaagggacagcctggtgctccaggtgtgaagggtgaacctggtgcccctggtgaaaatggaactccaggtcaaacgggagcccgtggtcttcctggtgagagaggacgtgttggtgcccctggcccagctggtgcccgtggaagtgatggaagtgtgggtcctgtgggccctgctggtcccattgggtctgctggccctccaggcttcccaggtgctcctggccccaagggtgaactcggacctgttggtaaccctggccctgctggtcccgcgggtccccgtggtgaagtgggtctcccaggcctttctggccctgtcggacctcctggaaaccccggagccaatgggcttcctggcgctaagggtgctgctggccttcccggtgttgctggggctcccggcctccctggaccccggggtattcctggccctgttggcgctgctggtgctactggcgccagaggacttgttggtgagcccggcccagctggttcgaaaggagagagcggcaacaagggcgagcctggtgctgttgggcagccaggtcctcctggccccagtggtgaagaaggaaagagaggctccactggagaaatcggacccgctggccccccaggacctcctgggctgaggggaaatcctggctcccgtggtctacctggagctgacggcagagctggtgtcatgggtcctgctggtagccgtggtgcaactggccctgctggtgtgcgaggtcccaatggagattctggtcgccctggagagcctggcctcatgggaccccgaggtttcccaggttcccctggaaatatcggcccagctggtaaagaaggtcctgtgggtctccctggtattgacggcagacctgggcccattggcccagcgggagcaagaggagagcctggcaacattggattccctggacccaaaggccccagtggtgatcctggcaaagctggtgaaaaaggtcatgctggtcttgctggtgctcggggcgctccaggtcccgatggcaacaacggtgctcagggaccccctggactacagggtgtccaaggtggaaaaggtgaacagggtcctgctggtcctccaggcttccagggtctgcctggccctgcaggcacagctggtgaagctggcaaaccaggagaaaggggtatccctggtgaatttggtctccctggccctgctggtgcaagaggggagcgggggcccccaggtgaaagtggtgctgctgggcctactgggcctattggaagccgaggtccttctggacccccagggcctgatggaaacaagggtgaaccgggtgtggttggcgctccaggcactgctggcccatctggtcctagcggactcccaggagagaggggtgcggctggcattcctggaggcaagggagaaaagggtgaaactggtctcagaggtgacattggtagccctggtagagatggtgctcgtggtgctcctggtgctattggtgctcctggccctgctggagccaatggggaccggggtgaagctggtcccgctggccctgctggccctgctggtcctcgtggtagccctggtgaacgtggtgaggtcggtcccgctggccccaacggatttgctggtcctgctggtgctgctggtcaacctggtgctaaaggagagagaggaaccaaaggacccaagggtgaaaatggtcctgttggtcccacaggccccgttggagctgccggtccgtctggtccaaatggcccacctggtcctgctggaagtcgtggtgatggagggccccctggggctactggtttccctggtgctgctggacggactggtccccctggaccctctggtatctctggcccccctggcccccctggtcctgctggtaaagaagggcttcgtgggcctcgtggtgaccaaggtccagttggtcgaagtggagagacaggtgcctctggccctcctggctttgttggtgagaagggtccctctggagagcctggtactgctgggcctcctggaaccccaggtccacaaggccttcttggtgctcctggttttctgggtctcccaggctctagaggtgagcgtggtctaccaggtgtcgctggatctgtgggtgaacctggccccctcggcatcgcaggcccacctggggcccgtggtccccctggtaatgtcggtaatcctggcgtcaatggtgctcctggtgaagccggtcgtgacggcaaccctgggaatgacggtcccccaggccgcgatggtcaacccggacacaagggggagcgtggttaccccggtaacgcaggtcctgttggtgctgccggtgctcctggccctcaaggccctgtgggtcccgttggtaaacacggaaaccgtggtgaaccgggtcctgccggtgctgttggtcctgctggtgccgttggcccaagaggtcccagtggcccacaaggtattcgaggtgacaagggagagcctggtgataagggtcccagaggtcttcctggcttaaagggacacaatgggttgcaaggtctcccgggtcttgctggtcatcatggcgatcaaggtgctcccggtgctgtgggtcccgctggtcccaggggccctgctggtccttctggccccgctggcaaagacggtcgcattggacagcctggtgcagtcggacctgctggcattcgtggctctcagggtagccaaggtcctgctggccctcctggtccccctggccctcctggacctcctggcccaagtggtggtggttacgagtttggttttgatggagacttctacagggctgaccagcctcgctcaccaacttctctcagacccaaggattatgaagttgatgctactctgaaatctctcaacaaccagattgagacccttcttactccagaaggctctaggaagaacccagctcgcacatgccgagacttgagactcagccacccagaatggagcagtggttactactggattgaccctaaccaaggatgtactatggatgctatcaaagtatactgtgatttctctactggcgaaacctgcatccgggctcaacctgaagacatcccagtcaagaactggtacagaaattccaaggccaagaagcatgtctgggtaggagaaactatcaacggtggtacccagtttgaatataatgttgaaggagtaaccaccaaggaaatggctacccaacttgccttcatgcgtctgctggccaaccatgcctctcagaacatcacctaccattgcaagaacagcattgcatacatggatgaggaaactggcaacctgaaaaaggctgtcattctgcaaggatccaatgatgtcgaacttgttgccgagggcaacagcagattcacttacactgttcttgtagatggctgctctaaaaagacaaatgaatggcagaagacaatcattgaatataaaacaaacaagccatctcgcctgcctatccttgatattgcacctttggacatcggtggcgctgaccaagaaatcagattgaacattggcccagtctgtttcaaataaacgaactcaacctaaattaaagaaaaaggaaatctgaaacatttctcttggccatttctttttcttctttcctaactgaaagctgaatccttccatttcttctgcacatctacttgcttaaattgtggcaaaagaggagaaggattgatcagagcattgtgcaatacaatttaattcactccccctcccttttcccctctccaaaagatttggaattttttttttttcaacactcttacacctgttgtggaaaatgtcaacctttgtaagaaaaccaaaataaaaattgaaaaataaaaaccatgaacatttgcaccacttgtggcttttgaatatcttccacggagggaagtttaaaacccaaacttccaaaggtttaaactacctcaaaacactttcctgtgagtgtgatccacacctcgt

SEQ ID NO: 38 - protein, 1364 aa, Bos taurus
MLSFVDTRTLLLLAVTSCLATCQSLQEATARKGPSGDRGPRGERGPPGPPGRDGDDGIPGPPGPPGPPGPPGLGGNFAAQFDAKGGGPGPMGLMGPRGPPGASGAPGPQGFQGPPGEPGEPGQTGPAGARGPPGPPGKAGEDGHPGKPGRPGERGVVGPQGARGFPGTPGLPGFKGIRGHNGLDGLKGQPGAPGVKGEPGAPGENGTPGQTGARGLPGERGRVGAPGPAGARGSDGSVGPVGPAGPIGSAGPPGFPGAPGPKGELGPVGNPGPAGPAGPRGEVGLPGLSGPVGPPGNPGANGLPGAKGAAGLPGVAGAPGLPGPRGIPGPVGAAGATGARGLVGEPGPAGSKGESGNKGEPGAVGQPGPPGPSGEEGKRGSTGEIGPAGPPGPPGLRGNPGSRGLPGADGRAGVMGPAGSRGATGPAGVRGPNGDSGRPGEPGLMGPRGFPGSPGNIGPAGKEGPVGLPGIDGRPGPIGPAGARGEPGNIGFPGPKGPSGDPGKAGEKGHAGLAGARGAPGPDGNNGAQGPPGLQGVQGGKGEQGPAGPPGFQGLPGPAGTAGEAGKPGERGIPGEFGLPGPAGARGERGPPGESGAAGPTGPIGSRGPSGPPGPDGNKGEPGVVGAPGTAGPSGPSGLPGERGAAGIPGGKGEKGETGLRGDIGSPGRDGARGAPGAIGAPGPAGANGDRGEAGPAGPAGPAGPRGSPGERGEVGPAGPNGFAGPAGAAGQPGAKGERGTKGPKGENGPVGPTGPVGAAGPSGPNGPPGPAGSRGDGGPPGATGFPGAAGRTGPPGPSGISGPPGPPGPAGKEGLRGPRGDQGPVGRSGETGASGPPGFVGEKGPSGEPGTAGPPGTPGPQGLLGAPGFLGLPGSRGERGLPGVAGSVGEPGPLGIAGPPGARGPPGNVGNPGVNGAPGEAGRDGNPGNDGPPGRDGQPGHKGERGYPGNAGPVGAAGAPGPQGPVGPVGKHGNRGEPGPAGAVGPAGAVGPRGPSGPQGIRGDKGEPGDKGPRGLPGLKGHNGLQGLPGLAGHHGDQGAPGAVGPAGPRGPAGPSGPAGKDGRIGQPGAVGPAGIRGSQGSQGPAGPPGPPGPPGPPGPSGGGYEFGFDGDFYRADQPRSPTSLRPKDYEVDATLKSLNNQIETLLTPEGSRKNPARTCRDLRLSHPEWSSGYYWIDPNQGCTMDAIKVYCDFSTGETCIRAQPEDIPVKNWYRNSKAKKHVWVGETINGGTQFEYNVEGVTTKEMATQLAFMRLLANHASQNITYHCKNSIAYMDEETGNLKKAVILQGSNDVELVAEGNSRFTYTVLVDGCSKKTNEWQKTIIEYKTNKPSRLPILDIAPLDIGGADQEIRLNIGPVCFK

SEQ ID NO: 39 - DNA, 623 bp, Artificial Sequence
  pDF promoter
aatgtatctaaacgcaaactccgagctggaaaaatgttaccggcgatgcgcggacaatttagaggcggcgatcaagaaacacctgctgggcgagcagtctggagcacagtcttcgatgggcccgagatcccaccgcgttcctgggtaccgggacgtgaggcagcgcgacatccatcaaatataccaggcgccaaccgagtgtctcggaaaacagcttctggatatcttccgctggcggcgcaacgacgaataatagtccctggaggtgacggaatatatatgtgtggagggtaaatctgacagggtgtagcaaaggtaatattttcctaaaacatgcaatcggctgccccgcaacgggaaaaagaatgactttggcactcttcaccagagtggggtgtcccgctcgtgtgtgcaaataggctcccactggtcaccccggattttgcagaaaaacagcaagttccggggtgtctcactggtgtccgccaataagaggagccggcaggcacggagtttacatcaagctgtctccgatacactcgactaccatccgggtctctcagagaggggaatggcactataaataccgcctccttgcgctctctgccttcatcaatcaaatc

SEQ ID NO: 40 - DNA, 822 bp, Artificial Sequence
  pGCEW14 promoter
caggtgaacccacctaactatttttaactgggatccagtgagctcgctgggtgaaagccaaccatcttttgtttcggggaaccgtgctcgccccgtaaagttaatttttttttcccgcgcagctttaatctttcggcagagaaggcgttttcatcgtagcgtgggaacagaataatcagttcatgtgctatacaggcacatggcagcagtcactattttgctttttaaccttaaagtcgttcatcaatcattaactgaccaatcagattttttgcatttgccacttatctaaaaatacttttgtatctcgcagatacgttcagtggtttccaggacaacacccaaaaaaaggtatcaatgccactaggcagtcggttttatttttggtcacccacgcaaagaagcacccacctcttttaggttttaagttgtgggaacagtaacaccgcctagagcttcaggaaaaaccagtacctgtgaccgcaattcaccatgatgcagaatgttaatttaaacgagtgccaaatcaagatttcaacagacaaatcaatcgatccatagttacccattccagccttttcgtcgtcgagcctgcttcattcctgcctcaggtgcataactttgcatgaaaagtccagattagggcagattttgagtttaaaataggaaatataaacaaatataccgcgaaaaaggtttgtttatagcttttcgcctggtgccgtacggtataaatacatactctcctcccccccctggttctctttttcttttgttacttacattttaccgttccgtcactcgcttcactcaacaacaaaa

SEQ ID NO: 41 - DNA, 476 bp, Artificial Sequence
  pGAP1 promoter
tttttgtagaaatgtcttggtgtcctcgaccaatcaggtagccatccctgaaatacctggctccgtggcaacaccgaacgacctgctggcaacgttaaattctccggggtaaaacttaaatgtggagtaatagaaccagaaacgtctcttcccttctctctccttccaccgcccgttaccgtccctaggaaattttactctgctggagagcttcttctacggcccccttgcagcaatgctcttcccagcattacgttgcgggtaaaacggaggtcgtgtacccgacctagcagcccagggatggaaagtcccggccgtcgctggcaataactgcgggcggacgcatgtcttgagattattggaaaccaccagaatcgaatataaaaggcgaacacctttcccaattttggtttctcctgacccaaagactttaaatttaatttatttgtccctatttcaatcaattgaacaactat

SEQ ID NO: 42 - DNA, 550 bp, Artificial Sequence; identical to SEQ ID NO: 26
  pHTX1 bi-directional promoter

SEQ ID NO: 43 - DNA, 931 bp, Artificial Sequence
  pAOX1 promoter
aacatccaaagacgaaaggttgaatgaaacctttttgccatccgacatccacaggtccattctcacacataagtgccaaacgcaacaggaggggatacactagcagcagaccgttgcaaacgcaggacctccactcctcttctcctcaacacccacttttgccatcgaaaaaccagcccagttattgggcttgattggagctcgctcattccaattccttctattaggctactaacaccatgactttattagcctgtctatcctggcccccctggcgaggttcatgtttgtttatttccgaatgcaacaagctccgcattacacccgaacatcactccagatgagggctttctgagtgtggggtcaaatagtttcatgttccccaaatggcccaaaactgacagtttaaacgctgtcttggaacctaatatgacaaaagcgtgatctcatccaagatgaactaagtttggttcgttgaaatgctaacggccagttggtcaaaaagaaacttccaaaagtcggcataccgtttgtcttgtttggtattgattgacgaatgctcaaaaataatctcattaatgcttagcgcagtctctctatcgcttctgaaccccggtgcacctgtgccgaaacgcaaatggggaaacacccgctttttggatgattatgcattgtctccacattgtatgcttccaagattctggtgggaatactgctgatagcctaacgttcatgatcaaaatttaactgttctaacccctacttgacagcaatatataaacagaaggaagctgccctgtcttaaacctttttttttatcatcattattagcttactttcataattgcgactggttccaattgacaagcttttgattttaacgacttttaacgacaacttgagaagatcaaaaaacaactaattattgaaa

SEQ ID NO: 44 - DNA, 699 bp, Artificial Sequence
  pDas1 promoter
ctatgctaccccacagaaataccccaaaagttgaagtgaaaaaatgaaaattactggtaacttcaccccataacaaacttaataatttctgtagccaatgaaagtaaaccccattcaatgttccgagatttagtatacttgcccctataagaaacgaaggatttcagcttccttaccccatgaacagaaatcttccatttaccccccactggagagatccgcccaaacgaacagataatagaaaaaagaaattcggacaaatagaacactttctcagccaattaaagtcattccatgcactccctttagctgccgttccatccctttgttgagcaacaccatcgttagccagtacgaaagaggaaacttaaccgataccttggagaaatctaaggcgcgaatgagtttagcctagatatccttagtgaagggttgttccgatacttctccacattcagtcatagatgggcagctttgttatcatgaagagacggaaacgggcattaagggttaaccgccaaattatataaagacaacatgtccccagtttaaagtttttctttcctattcttgtatcctgagtgaccgttgtgtttaatataacaagttcgttttaacttaagaccaaaaccagttacaacaaattataacccctctaaacactaaagttcactcttatcaaactatcaaacatcaaaa

SEQ ID NO: 45 - DNA, 552 bp, Artificial Sequence
  pDas2 promoter
agcaatgatataaacaacaattgagtgacaggtctactttgttctcaaaaggccataaccatctgtttgcatctcttatcaccacaccatcctcctcatctggccttcaattgtggggaacaactagcatcccaacaccagactaactccacccagatgaaaccagttgtcgcttaccagtcaatgaatgttgagctaacgttccttgaaactcgaatgatcccagccttgctgcgtatcatccctccgctattccgccgcttgctccaaccatgtttccgcctttttcgaacaagttcaaatacctatctttggcaggacttttcctcctgccttttttagcctcagctctcggttagcctctaggcaaattctggtcttcatacctatatcaacttttcatcagatagcctttgggttcaaaaaagaactaaagcaggatgcctgatatataaatcccagatgatctgcttttgaaactattttcagtatcttgattcgtttacttacaaacaactattgttgattttatctggagaataatcgaacaaa

SEQ ID NO: 46 - DNA, 2326 bp, Bos taurus
  misc_feature (1)..(2326): Bos taurus prolyl 4-hydroxylase, alpha polypeptide II, mRNA (cDNA clone MGC:127031 IMAGE:7942056), complete cds
  CDS (413)..(1876): Bos taurus prolyl 4-hydroxylase, alpha polypeptide II, mRNA (cDNA clone MGC:127031 IMAGE:7942056), complete cds
aaaaagttcgagtctgtaccggactgtgcaacggagcagggaaaggctcagggccgccctaccacgctgtcaccgccgggcctccgaggaagagtggcgttttctctcgactttggaggttctgggttctaggctctgtgctggacctggatacacagtgataaacaggccagaagcagctcccatccctaggaaggcaaagtggtgaaggatgcagacatgacagtcagatcatcctgattacccagttttgcctcagcagccgcggagactgtaactagttaactaattcaagaaacgaacccttcagtgttaatcagaaactgcaaggagttgctggcctagtggggcacgtggactggagaccaggaaaggccaggccccggtcagtgtgacactgccctctgtgaccatgaaaccctgggagtccacgttgctggtggcctggtttggtgtcctgagctgcgtgcaggctgaattcttcacttctattggacacatgacagacctgatttatgcagagaaggacctggtgcagtccctgaaggagtacatcctggtggaggaagccaagctctccaagattaagagctgggctgacaaaatggaagccctgaccagcaagtcggctgctgaccctgagggctacctggcccaccctgtgaatgcctataaactggtgaagcggctaaacacggactggcctgcactggaggaccttgtcctgcagaactcggccgcaggaaccaaataccaggccatgctgagtgtggatgactgctttgggatgggccgctcggcctacaacgaaggcgactattaccacacggtgttgtggatggaacaggtgctaaagcagctcgatgctggggaggaggccaccacatccaaggcccaggtgctggactatctgagctacgctgtcttccagttgggtgacctgcaccgtgccgtggagctcacccgccgcctgctctcccttgacccgagccatgaacgagctggagggaatctgcactactttgaacggttgttggaagaagaaagagaaaaaatgttatcgaatcacacagaagctgagcttgcatcccagcaaggcatatacgagaggcctgtggactacctgccggagagggatgtctacgagagcctctgtcgtggggagggtgtcaaactgaccccccgaaggcagaagaggctcttctgtaggtatcaccatggcaacagggtgccgcagctgctcatcgcccccttcaaagaggaggatgagtgggacagcccgcacatcgtcaggtactacgacgtcatgtctgacgaggaaatcgagaggatcaaggagattgcgaaacccaaacttgcacgagccactgttcgtgatcccaagacaggtgtgcttactgtcgccagctacagggtttccaaaagctcctggctggaggaggacgatgaccccgttgtggctcgggtgaatctgcggatgcagcacatcacagggctaacagtgaagactgcagaattgttgcaggttgctaattatggaatgggaggacagtacgagccacattttgacttctccaggcgaccttttgacagcggcctcaaaacggaggggaataggttagcgacgtttcttaactatatgagtgatgtagaagctggtggtgccaccgtctttcctgatctgggggctgcaatttggcctaagaagggcacagctgtattctggtacaacctcctacggagtggggaaggtgactatcgaacaagacatgctgcctgccctgtgcttgtgggctgcaagtgggtctccaataagtggttccatgaacgaggacaggaattcttgaggccgtgtggatcgacagaagttgactgacatcattttctgcccttcgccttcctggccccacagtccgtgttgtcttcaagttcaatgtgacagactcctgtctatgttccagtcccatcaggcgggtctctggaggcataaatgttttgtgtggagtagagagtggactagggaaggtcctggacgacctgggccccagcctctctgaccagcccgtgctatctctggacgctcgggtagggttggagcagagtcaggtggtctgcacctagcaaggtgcttttgtacctcagatgctttaggtgtgagatgtttcagtgaaccaaagttctgattccttgtttacatgcttgtttttatggaatttctattaatgtggctttaaccaaaataaaacgtccctgccagaagccttaaaaaaaaaaaaaaaaaaaaaaaaaaaaaaaaaaaaaaaaaaaagaaaataaaaaaaaaaga

SEQ ID NO: 47 - protein, 487 aa, Bos taurus
MKPWESTLLVAWFGVLSCVQAEFFTSIGHMTDLIYAEKDLVQSLKEYILVEEAKLSKIKSWADKMEALTSKSAADPEGYLAHPVNAYKLVKRLNTDWPALEDLVLQNSAAGTKYQAMLSVDDCFGMGRSAYNEGDYYHTVLWMEQVLKQLDAGEEATTSKAQVLDYLSYAVFQLGDLHRAVELTRRLLSLDPSHERAGGNLHYFERLLEEEREKMLSNHTEAELASQQGIYERPVDYLPERDVYESLCRGEGVKLTPRRQKRLFCRYHHGNRVPQLLIAPFKEEDEWDSPHIVRYYDVMSDEEIERIKEIAKPKLARATVRDPKTGVLTVASYRVSKSSWLEEDDDPVVARVNLRMQHITGLTVKTAELLQVANYGMGGQYEPHFDFSRRPFDSGLKTEGNRLATFLNYMSDVEAGGATVFPDLGAAIWPKKGTAVFWYNLLRSGEGDYRTRHAACPVLVGCKWVSNKWFHERGQEFLRPCGSTEVD

SEQ ID NO: 48 - DNA, 2580 bp, Bos taurus
  misc_feature (1)..(2580): Bos taurus prolyl 3-hydroxylase 1 (P3H1), mRNA; NCBI Reference Sequence: NM_001103291.1
  CDS (28)..(2238)
caagggtcccgttaggtctgagcggccatggcggcacgcgctttaaggctgctgaccatattgctggccgtcgccgccactgcctcccaggctgaggccgagtccgaggcgggatgggacctgacggcgcctgatctgctgttcgcggaggggacggcggcctatgctcgcggggactgggccggtgtggttctgagcatggagcgggcgctccgctcgcgggccgccctgcgcgccctccgtctgcgctgccgcactcggtgtgccgccgacctcccatgggaagtggacccagactcgcccccaagcttggcgcaggcttcaggtgcctccgccctgcacgacctgcggttcttcggaggcttgctgcgccgcgccgcttgcctgcgccgctgcctcgggccgtcgaccgcccactcgctcagcgaggagctggagttggagttccgcaagcggagcccctacaactacctgcaggtcgcctacttcaagataaacaagttggagaaagctgtagcagcagcccataccttcttcgtgggcaaccctgagcacatggagatgcgacagaacctggactattaccagaccatgtctggggtgaaggaggctgacttcaaggatcttgaggccaaaccccatatgcacgaatttcggctgggagtgcgcctctactccgaggagcagccgcaggaagccgtgccccacctggaggcggcgctgcgggagtacttcgtggcggccgaggagtgccgcgcgctctgcgaagggccctatgactacgacggctacaactacctggagtacaatgccgacctcttccaggccatcacagatcattacatccaggtcctcagctgtaagcagaactgtgtcacggagcttgcttcccacccaagtcgagagaagccctttgaagacttcctgccatctcattataattatctgcagtttgcctactataacattgggaattacacacaggccattgaatgtgccaagacctatctcctcttctttcccaatgatgaggtgatgagccagaatctggcctactatacagccatgcttggagaagagcaagccagatccattggcccccgtgagagtgcccaggagtaccgccagcggagcctgctggagaaggaactgcttttcttcgcctatgacgtttttggaattccctttgttgatccggattcatggactccagtggaggtgattcctaagagactgcaagagaaacagaagtcagaacgggaaacagctgcccgcatctcccaggaaatcgggaaccttatgaaggagatcgagaccctcgtggaggagaagaccaaggagtcactggacgtgagcaggctgacccgggaaggtggccccctgctgtatgatggcatcagactcaccatgaactccaaagtcctgaatggttcccagcgggtggtgatggatggcgtcatctctgacgaggagtgccaggagctgcagagactgaccaatgcagcagcaacttcaggagatggctaccggggtcagacctccccacacacccccagcgagaagttctacggtgtcaccgtcttcaaggccctcaagctggggcaggaagggaaggttcctctgcagagcgcccacctgtactacaacgtgacggagaaggtgcgccgcgtcatggagtcgtacttccgcctggataccccgctctacttctcctactcccacctggtgtgccgcaccgccatcgaagaggcacaggctgagaggaaggacggtagccaccccgtccacgtggacaactgcatcctgaatgccgaggccctcgtgtgcatcaaggagccccctgcctacactttccgggacttcagcgccattctttatctgaacgaagacttcgatggaggaaacttttatttcactgaactagatgccaagaccgtgacggcagaggtgcagccccagtgcggaagggctgtgggattctcttccggcacggaaaacccgcatggagtaaaggccgtcaccagagggcagcgctgtgccattgccctctggttcactttggatgctcgacacagcgagagggagcgagtgcaggcggacgacctggtaaagatgctctttagcccagaagagatggacctcccccacgagcagccccaagaagcccaggaggggacccccgagcccctacaggagcccgtctccagcagtgagtcagggcacaaggatgagctctgacaactcccgtggatggtgatcagacccacacgagggactctgtcctgcagcctggactggccagccccgggcgaggagcagtgggaacccaggcctgccgcccagctgagggggctctgctcacggccgtccgcatggtgctgctgctcttggagtggacatggcgagatggccctctcccctctgggcctgactgagggctcaggacgcaggcccagagccactctgggggcccacacaggcagccacgtgacagcaatacagtatttaagtgcctgtgtagacaaccaaagaataaatgattcgtggttttttttaaaaaaaaaaaaaaaaaaaaaaaaa

SEQ ID NO: 49 - protein, 736 aa, Bos taurus
MAARALRLLTILLAVAATASQAEAESEAGWDLTAPDLLFAEGTAAYARGDWAGVVLSMERALRSRAALRALRLRCRTRCAADLPWEVDPDSPPSLAQASGASALHDLRFFGGLLRRAACLRRCLGPSTAHSLSEELELEFRKRSPYNYLQVAYFKINKLEKAVAAAHTFFVGNPEHMEMRQNLDYYQTMSGVKEADFKDLEAKPHMHEFRLGVRLYSEEQPQEAVPHLEAALREYFVAAEECRALCEGPYDYDGYNYLEYNADLFQAITDHYIQVLSCKQNCVTELASHPSREKPFEDFLPSHYNYLQFAYYNIGNYTQAIECAKTYLLFFPNDEVMSQNLAYYTAMLGEEQARSIGPRESAQEYRQRSLLEKELLFFAYDVFGIPFVDPDSWTPVEVIPKRLQEKQKSERETAARISQEIGNLMKEIETLVEEKTKESLDVSRLTREGGPLLYDGIRLTMNSKVLNGSQRVVMDGVISDEECQELQRLTNAAATSGDGYRGQTSPHTPSEKFYGVTVFKALKLGQEGKVPLQSAHLYYNVTEKVRRVMESYFRLDTPLYFSYSHLVCRTAIEEAQAERKDGSHPVHVDNCILNAEALVCIKEPPAYTFRDFSAILYLNEDFDGGNFYFTELDAKTVTAEVQPQCGRAVGFSSGTENPHGVKAVTRGQRCAIALWFTLDARHSERERVQADDLVKMLFSPEEMDLPHEQPQEAQEGTPEPLQEPVSSSESGHKDEL

SEQ ID NO: 50 - DNA, 2030 bp, Bos taurus
  misc_feature (1)..(2030): Bos taurus lysyl oxidase (LOX), mRNA; NCBI Reference Sequence: NM_173932.4
  CDS (25)..(1281)
ggggacagtccaggaaagggagcgatgcgcttcgcctggaccgcactcctcgggtcgctgcagctctgcgcactcgtgcgctgcgccccgccggccgccagccaccggcagccccctcgcgaacaggcggcggctcccggcgcctggcgccagaagatccaatgggagaacaacgggcaggtgttcagcctgctgagcctgggctcgcagtaccagccgcaacggcgacgggaccccggcgccaccgccccgggggccgccaacgccactgccccacagatgcgcacaccaatcctgctgctccgcaacaaccgcaccgcggcggcgcgagtgcggacggccggcccctctgcggccgcagctggccgccccaggcccgccgcccgccactggttccaagctggctactcgacgtccggggcccacgacgctgggacctcgcgcgctgataaccagacggcaccgggagaggtcccgacgctcagtaacctgcgaccgcccaaccgcgtggacgtggacggcatggtgggcgacgacccgtacaacccctataagtacaccgacgacaacccctattacaactattacgacacgtacgaaaggcccaggcctgggagcaggtaccggcccggatacggcaccggctacttccagtatggtcttccggacctggtgcccgatccctactacatccaggcgtccacatacgtgcaaaagatggccatgtacaaccttagatgcgctgcggaggaaaactgcttggccagctcagcatacaggggagatgtcagagattatgatcacagggtgctgctaagatttccccagagagtgaaaaaccaagggacatctgatttcctaccaagtcgaccaagatattcctgggaatggcacagttgtcaccagcattaccacagcatggatgaattcagccactatgacctgcttgatgccagcacccagaggagagtggctgagggccataaagcgagtttctgtcttgaggacacatcgtgtgactacggctaccacaggcgatttgcatgtactgcacacacacagggcttgagtcctggctgctatgatacctataatgcagacatagactgccaatggattgatatcactgatgtcaaacctggaaactatattctcaaggtcagtgtgaatcccagctatttggtgcctgagtcggattattccaacaatgtcgtccgctgtgaaattcgctacacaggacatcacgcatatgcctcgggctgcacaatttcaccgtattagaaagcaagccaaaactcccaaaggatatatcagtgcctggtgttctgaagtggaaaaaaatagattaacttcagtaggatttatgtattttgaaagagagaacagaaaacaacaaaagaatttttgtttggactgttttataacaaagcacataactggattttgaacatttcaatcggcattatttgggaaatttttaatattattattcacattactttgtgaattaacacagtgtttcaattctgtaattgcacacttggctctttctgagaaatccaaatttcttatgcttcttctgaaattatagtgcaaaagggaaaaaaaattcgatgaatgagtcaaaattattttaaaactgagaattttctaaagttctaaaactttagtgaaccttaataataactggcttatatatgtcctagcatagatcactttagaaatgaagctcctactgtttaaatagatatggacacatttggtactgagggaggaataaacaggttaccattggtgtcaagaaatgttactatatagcagagaaatggcaatgtatgtattcagatagttacatccctatataaaatttgtttacattttaaaaattagtagataaactcctttctttctgtcaagtgtacaagttcattctgacttaagtcagcttttgttgtggaacaaattaagtaattgagctgcccaaaaaaaaaaaaaaaaaaaaaaaaaaaaaaaaaaaaaaaaaaaaaaaa

SEQ ID NO: 51 - protein, 418 aa, Bos taurus
MRFAWTALLGSLQLCALVRCAPPAASHRQPPREQAAAPGAWRQKIQWENNGQVFSLLSLGSQYQPQRRRDPGATAPGAANATAPQMRTPILLLRNNRTAAARVRTAGPSAAAAGRPRPAARHWFQAGYSTSGAHDAGTSRADNQTAPGEVPTLSNLRPPNRVDVDGMVGDDPYNPYKYTDDNPYYNYYDTYERPRPGSRYRPGYGTGYFQYGLPDLVPDPYYIQASTYVQKMAMYNLRCAAEENCLASSAYRGDVRDYDHRVLLRFPQRVKNQGTSDFLPSRPRYSWEWHSCHQHYHSMDEFSHYDLLDASTQRRVAEGHKASFCLEDTSCDYGYHRRFACTAHTQGLSPGCYDTYNADIDCQWIDITDVKPGNYILKVSVNPSYLVPESDYSNNVVRCEIRYTGHHAYASGCTISPY

SEQ ID NO: 52 - DNA, 2375 bp, Bos taurus
  misc_feature (1)..(2375): Bos taurus prolyl 4-hydroxylase subunit beta (P4HB), mRNA;       NCBI Reference Sequence: NM_174135.3
  misc_feature (6)..(65): Bos taurus prolyl 4-hydroxylase subunit beta (P4HB): signal peptide
  CDS (66)..(1535)
ccgacatgctgcgccgcgctctgctctgcctggccctgaccgcgctattccgcgcgggtgccggcgcccccgacgaggaggaccacgtcctggtgctccataagggcaacttcgacgaggcgctggcggcccacaagtacctgctggtggagttctacgccccatggtgcggccactgcaaggctctggccccggagtatgccaaagcagctgggaagctgaaggcagaaggttctgagatcagactggccaaggtggatgccactgaagagtctgacctggcccagcagtatggtgtccgaggctaccccaccatcaagttcttcaagaatggagacacagcttcccccaaagagtacacagctggccgagaagcggatgatatcgtgaactggctgaagaagcgcacgggccccgctgccagcacgctgtccgacggggctgctgcagaggccttggtggagtccagtgaggtggccgtcattggcttcttcaaggacatggagtcggactccgcaaagcagttcttcttggcagcagaggtcattgatgacatccccttcgggatcacatctaacagcgatgtgttctccaaataccagctggacaaggatggggttgtcctctttaagaagtttgacgaaggccggaacaactttgagggggaggtcaccaaagaaaagcttctggacttcatcaagcacaaccagttgcccctggtcattgagttcaccgagcagacagccccgaagatcttcggaggggaaatcaagactcacatcctgctgttcctgccgaaaagcgtgtctgactatgagggcaagctgagcaacttcaaaaaagcggctgagagcttcaagggcaagatcctgtttatcttcatcgacagcgaccacactgacaaccagcgcatcctggaattcttcggcctaaagaaagaggagtgcccggccgtgcgcctcatcacgctggaggaggagatgaccaaatataagccagagtcagatgagctgacggcagagaagatcaccgagttctgccaccgcttcctggagggcaagattaagccccacctgatgagccaggagctgcctgacgactgggacaagcagcctgtcaaagtgctggttgggaagaactttgaagaggttgcttttgatgagaaaaagaacgtctttgtagagttctatgccccgtggtgcggtcactgcaagcagctggcccccatctgggataagctgggagagacgtacaaggaccacgagaacatagtcatcgccaagatggactccacggccaacgaggtggaggcggtgaaagtgcacagcttccccacgctcaagttcttccccgccagcgccgacaggacggtcatcgactacaatggggagcggacactggatggttttaagaagttcctggagagtggtggccaggatggggccggagatgatgacgatctagaagatcttgaagaagcagaagagcctgatctggaggaagatgatgatcaaaaagctgtgaaagatgaactgtaacacagagagccagacctgggcaccaaacccggacctcccagtgggctgcacacccagcagcacagcctccagacgcccgcagaccctcccagcgagggagcgtcgattggaaatgcagggaacttttctgaagccacacttcactctaccacacgtgcaaatctaaacccgtcttcctttgcttttcaacttttggaaaagggtttatttccaggccagcccagcccagcccatcttggtgggcctttttttttaaatcgtgatgtactttttttgtacctggttttgtccagagtgctcgctaaaatgttttggactctcacgctggcaatgtctctcattcctgttaggtttatactatcactttaaaaaaattccgtctgtgggatttttagacatttttggacgtcagggtgtgtgctccaccttggccaggcctccctgggactcctgccctctgtggggcagaaccaggcaaggctggacgggtccctcacctcatgcggtattgccatggtggagcgtggctcctgcatcatttgattaaatggagactttccggtctctgtcacaggccgctccccaaccgtgagtggagggtgtggctgggccaggacaagcccagcactgtgccaggcagaaccgggacccttcgtttccaggctgggagacagccaaggatgcttggccccctccttccccaagccagggtccttattgctctgtgatgtccagggtggcctgaggagctgaatcacatgttgacagttcttcaggcatttctaccacaatattggaattggacacattggccaaataaagttaaaattttctgcc

SEQ ID NO: 53 - protein, 490 aa, Bos taurus
APDEEDHVLVLHKGNFDEALAAHKYLLVEFYAPWCGHCKALAPEYAKAAGKLKAEGSEIRLAKVDATEESDLAQQYGVRGYPTIKFFKNGDTASPKEYTAGREADDIVNWLKKRTGPAASTLSDGAAAEALVESSEVAVIGFFKDMESDSAKQFFLAAEVIDDIPFGITSNSDVFSKYQLDKDGVVLFKKFDEGRNNFEGEVTKEKLLDFIKHNQLPLVIEFTEQTAPKIFGGEIKTHILLFLPKSVSDYEGKLSNFKKAAESFKGKILFIFIDSDHTDNQRILEFFGLKKEECPAVRLITLEEEMTKYKPESDELTAEKITEFCHRFLEGKIKPHLMSQELPDDWDKQPVKVLVGKNFEEVAFDEKKNVFVEFYAPWCGHCKQLAPIWDKLGETYKDHENIVIAKMDSTANEVEAVKVHSFPTLKFFPASADRTVIDYNGERTLDGFKKFLESGGQDGAGDDDDLEDLEEAEEPDLEEDDDQKAVKDEL

SEQ ID NO: 54 - DNA, 2786 bp, Bos taurus
  misc_feature (1)..(2786): Bos taurus prolyl 4-hydroxylase subunit alpha 1 (P4HA1), mRNA;       NCBI Reference Sequence: NM_001075770.1
  CDS (104)..(1708)
gagtaggtagccggccgggtgcaggcgaccgggtactgaagaacgcgcagctctcgcgtgccacttcccaggtgtgtgagcctgtaaaattaaacctttgaagatgatctggtatattttagttgtagggattctacttccccagtctttggcccatccaggcttttttacttctattggtcagatgactgatttgattcatactgaaaaagatctggtgacttccctgaaagactatataaaggcagaagaggacaaattagaacaaataaaaaaatgggcagagaaattagatcgattaaccagcacagcgacaaaagatccagaaggatttgttggacaccctgtaaatgcattcaaattaatgaaacgtctgaacactgagtggagtgagttggagaatctggtccttaaggatatgtcagatggttttatctctaacctaaccattcagagacagtacttccctaatgatgaagatcaggttggggcagccaaagctctgttgcgtctacaggacacctacaatttggatacagataccatctcaaagggtgatcttccaggagtaaaacacaaatcttttctaacagttgaggactgttttgagttgggcaaagtggcctacacagaagcagattattaccatacagagctgtggatggaacaagcactgaggcagctggatgaaggcgaggtttctaccgttgataaagtctctgttctggattatttgagctatgcagtataccagcagggagacctggataaggcgcttttgctcacaaagaagcttcttgaactagatcctgaacatcagagagctaacggtaacttaaaatactttgagtatataatggctaaagaaaaagatgccaataagtcttcttcagatgaccaatctgatcagaaaaccacactgaagaagaaaggtgctgctgtggattacctgccagagagacagaagtacgaaatgctgtgccgtggggagggtatcaaaatgactcctcggagacagaaaaaactcttctgtcgctaccatgatggaaaccggaatcctaaatttatcctggctccagccaaacaggaggatgagtgggacaagcctcgtattatccgcttccatgatattatttctgatgcagaaattgaagtcgttaaagatctagcaaaaccaaggctgaggcgagccaccatttcaaacccaataacaggagacttggagacggtacattacagaattagcaaaagtgcctggctgtctggctatgaaaaccctgtggtgtcacgaattaatatgagaatccaagatctgacaggactagatgtctccacagcagaggaattacaggtagcaaattatggagttggaggacagtatgaaccccattttgattttgcacggaaagatgagccagatgctttcaaagagctggggacaggaaatagaattgctacatggctgttttatatgagtgatgtgttagcaggaggagccactgtttttcctgaagtaggagctagtgtttggcccaaaaagggaactgctgttttctggtataatctgtttgccagtggagaaggagattatagtacacggcatgcagcctgtccagtgctggttggaaacaaatgggtatccaataaatggctccatgaacgtggacaggaatttcgaagaccatgcaccttgtcagaattggaatgacaaatgaactttctctcctgttgtactctaatgtgtctgatacacacaattcccagtcttaactttcaagagtttacaattgactaacactccgtgattgattcagtcatgaacctcatcccatgtttcatctgtggacaatcactaactttgtggggtttgttttttttttcttttaaaagtaacactaaatcaccacattgtacatataaaaaaccttaaagttcagttggcatcacagaggacaaaaagacagggttaaaaatgaggaacttttacctttatattaaaaaaatttttttttagttggggaaaaaaaaagtcaagcatctgattataatatttcagtatatctctgttggtgggtggtggactaaaatggtccatctgattaaggaacagatgccttatagtgtatacctaggtactgtgtttacctagtcttaactttcttctggatctgcctgacgactaggaataaattagccctctaaactcggttcagtttaacgtttgcccctatgtttactaagtagattttttcttctcccaagtcctttctaaagtattctttatttttaccaatctgttcctttcatagctcctctgtggtgaattaaatttgagttaaaatactttgattttaaaaaaaatttaacagaaggtcctacattaaaaagttttggccttcttaacagaaatgatcatgacttagtctgtttctgctttttcttaaatgactcatgattttgtccaggaatttttgttgttttccttagtgctaattccttgcctcttgttccagctatagacagcgggggatgatgatgttggcattcagattaaataaatactgtgccttaggagactggaaattttaaaatgtacaagttctttcaatgatgagggaattgataaaaaaaaaaaaaaaaaaaaaaaaaaaaaaaaaaaaaaaaaaaaaaaaaaaaaaaaaaaaaaaaaaaaaaaaaaaaaaaaaaaaaaaaaaaaaaaaaaaaaaaaaaaaaaaaaaaaaaaaaaaaaaaaaaaaaaaaaaaaaaaaaaaaaaaaaaaaaaaaaa

SEQ ID NO: 55 - protein, 534 aa, Bos taurus
MIWYILVVGILLPQSLAHPGFFTSIGQMTDLIHTEKDLVTSLKDYIKAEEDKLEQIKKWAEKLDRLTSTATKDPEGFVGHPVNAFKLMKRLNTEWSELENLVLKDMSDGFISNLTIQRQYFPNDEDQVGAAKALLRLQDTYNLDTDTISKGDLPGVKHKSFLTVEDCFELGKVAYTEADYYHTELWMEQALRQLDEGEVSTVDKVSVLDYLSYAVYQQGDLDKALLLTKKLLELDPEHQRANGNLKYFEYIMAKEKDANKSSSDDQSDQKTTLKKKGAAVDYLPERQKYEMLCRGEGIKMTPRRQKKLFCRYHDGNRNPKFILAPAKQEDEWDKPRIIRFHDIISDAEIEVVKDLAKPRLRRATISNPITGDLETVHYRISKSAWLSGYENPVVSRINMRIQDLTGLDVSTAEELQVANYGVGGQYEPHFDFARKDEPDAFKELGTGNRIATWLFYMSDVLAGGATVFPEVGASVWPKKGTAVFWYNLFASGEGDYSTRHAACPVLVGNKWVSNKWLHERGQEFRRPCTLSELE